European Patent Application EP 4 814 121 A1, published September 30, 2026. Title: Method for increasing Prime Editing efficiency in plants. Applicant: INDUSTRY-ACADEMIC COOPERATION FOUNDATION GYEONGSANG NATIONAL UNIVERSITY. Application KR. The sequence listing filed with the application follows.

SEQUENCE LISTING (278 sequences)

SEQ ID NO: 1 - DNA, 6396 bp, synthetic construct
  source 1..6396: mol_type = other DNA
atgaaacggacagccgacggaagcgagttcgagtcaccaaagaagaagcggaaagtcgacaagaagtacagcatcggcctggacatcggcaccaactctgtgggctgggccgtgatcaccgacgagtacaaggtgcccagcaagaaattcaaggtgctgggcaacaccgaccggcacagcatcaagaagaacctgatcggagccctgctgttcgacagcggcgaaacagccgaggccacccggctgaagagaaccgccagaagaagatacaccagacggaagaaccggatctgctatctgcaagagatcttcagcaacgagatggccaaggtggacgacagcttcttccacagactggaagagtccttcctggtggaagaggataagaagcacgagcggcaccccatcttcggcaacatcgtggacgaggtggcctaccacgagaagtaccccaccatctaccacctgagaaagaaactggtggacagcaccgacaaggccgacctgcggctgatctatctggccctggcccacatgatcaagttccggggccacttcctgatcgagggcgacctgaaccccgacaacagcgacgtggacaagctgttcatccagctggtgcagacctacaaccagctgttcgaggaaaaccccatcaacgccagcggcgtggacgccaaggccatcctgtctgccagactgagcaagagcagaaagctggaaaatctgatcgcccagctgcccggcgagaagaagaatggcctgttcggaaacctgattgccctgagcctgggcctgacccccaacttcaagagcaacttcgacctggccgaggatgccaaactgcagctgagcaaggacacctacgacgacgacctggacaacctgctggcccagatcggcgaccagtacgccgacctgtttctggccgccaagaacctgtccgacgccatcctgctgagcgacatcctgagagtgaacaccgagatcaccaaggcccccctgagcgcctctatgatcaagagatacgacgagcaccaccaggacctgaccctgctgaaagctctcgtgcggcagcagctgcctgagaagtacaaagagattttcttcgaccagagcaagaacggctacgccggctacattgacggcggagccagccaggaagagttctacaagttcatcaagcccatcctggaaaagatggacggcaccgaggaactgctcgtgaagctgaagagagaggacctgctgcggaagcagcggaccttcgacaacggcagcatcccccaccagatccacctgggagagctgcacgccattctgcggcggcaggaagatttttacccattcctgaaggacaaccgggaaaagatcgagaagatcctgaccttccgcatcccctactacgtgggccctctggccaggggaaacagcagattcgcctggatgaccagaaagagcgaggaaaccatcaccccctggaacttcgaggaagtggtggacaagggcgcttccgcccagagcttcatcgagcggatgaccaacttcgataagaacctgcccaacgagaaggtgctgcccaagcacagcctgctgtacgagtacttcaccgtgtataacgagctgaccaaagtgaaatacgtgaccgagggaatgagaaagcccgccttcctgagcggcgagcagaaaaaggccatcgtggacctgctgttcaagaccaaccggaaagtgaccgtgaagcagctgaaagaggactacttcaagaaaatcgagtgcttcgactccgtggaaatctccggcgtggaagatcggttcaacgcctccctgggcacataccacgatctgctgaaaattatcaaggacaaggacttcctggacaatgaggaaaacgaggacattctggaagatatcgtgctgaccctgacactgtttgaggacagagagatgatcgaggaacggctgaaaacctatgcccacctgttcgacgacaaagtgatgaagcagctgaagcggcggagatacaccggctggggcaggctgagccggaagctgatcaacggcatccgggacaagcagtccggcaagacaatcctggatttcctgaagtccgacggcttcgccaacagaaacttcatgcagctgatccacgacgacagcctgacctttaaagaggacatccagaaagcccaggtgtccggccagggcgatagcctgcacgagcacattgccaatctggccggcagccccgccattaagaagggcatcctgcagacagtgaaggtggtggacgagctcgtgaaagtgatgggccggcacaagcccgagaacatcgtgatcgaaatggccagagagaaccagaccacccagaagggacagaagaacagccgcgagagaatgaagcggatcgaagagggcatcaaagagctgggcagccagatcctgaaagaacaccccgtggaaaacacccagctgcagaacgagaagctgtacctgtactacctgcagaatgggcgggatatgtacgtggaccaggaactggacatcaaccggctgtccgactacgatgtggacgctatcgtgcctcagagctttctgaaggacgactccatcgacaacaaggtgctgaccagaagcgacaagaaccggggcaagagcgacaacgtgccctccgaagaggtcgtgaagaagatgaagaactactggcggcagctgctgaacgccaagctgattacccagagaaagttcgacaatctgaccaaggccgagagaggcggcctgagcgaactggataaggccggcttcatcaagagacagctggtggaaacccggcagatcacaaagcacgtggcacagatcctggactcccggatgaacactaagtacgacgagaatgacaagctgatccgggaagtgaaagtgatcaccctgaagtccaagctggtgtccgatttccggaaggatttccagttttacaaagtgcgcgagatcaacaactaccaccacgcccacgacgcctacctgaacgccgtcgtgggaaccgccctgatcaaaaagtaccctaagctggaaagcgagttcgtgtacggcgactacaaggtgtacgacgtgcggaagatgatcgccaagagcgagcaggaaatcggcaaggctaccgccaagtacttcttctacagcaacatcatgaactttttcaagaccgagattaccctggccaacggcgagatccggaagcggcctctgatcgagacaaacggcgaaaccggggagatcgtgtgggataagggccgggattttgccaccgtgcggaaagtgctgagcatgccccaagtgaatatcgtgaaaaagaccgaggtgcagacaggcggcttcagcaaagagtctatcctgcccaagaggaacagcgataagctgatcgccagaaagaaggactgggaccctaagaagtacggcggcttcgacagccccaccgtggcctattctgtgctggtggtggccaaagtggaaaagggcaagtccaagaaactgaagagtgtgaaagagctgctggggatcaccatcatggaaagaagcagcttcgagaagaatcccatcgactttctggaagccaagggctacaaagaagtgaaaaaggacctgatcatcaagctgcctaagtactccctgttcgagctggaaaacggccggaagagaatgctggcctctgccggcgaactgcagaagggaaacgaactggccctgccctccaaatatgtgaacttcctgtacctggccagccactatgagaagctgaagggctcccccgaggataatgagcagaaacagctgtttgtggaacagcacaagcactacctggacgagatcatcgagcagatcagcgagttctccaagagagtgatcctggccgacgctaatctggacaaagtgctgtccgcctacaacaagcaccgggataagcccatcagagagcaggccgagaatatcatccacctgtttaccctgaccaatctgggagcccctgccgccttcaagtactttgacaccaccatcgaccggaagaggtacaccagcaccaaagaggtgctggacgccaccctgatccaccagagcatcaccggcctgtacgagacacggatcgacctgtctcagctgggaggtgactccggcggaagctctggtggcagcaagcggaccgccgacggctctgaattcgagagccctaagaagaaaagaaaggtgagcggaggctctagcggcggaagcaccctgaacattgaagatgagtatagactgcatgaaacaagcaaggaacccgacgtgtccctgggctccacctggctgtccgactttccccaggcctgggccgagacaggaggaatgggcctggccgtgcggcaggcacccctgatcatccctctgaaggccacctctacacccgtgagcatcaagcagtaccctatgtctcaggaggccagactgggcatcaagcctcacatccagaggctgctggaccagggcatcctggtgccatgccagagcccctggaacacaccactgctgcccgtgaagaagccaggcaccaatgactatagacccgtgcaggatctgagagaggtgaacaagagggtggaggatatccaccccaccgtgcccaacccttacaatctgctgtccggcctgcccccttctcaccagtggtatacagtgctggacctgaaggatgccttcttttgtctgagactgcaccctaccagccagccactgttcgcctttgagtggagggaccctgagatgggcatctctggccagctgacctggacacgcctgcctcagggcttcaagaatagcccaacactgtttaacgaggccctgcaccgcgacctggcagatttccggatccagcacccagatctgatcctgctgcagtacgtggacgatctgctgctggccgccaccagcgagctggattgccagcagggaacacgcgccctgctgcagaccctgggaaacctgggatatagggcatccgccaagaaggcccagatctgtcagaagcaggtgaagtacctgggctatctgctgaaggagggccagagatggctgacagaggccaggaaggagacagtgatgggccagccaacacccaagaccccaagacagctgagggagttcctgggcaaagcaggattttgcaggctgttcatcccaggattcgcagagatggcagcacctctgtacccactgaccaagccgggcaccctgtttaattggggccctgaccagcagaaggcctatcaggagatcaagcaggccctgctgacagcaccagccctgggcctgccagacctgaccaagcctttcgagctgtttgtggatgagaagcagggctacgccaagggcgtgctgacccagaagctgggaccatggagacggcccgtggcctatctgtccaagaagctggacccagtggcagcaggatggccaccatgcctgaggatggtggcagcaatcgccgtgctgacaaaggatgccggcaagctgaccatgggacagccactggtcatcctggcaccacacgcagtggaggccctggtgaagcagcctccagatcgctggctgtctaacgcccggatgacacactaccaggccctgctgctggacaccgatcgcgtgcagtttggccctgtggtggccctgaatccagccaccctgctgcctctgccagaggagggcctgcagcacaactgtctggacatcctggcagaggcacacggaacaaggccagacctgaccgatcagcccctgcctgacgccgatcacacatggtataccgatggaagctccctgctgcaggagggccagaggaaggcaggagcagcagtgaccacagagacagaagtgatctgggccaaggccctgccagcaggcacatccgcccagcgggccgagctgatcgccctgacccaggccctgaagatggccgagggcaagaagctgaacgtgtacacagactccagatatgccttcgccaccgcacacatccacggagagatctacaggcgccggggctggctgacctctgagggcaaggagatcaagaacaaggatgagatcctggccctgctgaaggccctgtttctgcccaagcggctgagcatcatccactgtcctggacaccagaagggacactccgccgaggcaaggggcaatcggatggccgaccaggccgccagaaaggctgctattactgaaactcccgacacttccactctgctgattgaaaactcctccccttctggcggctcaaaaagaaccgccgacggcagcgaattcgagtctcccaagaagaagaggaaagtcggctctggccctgccgctaagagagtgaagctggactaa

SEQ ID NO: 2 - DNA, 8745 bp, synthetic construct
  source 1..8745: mol_type = other DNA
atgaaacggacagccgacggaagcgagttcgagtcaccaaagaagaagcggaaagtcgacaagaagtacagcatcggcctggacatcggcaccaactctgtgggctgggccgtgatcaccgacgagtacaaggtgcccagcaagaaattcaaggtgctgggcaacaccgaccggcacagcatcaagaagaacctgatcggagccctgctgttcgacagcggcgaaacagccgaggccacccggctgaagagaaccgccagaagaagatacaccagacggaagaaccggatctgctatctgcaagagatcttcagcaacgagatggccaaggtggacgacagcttcttccacagactggaagagtccttcctggtggaagaggataagaagcacgagcggcaccccatcttcggcaacatcgtggacgaggtggcctaccacgagaagtaccccaccatctaccacctgagaaagaaactggtggacagcaccgacaaggccgacctgcggctgatctatctggccctggcccacatgatcaagttccggggccacttcctgatcgagggcgacctgaaccccgacaacagcgacgtggacaagctgttcatccagctggtgcagacctacaaccagctgttcgaggaaaaccccatcaacgccagcggcgtggacgccaaggccatcctgtctgccagactgagcaagagcagaaagctggaaaatctgatcgcccagctgcccggcgagaagaagaatggcctgttcggaaacctgattgccctgagcctgggcctgacccccaacttcaagagcaacttcgacctggccgaggatgccaaactgcagctgagcaaggacacctacgacgacgacctggacaacctgctggcccagatcggcgaccagtacgccgacctgtttctggccgccaagaacctgtccgacgccatcctgctgagcgacatcctgagagtgaacaccgagatcaccaaggcccccctgagcgcctctatgatcaagagatacgacgagcaccaccaggacctgaccctgctgaaagctctcgtgcggcagcagctgcctgagaagtacaaagagattttcttcgaccagagcaagaacggctacgccggctacattgacggcggagccagccaggaagagttctacaagttcatcaagcccatcctggaaaagatggacggcaccgaggaactgctcgtgaagctgaagagagaggacctgctgcggaagcagcggaccttcgacaacggcagcatcccccaccagatccacctgggagagctgcacgccattctgcggcggcaggaagatttttacccattcctgaaggacaaccgggaaaagatcgagaagatcctgaccttccgcatcccctactacgtgggccctctggccaggggaaacagcagattcgcctggatgaccagaaagagcgaggaaaccatcaccccctggaacttcgaggaagtggtggacaagggcgcttccgcccagagcttcatcgagcggatgaccaacttcgataagaacctgcccaacgagaaggtgctgcccaagcacagcctgctgtacgagtacttcaccgtgtataacgagctgaccaaagtgaaatacgtgaccgagggaatgagaaagcccgccttcctgagcggcgagcagaaaaaggccatcgtggacctgctgttcaagaccaaccggaaagtgaccgtgaagcagctgaaagaggactacttcaagaaaatcgagtgcttcgactccgtggaaatctccggcgtggaagatcggttcaacgcctccctgggcacataccacgatctgctgaaaattatcaaggacaaggacttcctggacaatgaggaaaacgaggacattctggaagatatcgtgctgaccctgacactgtttgaggacagagagatgatcgaggaacggctgaaaacctatgcccacctgttcgacgacaaagtgatgaagcagctgaagcggcggagatacaccggctggggcaggctgagccggaagctgatcaacggcatccgggacaagcagtccggcaagacaatcctggatttcctgaagtccgacggcttcgccaacagaaacttcatgcagctgatccacgacgacagcctgacctttaaagaggacatccagaaagcccaggtgtccggccagggcgatagcctgcacgagcacattgccaatctggccggcagccccgccattaagaagggcatcctgcagacagtgaaggtggtggacgagctcgtgaaagtgatgggccggcacaagcccgagaacatcgtgatcgaaatggccagagagaaccagaccacccagaagggacagaagaacagccgcgagagaatgaagcggatcgaagagggcatcaaagagctgggcagccagatcctgaaagaacaccccgtggaaaacacccagctgcagaacgagaagctgtacctgtactacctgcagaatgggcgggatatgtacgtggaccaggaactggacatcaaccggctgtccgactacgatgtggacgctatcgtgcctcagagctttctgaaggacgactccatcgacaacaaggtgctgaccagaagcgacaagaaccggggcaagagcgacaacgtgccctccgaagaggtcgtgaagaagatgaagaactactggcggcagctgctgaacgccaagctgattacccagagaaagttcgacaatctgaccaaggccgagagaggcggcctgagcgaactggataaggccggcttcatcaagagacagctggtggaaacccggcagatcacaaagcacgtggcacagatcctggactcccggatgaacactaagtacgacgagaatgacaagctgatccgggaagtgaaagtgatcaccctgaagtccaagctggtgtccgatttccggaaggatttccagttttacaaagtgcgcgagatcaacaactaccaccacgcccacgacgcctacctgaacgccgtcgtgggaaccgccctgatcaaaaagtaccctaagctggaaagcgagttcgtgtacggcgactacaaggtgtacgacgtgcggaagatgatcgccaagagcgagcaggaaatcggcaaggctaccgccaagtacttcttctacagcaacatcatgaactttttcaagaccgagattaccctggccaacggcgagatccggaagcggcctctgatcgagacaaacggcgaaaccggggagatcgtgtgggataagggccgggattttgccaccgtgcggaaagtgctgagcatgccccaagtgaatatcgtgaaaaagaccgaggtgcagacaggcggcttcagcaaagagtctatcctgcccaagaggaacagcgataagctgatcgccagaaagaaggactgggaccctaagaagtacggcggcttcgacagccccaccgtggcctattctgtgctggtggtggccaaagtggaaaagggcaagtccaagaaactgaagagtgtgaaagagctgctggggatcaccatcatggaaagaagcagcttcgagaagaatcccatcgactttctggaagccaagggctacaaagaagtgaaaaaggacctgatcatcaagctgcctaagtactccctgttcgagctggaaaacggccggaagagaatgctggcctctgccggcgaactgcagaagggaaacgaactggccctgccctccaaatatgtgaacttcctgtacctggccagccactatgagaagctgaagggctcccccgaggataatgagcagaaacagctgtttgtggaacagcacaagcactacctggacgagatcatcgagcagatcagcgagttctccaagagagtgatcctggccgacgctaatctggacaaagtgctgtccgcctacaacaagcaccgggataagcccatcagagagcaggccgagaatatcatccacctgtttaccctgaccaatctgggagcccctgccgccttcaagtactttgacaccaccatcgaccggaagaggtacaccagcaccaaagaggtgctggacgccaccctgatccaccagagcatcaccggcctgtacgagacacggatcgacctgtctcagctgggaggtgactccggcggaagctctggtggcagcaagcggaccgccgacggctctgaattcgagagccctaagaagaaaagaaaggtgagcggaggctctagcggcggaagcaccctgaacattgaagatgagtatagactgcatgaaacaagcaaggaacccgacgtgtccctgggctccacctggctgtccgactttccccaggcctgggccgagacaggaggaatgggcctggccgtgcggcaggcacccctgatcatccctctgaaggccacctctacacccgtgagcatcaagcagtaccctatgtctcaggaggccagactgggcatcaagcctcacatccagaggctgctggaccagggcatcctggtgccatgccagagcccctggaacacaccactgctgcccgtgaagaagccaggcaccaatgactatagacccgtgcaggatctgagagaggtgaacaagagggtggaggatatccaccccaccgtgcccaacccttacaatctgctgtccggcctgcccccttctcaccagtggtatacagtgctggacctgaaggatgccttcttttgtctgagactgcaccctaccagccagccactgttcgcctttgagtggagggaccctgagatgggcatctctggccagctgacctggacacgcctgcctcagggcttcaagaatagcccaacactgtttaacgaggccctgcaccgcgacctggcagatttccggatccagcacccagatctgatcctgctgcagtacgtggacgatctgctgctggccgccaccagcgagctggattgccagcagggaacacgcgccctgctgcagaccctgggaaacctgggatatagggcatccgccaagaaggcccagatctgtcagaagcaggtgaagtacctgggctatctgctgaaggagggccagagatggctgacagaggccaggaaggagacagtgatgggccagccaacacccaagaccccaagacagctgagggagttcctgggcaaagcaggattttgcaggctgttcatcccaggattcgcagagatggcagcacctctgtacccactgaccaagccgggcaccctgtttaattggggccctgaccagcagaaggcctatcaggagatcaagcaggccctgctgacagcaccagccctgggcctgccagacctgaccaagcctttcgagctgtttgtggatgagaagcagggctacgccaagggcgtgctgacccagaagctgggaccatggagacggcccgtggcctatctgtccaagaagctggacccagtggcagcaggatggccaccatgcctgaggatggtggcagcaatcgccgtgctgacaaaggatgccggcaagctgaccatgggacagccactggtcatcctggcaccacacgcagtggaggccctggtgaagcagcctccagatcgctggctgtctaacgcccggatgacacactaccaggccctgctgctggacaccgatcgcgtgcagtttggccctgtggtggccctgaatccagccaccctgctgcctctgccagaggagggcctgcagcacaactgtctggacatcctggcagaggcacacggaacaaggccagacctgaccgatcagcccctgcctgacgccgatcacacatggtataccgatggaagctccctgctgcaggagggccagaggaaggcaggagcagcagtgaccacagagacagaagtgatctgggccaaggccctgccagcaggcacatccgcccagcgggccgagctgatcgccctgacccaggccctgaagatggccgagggcaagaagctgaacgtgtacacagactccagatatgccttcgccaccgcacacatccacggagagatctacaggcgccggggctggctgacctctgagggcaaggagatcaagaacaaggatgagatcctggccctgctgaaggccctgtttctgcccaagcggctgagcatcatccactgtcctggacaccagaagggacactccgccgaggcaaggggcaatcggatggccgaccaggccgccagaaaggctgctattactgaaactcccgacacttccactctgctgattgaaaactcctccccttctggcggctcaaaaagaaccgccgacggcagcgaattcgagtctcccaagaagaagaggaaagtcggctctggccctgccgctaagagagtgaagctggacggaagcggagctactaacttcagcctgctgaagcaggctggagacgtggaggagaaccctggacctagcttcgttgctggagtcatccggagactggacgagacagtggtgaacagaattgccgccggcgaggtgatccaaagacctgccaatgcaataaaggagatgatcgagaactgtctggacgccaagtccacaagcattcaggtgatcgtgaaggagggcggactgaagctgatccagatccaagacaacggcacaggcatcagaaaggaagatctggacatcgtgtgtgaacggttcaccacatctaagctgcagtcttttgaggatctggcctctatcagtacctacggcttcagaggcgaggccctggccagcatcagccacgtggcccatgtgaccatcaccaccaaaaccgccgacggcaaatgcgcttatcgcgctagctacagcgacggcaagctgaaagccccgccaaagccttgcgccggcaaccagggtacacagataacagtggaggatctgttctacaacatcgccacccggagaaaggccctgaaaaatcccagcgaggagtacggcaagatcctggaagtcgtcggcagatactccgtgcacaacgccggaatcagctttagcgtaaagaagcagggagaaaccgtggccgatgtgcgcaccctgccaaatgccagcaccgtggataacatcagaagcattttcggaaatgccgtgtccagagaactgatcgagatcggctgcgaagataagaccctggcttttaagatgaacggctacatcagcaacgccaattactctgtgaagaagtgcatctttcttctgttcatcaaccacagactggtggaaagcaccagcctgcggaaagccatcgagacagtgtacgccgcctacctgcctaagaacacccaccccttcctgtacctgagcctcgagatcagccctcagaacgtggacgtcaatgtgcatcctacaaagcacgaggtgcacttcctgcacgaggaaagcatcctggaaagagtgcagcagcacattgagagcaagctgctgggctctaacagcagcagaatgtacttcacacagaccctgctgcctggcctggccggcccctcaggcgaaatggttaagtccacaacctctctgacctcatccagcaccagcggttcttccgataaggtgtacgcccaccagatggtgcggaccgactctcgggagcagaagctggacgcctttctgcaacctctgagcaaacctctgagctctcagcctcaggccatcgtgaccgaggacaagacagatatctcctccggccgtgccagacagcaggacgaagaaatgctcgagctgccagctcctgccgaggtggccgccaagaaccagagcctggagggagataccacaaagggcaccagcgaaatgagcgagaagcggggccctacctccagcaaccccagaaaacggcaccgggaggacagcgacgtggaaatggtggaggacgacagcagaaaggaaatgacagccgcttgtacccctagaagaagaatcatcaacctgacctccgtgctgagcctgcaggaggagatcaacgagcagggccacgaggtgctgagagagatgctgcacaatcacagcttcgtgggctgcgtgaaccctcaatgggccctggctcagcatcaaacaaagctgtacctgctgaacaccaccaagctgagcgaagagctgttctaccagatcctcatctacgacttcgccaacttcggcgtgctacgcctgagcgagcccgcccctctgtttgacctggccatgctggctctggatagcccagaaagcggctggacagaagaggacggacctaaagaggggctggctgaatacatcgtggagttcctgaagaaaaaggccgagatgctggccgactacttttctctggaaatcgacgaggaaggcaacctgatcggcctgcctctgctgatcgataactacgtgcctcccctggaaggcctgcccatcttcatcctgagactggctacagaggtgaactgggacgaggaaaaggaatgcttcgagtctctgagcaaggagtgcgccatgttctatagcatcagaaaacagtacatctctgaagagagcactctgtctggccagcagagtgaagtgcccggaagcatccccaacagctggaagtggaccgtggaacacatcgtgtacaaggccctgcggagccacattctccctcctaagcacttcaccgaggacggcaacatcctgcagctggccaacctgcccgacctttataaggttttcggcagcccgaagaagaaaaggaaggtgtaa

SEQ ID NO: 3 - DNA, 6549 bp, synthetic construct
  source 1..6549: mol_type = other DNA
atgcctaagaaaaagagaaaagtggacaagaagtactcgatcggcctcgatattgggactaactctgttggctgggccgtgatcaccgacgagtacaaggtgccctcaaagaagttcaaggtcctgggcaacaccgatcggcattccatcaagaagaatctcattggcgctctcctgttcgacagcggcgagacggctgaggctacgcggctcaagcgcaccgcccgcaggcggtacacgcgcaggaagaatcgcatctgctacctgcaggagattttctccaacgagatggcgaaggttgacgattctttcttccacaggctggaggagtcattcctcgtggaggaggataagaagcacgagcggcatccaatcttcggcaacattgtcgacgaggttgcctaccacgagaagtaccctacgatctaccatctgcggaagaagctcgtggactccacagataaggcggacctccgcctgatctacctcgctctggcccacatgattaagttcaggggccatttcctgatcgagggggatctcaacccggacaatagcgatgttgacaagctgttcatccagctcgtgcagacgtacaaccagctcttcgaggagaaccccattaatgcgtcaggcgtcgacgcgaaggctatcctgtccgctaggctctcgaagtctcggcgcctcgagaacctgatcgcccagctgccgggcgagaagaagaacggcctgttcgggaatctcattgcgctcagcctggggctcacgcccaacttcaagtcgaatttcgatctcgctgaggacgccaagctgcagctctccaaggacacatacgacgatgacctggataacctcctggcccagatcggcgatcagtacgcggacctgttcctcgctgccaagaatctgtcggacgccatcctcctgtctgatattctcagggtgaacaccgagattacgaaggctccgctctcagcctccatgatcaagcgctacgacgagcaccatcaggatctgaccctcctgaaggcgctggtcaggcagcagctccccgagaagtacaaggagatcttcttcgatcagtcgaagaacggctacgctgggtacattgacggcggggcctctcaggaggagttctacaagttcatcaagccgattctggagaagatggacggcacggaggagctgctggtgaagctcaatcgcgaggacctcctgaggaagcagcggacattcgataacggcagcatcccacaccagattcatctcggggagctgcacgctatcctgaggaggcaggaggacttctaccctttcctcaaggataaccgcgagaagatcgagaagattctgactttcaggatcccgtactacgtcggcccactcgctaggggcaactcccgcttcgcttggatgacccgcaagtcagaggagacgatcacgccgtggaacttcgaggaggtggtcgacaagggcgctagcgctcagtcgttcatcgagaggatgacgaatttcgacaagaacctgccaaatgagaaggtgctccctaagcactcgctcctgtacgagtacttcacagtctacaacgagctgactaaggtgaagtatgtgaccgagggcatgaggaagccggctttcctgtctggggagcagaagaaggccatcgtggacctcctgttcaagaccaaccggaaggtcacggttaagcagctcaaggaggactacttcaagaagattgagtgcttcgattcggtcgagatctctggcgttgaggaccgcttcaacgcctccctggggacctaccacgatctcctgaagatcattaaggataaggacttcctggacaacgaggagaatgaggatatcctcgaggacattgtgctgacactcactctgttcgaggaccgggagatgatcgaggagcgccttaagacttacgcccatctcttcgatgacaaggtcatgaagcagctcaagaggaggaggtacaccggctgggggaggctgagcaggaagctcatcaacggcattcgggacaagcagtccggaaagacgatcctcgacttcctgaagagcgatggcttcgcgaaccgcaatttcatgcagctgattcacgatgacagcctcacattcaaggaggatatccagaaggctcaggtgagcggccagggggactcgctgcacgagcatatcgcgaacctcgctggctcgccagctatcaagaaggggattctgcagaccgtgaaggttgtggacgagctggtgaaggtcatgggcaggcacaagcctgagaacatcgtcattgagatggcccgggagaatcagaccacgcagaagggccagaagaactcacgcgagaggatgaagaggatcgaggagggcattaaggagctggggtcccagatcctcaaggagcacccggtggagaacacgcagctgcagaatgagaagctctacctgtactacctccagaatggccgcgatatgtatgtggaccaggagctggatattaacaggctcagcgattacgacgtcgatgccatcgttccacagtcattcctgaaggatgactccattgacaacaaggtcctcaccaggtcggacaagaaccggggcaagtctgataatgttccttcagaggaggtcgttaagaagatgaagaactactggcgccagctcctgaatgccaagctgatcacgcagcggaagttcgataacctcacaaaggctgagaggggcgggctctctgagctggacaaggcgggcttcatcaagaggcagctggtcgagacacggcagatcactaagcacgttgcgcagattctcgactcacggatgaacactaagtacgatgagaatgacaagctgatccgcgaggtgaaggtcatcaccctgaagtcaaagctcgtctccgacttcaggaaggatttccagttctacaaggttcgggagatcaacaattaccaccatgcccatgacgcgtacctgaacgcggtggtcggcacagctctgatcaagaagtacccaaagctcgagagcgagttcgtgtacggggactacaaggtttacgatgtgaggaagatgatcgccaagtcggagcaggagattggcaaggctaccgccaagtacttcttctactctaacattatgaatttcttcaagacagagatcactctggccaatggcgagatccggaagcgccccctcatcgagacgaacggcgagacgggggagatcgtgtgggacaagggcagggatttcgcgaccgtcaggaaggttctctccatgccacaagtgaatatcgtcaaaaagacagaggtccagactggcgggttctctaaggagtcaattctgcctaagcggaacagcgacaagctcatcgcccgcaagaaggactgggatccgaagaagtacggcgggttcgacagccccactgtggcctactcggtcctggttgtggcgaaggttgagaagggcaagtccaagaagctcaagagcgtgaaggagctgctggggatcacgattatggagcgctccagcttcgagaagaacccgatcgatttcctggaggcgaagggctacaaggaggtgaagaaggacctgatcattaagctccccaagtactcactcttcgagctggagaacggcaggaagcggatgctggcttccgctggcgagctgcagaaggggaacgagctggctctgccgtccaagtatgtgaacttcctctacctggcctcccactacgagaagctcaagggcagccccgaggacaacgagcagaagcagctgttcgtcgagcagcacaagcattacctcgacgagatcattgagcagatttccgagttctccaagcgcgtgatcctggccgacgcgaatctggataaggtcctctccgcgtacaacaagcaccgcgacaagccaatcagggagcaggctgagaatatcattcatctcttcaccctgacgaacctcggcgcccctgctgctttcaagtacttcgacacaactatcgatcgcaagaggtacacaagcactaaggaggtcctggacgcgaccctcatccaccagtcgattaccggcctctacgagacgcgcatcgacctgtctcagctcgggggcgacgaattctccgggagcgagacgccaggcacctccgagtcggccaccccagaatctgccacagtggtgtccggccaaaagcaggaccgccagggcggagaacgcagaaggtcccagctcgatagggatcagtgtgcctactgcaaggagaagggccactgggccaaagactgcccgaaaaagccgcgcggcccacgcggcccaaggccacaaacatccctccttggttcgccaaagaagaagcggaaggtggagctcagcggaggatcttccggaggatctagcggctccgagacaccaggaacatccgaaagcgctacaccagaatctagcggaggctcttccggaggatctaggcctaccctcaacatcgaggatgagtatcgcctccacgaaacctccaaagaaccggacgtgtccctcggcagcacatggctcagcgacttcccacaagcgtgggccgaaaccggcggcatgggcctcgccgtccgccaagccccactcattatcccgctgaaggcgacctccacaccggtgtccatcaagcagtacccgatgagccaagaggcgaggctcgggattaagccgcacattcagcgcctcctcgatcaaggcattctcgtgccgtgccaatccccgtggaatacaccactcctcccggtcaaaaagccgggcaccaacgactatcgcccggtccaagatctccgcgaggtcaacaagcgcgtggaagatatccacccgaccgtcccgaacccgtataatctgctctccgggctcccaccatcccaccagtggtatacagtgctggacctcaaagacgccttcttctgtctccgcctccacccaacaagccagccgctcttcgccttcgagtggcgcgacccggagatgggcatctccggccaactgacatggacacgcctcccgcaaggcttcaagaacagcccgacactcttcaacgaggcgctccatagggacctcgcggattttcgcatccagcatccggacctcatcctcctccagtatgtggatgatctcctcctcgccgcgacctccgagctggattgtcaacaaggcacacgcgcgctcctccaaacactcgggaacctcggctatcgcgcgtccgcgaaaaaggcccaaatctgccagaagcaagtgaagtacctcgggtatctgctcaaggaaggccaacgctggctcaccgaagcgcgcaaagaaacagtgatggggcaaccgacaccgaaaacaccacgccagctgcgcgagtttctcggcaaagccggcttctgtcgcctcttcatcccgggctttgccgagatggccgcgccactctacccactcaccaagccgggcacactgtttaactgggggccggatcagcagaaagcctaccaagagatcaaacaagcgctcctcaccgccccagcgctcgggctcccagatctcacaaagccgttcgagctgttcgtcgatgagaagcaaggctacgcgaagggcgtgctcacacagaagctcggcccgtggaggaggccagtggcctatctctccaaaaaactcgatccagtggccgccggctggccaccgtgtctgcgcatggtcgccgcgattgccgtgctcacaaaggatgccggcaaactcacaatgggccagccgctggtgatcctcgcgccacatgccgtggaagccctcgtcaaacagccgccggataggtggctctccaatgcgcgcatgacccattaccaagcgctcctcctcgacaccgatcgcgtccagttcggcccagtggtcgccctcaatccggcgacactgctgccactcccagaggagggcctccaacacaactgtctggatattctcgcggaagcgcatggcacaaggccagacctcacagatcaaccgctcccggatgcggatcacacatggtataccgacggctcctctctgctccaagagggccaaaggaaagccggcgccgcggtgaccacagaaacagaagtgatctgggccaaggccctcccagccggcacatccgcgcaaagggcggaactcatcgcgctcacacaagccctcaagatggccgagggcaagaagctcaacgtctacacagactcccgctatgccttcgccaccgcccacattcacggcgaaatctataggaggcgcggctggctcacaagcgaggggaaggagatcaagaacaaggatgagatcctcgcgctgctcaaggccctctttctcccgaagcgcctctccatcatccactgtccgggccaccaaaaggggcactccgcggaagcgaggggcaataggatggccgatcaagccgcgcgcaaagccgcgattaccgaaaccccagacacatccaccctcctcatcgaaaactcctccccaagcggcggcagcccgaagaagaaaaggaaggtgtaa

SEQ ID NO: 4 - DNA, 6054 bp, synthetic construct
  source 1..6054: mol_type = other DNA
atgcctaagaaaaagagaaaagtggacaagaagtactcgatcggcctcgatattgggactaactctgttggctgggccgtgatcaccgacgagtacaaggtgccctcaaagaagttcaaggtcctgggcaacaccgatcggcattccatcaagaagaatctcattggcgctctcctgttcgacagcggcgagacggctgaggctacgcggctcaagcgcaccgcccgcaggcggtacacgcgcaggaagaatcgcatctgctacctgcaggagattttctccaacgagatggcgaaggttgacgattctttcttccacaggctggaggagtcattcctcgtggaggaggataagaagcacgagcggcatccaatcttcggcaacattgtcgacgaggttgcctaccacgagaagtaccctacgatctaccatctgcggaagaagctcgtggactccacagataaggcggacctccgcctgatctacctcgctctggcccacatgattaagttcaggggccatttcctgatcgagggggatctcaacccggacaatagcgatgttgacaagctgttcatccagctcgtgcagacgtacaaccagctcttcgaggagaaccccattaatgcgtcaggcgtcgacgcgaaggctatcctgtccgctaggctctcgaagtctcggcgcctcgagaacctgatcgcccagctgccgggcgagaagaagaacggcctgttcgggaatctcattgcgctcagcctggggctcacgcccaacttcaagtcgaatttcgatctcgctgaggacgccaagctgcagctctccaaggacacatacgacgatgacctggataacctcctggcccagatcggcgatcagtacgcggacctgttcctcgctgccaagaatctgtcggacgccatcctcctgtctgatattctcagggtgaacaccgagattacgaaggctccgctctcagcctccatgatcaagcgctacgacgagcaccatcaggatctgaccctcctgaaggcgctggtcaggcagcagctccccgagaagtacaaggagatcttcttcgatcagtcgaagaacggctacgctgggtacattgacggcggggcctctcaggaggagttctacaagttcatcaagccgattctggagaagatggacggcacggaggagctgctggtgaagctcaatcgcgaggacctcctgaggaagcagcggacattcgataacggcagcatcccacaccagattcatctcggggagctgcacgctatcctgaggaggcaggaggacttctaccctttcctcaaggataaccgcgagaagatcgagaagattctgactttcaggatcccgtactacgtcggcccactcgctaggggcaactcccgcttcgcttggatgacccgcaagtcagaggagacgatcacgccgtggaacttcgaggaggtggtcgacaagggcgctagcgctcagtcgttcatcgagaggatgacgaatttcgacaagaacctgccaaatgagaaggtgctccctaagcactcgctcctgtacgagtacttcacagtctacaacgagctgactaaggtgaagtatgtgaccgagggcatgaggaagccggctttcctgtctggggagcagaagaaggccatcgtggacctcctgttcaagaccaaccggaaggtcacggttaagcagctcaaggaggactacttcaagaagattgagtgcttcgattcggtcgagatctctggcgttgaggaccgcttcaacgcctccctggggacctaccacgatctcctgaagatcattaaggataaggacttcctggacaacgaggagaatgaggatatcctcgaggacattgtgctgacactcactctgttcgaggaccgggagatgatcgaggagcgccttaagacttacgcccatctcttcgatgacaaggtcatgaagcagctcaagaggaggaggtacaccggctgggggaggctgagcaggaagctcatcaacggcattcgggacaagcagtccggaaagacgatcctcgacttcctgaagagcgatggcttcgcgaaccgcaatttcatgcagctgattcacgatgacagcctcacattcaaggaggatatccagaaggctcaggtgagcggccagggggactcgctgcacgagcatatcgcgaacctcgctggctcgccagctatcaagaaggggattctgcagaccgtgaaggttgtggacgagctggtgaaggtcatgggcaggcacaagcctgagaacatcgtcattgagatggcccgggagaatcagaccacgcagaagggccagaagaactcacgcgagaggatgaagaggatcgaggagggcattaaggagctggggtcccagatcctcaaggagcacccggtggagaacacgcagctgcagaatgagaagctctacctgtactacctccagaatggccgcgatatgtatgtggaccaggagctggatattaacaggctcagcgattacgacgtcgatgccatcgttccacagtcattcctgaaggatgactccattgacaacaaggtcctcaccaggtcggacaagaaccggggcaagtctgataatgttccttcagaggaggtcgttaagaagatgaagaactactggcgccagctcctgaatgccaagctgatcacgcagcggaagttcgataacctcacaaaggctgagaggggcgggctctctgagctggacaaggcgggcttcatcaagaggcagctggtcgagacacggcagatcactaagcacgttgcgcagattctcgactcacggatgaacactaagtacgatgagaatgacaagctgatccgcgaggtgaaggtcatcaccctgaagtcaaagctcgtctccgacttcaggaaggatttccagttctacaaggttcgggagatcaacaattaccaccatgcccatgacgcgtacctgaacgcggtggtcggcacagctctgatcaagaagtacccaaagctcgagagcgagttcgtgtacggggactacaaggtttacgatgtgaggaagatgatcgccaagtcggagcaggagattggcaaggctaccgccaagtacttcttctactctaacattatgaatttcttcaagacagagatcactctggccaatggcgagatccggaagcgccccctcatcgagacgaacggcgagacgggggagatcgtgtgggacaagggcagggatttcgcgaccgtcaggaaggttctctccatgccacaagtgaatatcgtcaaaaagacagaggtccagactggcgggttctctaaggagtcaattctgcctaagcggaacagcgacaagctcatcgcccgcaagaaggactgggatccgaagaagtacggcgggttcgacagccccactgtggcctactcggtcctggttgtggcgaaggttgagaagggcaagtccaagaagctcaagagcgtgaaggagctgctggggatcacgattatggagcgctccagcttcgagaagaacccgatcgatttcctggaggcgaagggctacaaggaggtgaagaaggacctgatcattaagctccccaagtactcactcttcgagctggagaacggcaggaagcggatgctggcttccgctggcgagctgcagaaggggaacgagctggctctgccgtccaagtatgtgaacttcctctacctggcctcccactacgagaagctcaagggcagccccgaggacaacgagcagaagcagctgttcgtcgagcagcacaagcattacctcgacgagatcattgagcagatttccgagttctccaagcgcgtgatcctggccgacgcgaatctggataaggtcctctccgcgtacaacaagcaccgcgacaagccaatcagggagcaggctgagaatatcattcatctcttcaccctgacgaacctcggcgcccctgctgctttcaagtacttcgacacaactatcgatcgcaagaggtacacaagcactaaggaggtcctggacgcgaccctcatccaccagtcgattaccggcctctacgagacgcgcatcgacctgtctcagctcgggggcgacgaattctccgggagcgagacgccaggcacctccgagtcggccaccccagaatctgccacagtggtgtccggccaaaagcaggaccgccagggcggagaacgcagaaggtcccagctcgatagggatcagtgtgcctactgcaaggagaagggccactgggccaaagactgcccgaaaaagccgcgcggcccacgcggcccaaggccacaaacatccctccttccaaagaagaagcggaaggtggagctcagcggaggatcttccggaggatctagcggctccgagacaccaggaacatccgaaagcgctacaccagaatctagcggaggctcttccggaggatctaggcctaccctcaacatcgaggatgagtatcgcctccacgaaacctccaaagaaccggacgtgtccctcggcagcacatggctcagcgacttcccacaagcgtgggccgaaaccggcggcatgggcctcgccgtccgccaagccccactcattatcccgctgaaggcgacctccacaccggtgtccatcaagcagtacccgatgagccaagaggcgaggctcgggattaagccgcacattcagcgcctcctcgatcaaggcattctcgtgccgtgccaatccccgtggaatacaccactcctcccggtcaaaaagccgggcaccaacgactatcgcccggtccaagatctccgcgaggtcaacaagcgcgtggaagatatccacccgaccgtcccgaacccgtataatctgctctccgggctcccaccatcccaccagtggtatacagtgctggacctcaaagacgccttcttctgtctccgcctccacccaacaagccagccgctcttcgccttcgagtggcgcgacccggagatgggcatctccggccaactgacatggacacgcctcccgcaaggcttcaagaacagcccgacactcttcaacgaggcgctccatagggacctcgcggattttcgcatccagcatccggacctcatcctcctccagtatgtggatgatctcctcctcgccgcgacctccgagctggattgtcaacaaggcacacgcgcgctcctccaaacactcgggaacctcggctatcgcgcgtccgcgaaaaaggcccaaatctgccagaagcaagtgaagtacctcgggtatctgctcaaggaaggccaacgctggctcaccgaagcgcgcaaagaaacagtgatggggcaaccgacaccgaaaacaccacgccagctgcgcgagtttctcggcaaagccggcttctgtcgcctcttcatcccgggctttgccgagatggccgcgccactctacccactcaccaagccgggcacactgtttaactgggggccggatcagcagaaagcctaccaagagatcaaacaagcgctcctcaccgccccagcgctcgggctcccagatctcacaaagccgttcgagctgttcgtcgatgagaagcaaggctacgcgaagggcgtgctcacacagaagctcggcccgtggaggaggccagtggcctatctctccaaaaaactcgatccagtggccgccggctggccaccgtgtctgcgcatggtcgccgcgattgccgtgctcacaaaggatgccggcaaactcacaatgggccagccgctggtgatcctcgcgccacatgccgtggaagccctcgtcaaacagccgccggataggtggctctccaatgcgcgcatgacccattaccaagcgctcctcctcgacaccgatcgcgtccagttcggcccagtggtcgccctcaatccggcgacactgctgccactcccagaggagggcctccaacacaactgtctggatattctcgcggaagcgcatggcacaaggccagacctcacagatcaaccgctcagcggcggcagcccgaagaagaaaaggaaggtgtga

SEQ ID NO: 5 - DNA, 5931 bp, synthetic construct
  source 1..5931: mol_type = other DNA
atgaaacggacagccgacggaagcgagttcgagtcaccaaagaagaagcggaaagtcgacaagaagtacagcatcggcctggacatcggcaccaactctgtgggctgggccgtgatcaccgacgagtacaaggtgcccagcaagaaattcaaggtgctgggcaacaccgaccggcacagcatcaagaagaacctgatcggagccctgctgttcgacagcggcgaaacagccgaggccacccggctgaagagaaccgccagaagaagatacaccagacggaagaaccggatctgctatctgcaagagatcttcagcaacgagatggccaaggtggacgacagcttcttccacagactggaagagtccttcctggtggaagaggataagaagcacgagcggcaccccatcttcggcaacatcgtggacgaggtggcctaccacgagaagtaccccaccatctaccacctgagaaagaaactggtggacagcaccgacaaggccgacctgcggctgatctatctggccctggcccacatgatcaagttccggggccacttcctgatcgagggcgacctgaaccccgacaacagcgacgtggacaagctgttcatccagctggtgcagacctacaaccagctgttcgaggaaaaccccatcaacgccagcggcgtggacgccaaggccatcctgtctgccagactgagcaagagcagaaagctggaaaatctgatcgcccagctgcccggcgagaagaagaatggcctgttcggaaacctgattgccctgagcctgggcctgacccccaacttcaagagcaacttcgacctggccgaggatgccaaactgcagctgagcaaggacacctacgacgacgacctggacaacctgctggcccagatcggcgaccagtacgccgacctgtttctggccgccaagaacctgtccgacgccatcctgctgagcgacatcctgagagtgaacaccgagatcaccaaggcccccctgagcgcctctatgatcaagagatacgacgagcaccaccaggacctgaccctgctgaaagctctcgtgcggcagcagctgcctgagaagtacaaagagattttcttcgaccagagcaagaacggctacgccggctacattgacggcggagccagccaggaagagttctacaagttcatcaagcccatcctggaaaagatggacggcaccgaggaactgctcgtgaagctgaagagagaggacctgctgcggaagcagcggaccttcgacaacggcagcatcccccaccagatccacctgggagagctgcacgccattctgcggcggcaggaagatttttacccattcctgaaggacaaccgggaaaagatcgagaagatcctgaccttccgcatcccctactacgtgggccctctggccaggggaaacagcagattcgcctggatgaccagaaagagcgaggaaaccatcaccccctggaacttcgaggaagtggtggacaagggcgcttccgcccagagcttcatcgagcggatgaccaacttcgataagaacctgcccaacgagaaggtgctgcccaagcacagcctgctgtacgagtacttcaccgtgtataacgagctgaccaaagtgaaatacgtgaccgagggaatgagaaagcccgccttcctgagcggcgagcagaaaaaggccatcgtggacctgctgttcaagaccaaccggaaagtgaccgtgaagcagctgaaagaggactacttcaagaaaatcgagtgcttcgactccgtggaaatctccggcgtggaagatcggttcaacgcctccctgggcacataccacgatctgctgaaaattatcaaggacaaggacttcctggacaatgaggaaaacgaggacattctggaagatatcgtgctgaccctgacactgtttgaggacagagagatgatcgaggaacggctgaaaacctatgcccacctgttcgacgacaaagtgatgaagcagctgaagcggcggagatacaccggctggggcaggctgagccggaagctgatcaacggcatccgggacaagcagtccggcaagacaatcctggatttcctgaagtccgacggcttcgccaacagaaacttcatgcagctgatccacgacgacagcctgacctttaaagaggacatccagaaagcccaggtgtccggccagggcgatagcctgcacgagcacattgccaatctggccggcagccccgccattaagaagggcatcctgcagacagtgaaggtggtggacgagctcgtgaaagtgatgggccggcacaagcccgagaacatcgtgatcgaaatggccagagagaaccagaccacccagaagggacagaagaacagccgcgagagaatgaagcggatcgaagagggcatcaaagagctgggcagccagatcctgaaagaacaccccgtggaaaacacccagctgcagaacgagaagctgtacctgtactacctgcagaatgggcgggatatgtacgtggaccaggaactggacatcaaccggctgtccgactacgatgtggacgctatcgtgcctcagagctttctgaaggacgactccatcgacaacaaggtgctgaccagaagcgacaagaaccggggcaagagcgacaacgtgccctccgaagaggtcgtgaagaagatgaagaactactggcggcagctgctgaacgccaagctgattacccagagaaagttcgacaatctgaccaaggccgagagaggcggcctgagcgaactggataaggccggcttcatcaagagacagctggtggaaacccggcagatcacaaagcacgtggcacagatcctggactcccggatgaacactaagtacgacgagaatgacaagctgatccgggaagtgaaagtgatcaccctgaagtccaagctggtgtccgatttccggaaggatttccagttttacaaagtgcgcgagatcaacaactaccaccacgcccacgacgcctacctgaacgccgtcgtgggaaccgccctgatcaaaaagtaccctaagctggaaagcgagttcgtgtacggcgactacaaggtgtacgacgtgcggaagatgatcgccaagagcgagcaggaaatcggcaaggctaccgccaagtacttcttctacagcaacatcatgaactttttcaagaccgagattaccctggccaacggcgagatccggaagcggcctctgatcgagacaaacggcgaaaccggggagatcgtgtgggataagggccgggattttgccaccgtgcggaaagtgctgagcatgccccaagtgaatatcgtgaaaaagaccgaggtgcagacaggcggcttcagcaaagagtctatcctgcccaagaggaacagcgataagctgatcgccagaaagaaggactgggaccctaagaagtacggcggcttcgacagccccaccgtggcctattctgtgctggtggtggccaaagtggaaaagggcaagtccaagaaactgaagagtgtgaaagagctgctggggatcaccatcatggaaagaagcagcttcgagaagaatcccatcgactttctggaagccaagggctacaaagaagtgaaaaaggacctgatcatcaagctgcctaagtactccctgttcgagctggaaaacggccggaagagaatgctggcctctgccggcgaactgcagaagggaaacgaactggccctgccctccaaatatgtgaacttcctgtacctggccagccactatgagaagctgaagggctcccccgaggataatgagcagaaacagctgtttgtggaacagcacaagcactacctggacgagatcatcgagcagatcagcgagttctccaagagagtgatcctggccgacgctaatctggacaaagtgctgtccgcctacaacaagcaccgggataagcccatcagagagcaggccgagaatatcatccacctgtttaccctgaccaatctgggagcccctgccgccttcaagtactttgacaccaccatcgaccggaagaggtacaccagcaccaaagaggtgctggacgccaccctgatccaccagagcatcaccggcctgtacgagacacggatcgacctgtctcagctgggaggtgactccggcggaagctctggtggcagcaagcggaccgccgacggctctgaattcgagagcggtggttcgccaaagaagaagcggaaggtggagctcagcggaggatcttccggaggatctagcggctccgagacaccaggaacatccgaaagcgctacaccagaatctagcggaggctcttccggaggatctaggcctaccctcaacatcgaggatgagtatcgcctccacgaaacctccaaagaaccggacgtgtccctcggcagcacatggctcagcgacttcccacaagcgtgggccgaaaccggcggcatgggcctcgccgtccgccaagccccactcattatcccgctgaaggcgacctccacaccggtgtccatcaagcagtacccgatgagccaagaggcgaggctcgggattaagccgcacattcagcgcctcctcgatcaaggcattctcgtgccgtgccaatccccgtggaatacaccactcctcccggtcaaaaagccgggcaccaacgactatcgcccggtccaagatctccgcgaggtcaacaagcgcgtggaagatatccacccgaccgtcccgaacccgtataatctgctctccgggctcccaccatcccaccagtggtatacagtgctggacctcaaagacgccttcttctgtctccgcctccacccaacaagccagccgctcttcgccttcgagtggcgcgacccggagatgggcatctccggccaactgacatggacacgcctcccgcaaggcttcaagaacagcccgacactcttcaacgaggcgctccatagggacctcgcggattttcgcatccagcatccggacctcatcctcctccagtatgtggatgatctcctcctcgccgcgacctccgagctggattgtcaacaaggcacacgcgcgctcctccaaacactcgggaacctcggctatcgcgcgtccgcgaaaaaggcccaaatctgccagaagcaagtgaagtacctcgggtatctgctcaaggaaggccaacgctggctcaccgaagcgcgcaaagaaacagtgatggggcaaccgacaccgaaaacaccacgccagctgcgcgagtttctcggcaaagccggcttctgtcgcctcttcatcccgggctttgccgagatggccgcgccactctacccactcaccaagccgggcacactgtttaactgggggccggatcagcagaaagcctaccaagagatcaaacaagcgctcctcaccgccccagcgctcgggctcccagatctcacaaagccgttcgagctgttcgtcgatgagaagcaaggctacgcgaagggcgtgctcacacagaagctcggcccgtggaggaggccagtggcctatctctccaaaaaactcgatccagtggccgccggctggccaccgtgtctgcgcatggtcgccgcgattgccgtgctcacaaaggatgccggcaaactcacaatgggccagccgctggtgatcctcgcgccacatgccgtggaagccctcgtcaaacagccgccggataggtggctctccaatgcgcgcatgacccattaccaagcgctcctcctcgacaccgatcgcgtccagttcggcccagtggtcgccctcaatccggcgacactgctgccactcccagaggagggcctccaacacaactgtctggatattctcgcggaagcgcatggcacaaggccagacctcacagatcaaccgctcagcggcggcagcccgaagaagaaaaggaaggtgtga

SEQ ID NO: 6 - DNA, 6099 bp, synthetic construct
  source 1..6099: mol_type = other DNA
atgaaacggacagccgacggaagcgagttcgagtcaccaaagaagaagcggaaagtcgacaagaagtacagcatcggcctggacatcggcaccaactctgtgggctgggccgtgatcaccgacgagtacaaggtgcccagcaagaaattcaaggtgctgggcaacaccgaccggcacagcatcaagaagaacctgatcggagccctgctgttcgacagcggcgaaacagccgaggccacccggctgaagagaaccgccagaagaagatacaccagacggaagaaccggatctgctatctgcaagagatcttcagcaacgagatggccaaggtggacgacagcttcttccacagactggaagagtccttcctggtggaagaggataagaagcacgagcggcaccccatcttcggcaacatcgtggacgaggtggcctaccacgagaagtaccccaccatctaccacctgagaaagaaactggtggacagcaccgacaaggccgacctgcggctgatctatctggccctggcccacatgatcaagttccggggccacttcctgatcgagggcgacctgaaccccgacaacagcgacgtggacaagctgttcatccagctggtgcagacctacaaccagctgttcgaggaaaaccccatcaacgccagcggcgtggacgccaaggccatcctgtctgccagactgagcaagagcagaaagctggaaaatctgatcgcccagctgcccggcgagaagaagaatggcctgttcggaaacctgattgccctgagcctgggcctgacccccaacttcaagagcaacttcgacctggccgaggatgccaaactgcagctgagcaaggacacctacgacgacgacctggacaacctgctggcccagatcggcgaccagtacgccgacctgtttctggccgccaagaacctgtccgacgccatcctgctgagcgacatcctgagagtgaacaccgagatcaccaaggcccccctgagcgcctctatgatcaagagatacgacgagcaccaccaggacctgaccctgctgaaagctctcgtgcggcagcagctgcctgagaagtacaaagagattttcttcgaccagagcaagaacggctacgccggctacattgacggcggagccagccaggaagagttctacaagttcatcaagcccatcctggaaaagatggacggcaccgaggaactgctcgtgaagctgaagagagaggacctgctgcggaagcagcggaccttcgacaacggcagcatcccccaccagatccacctgggagagctgcacgccattctgcggcggcaggaagatttttacccattcctgaaggacaaccgggaaaagatcgagaagatcctgaccttccgcatcccctactacgtgggccctctggccaggggaaacagcagattcgcctggatgaccagaaagagcgaggaaaccatcaccccctggaacttcgaggaagtggtggacaagggcgcttccgcccagagcttcatcgagcggatgaccaacttcgataagaacctgcccaacgagaaggtgctgcccaagcacagcctgctgtacgagtacttcaccgtgtataacgagctgaccaaagtgaaatacgtgaccgagggaatgagaaagcccgccttcctgagcggcgagcagaaaaaggccatcgtggacctgctgttcaagaccaaccggaaagtgaccgtgaagcagctgaaagaggactacttcaagaaaatcgagtgcttcgactccgtggaaatctccggcgtggaagatcggttcaacgcctccctgggcacataccacgatctgctgaaaattatcaaggacaaggacttcctggacaatgaggaaaacgaggacattctggaagatatcgtgctgaccctgacactgtttgaggacagagagatgatcgaggaacggctgaaaacctatgcccacctgttcgacgacaaagtgatgaagcagctgaagcggcggagatacaccggctggggcaggctgagccggaagctgatcaacggcatccgggacaagcagtccggcaagacaatcctggatttcctgaagtccgacggcttcgccaacagaaacttcatgcagctgatccacgacgacagcctgacctttaaagaggacatccagaaagcccaggtgtccggccagggcgatagcctgcacgagcacattgccaatctggccggcagccccgccattaagaagggcatcctgcagacagtgaaggtggtggacgagctcgtgaaagtgatgggccggcacaagcccgagaacatcgtgatcgaaatggccagagagaaccagaccacccagaagggacagaagaacagccgcgagagaatgaagcggatcgaagagggcatcaaagagctgggcagccagatcctgaaagaacaccccgtggaaaacacccagctgcagaacgagaagctgtacctgtactacctgcagaatgggcgggatatgtacgtggaccaggaactggacatcaaccggctgtccgactacgatgtggacgctatcgtgcctcagagctttctgaaggacgactccatcgacaacaaggtgctgaccagaagcgacaagaaccggggcaagagcgacaacgtgccctccgaagaggtcgtgaagaagatgaagaactactggcggcagctgctgaacgccaagctgattacccagagaaagttcgacaatctgaccaaggccgagagaggcggcctgagcgaactggataaggccggcttcatcaagagacagctggtggaaacccggcagatcacaaagcacgtggcacagatcctggactcccggatgaacactaagtacgacgagaatgacaagctgatccgggaagtgaaagtgatcaccctgaagtccaagctggtgtccgatttccggaaggatttccagttttacaaagtgcgcgagatcaacaactaccaccacgcccacgacgcctacctgaacgccgtcgtgggaaccgccctgatcaaaaagtaccctaagctggaaagcgagttcgtgtacggcgactacaaggtgtacgacgtgcggaagatgatcgccaagagcgagcaggaaatcggcaaggctaccgccaagtacttcttctacagcaacatcatgaactttttcaagaccgagattaccctggccaacggcgagatccggaagcggcctctgatcgagacaaacggcgaaaccggggagatcgtgtgggataagggccgggattttgccaccgtgcggaaagtgctgagcatgccccaagtgaatatcgtgaaaaagaccgaggtgcagacaggcggcttcagcaaagagtctatcctgcccaagaggaacagcgataagctgatcgccagaaagaaggactgggaccctaagaagtacggcggcttcgacagccccaccgtggcctattctgtgctggtggtggccaaagtggaaaagggcaagtccaagaaactgaagagtgtgaaagagctgctggggatcaccatcatggaaagaagcagcttcgagaagaatcccatcgactttctggaagccaagggctacaaagaagtgaaaaaggacctgatcatcaagctgcctaagtactccctgttcgagctggaaaacggccggaagagaatgctggcctctgccggcgaactgcagaagggaaacgaactggccctgccctccaaatatgtgaacttcctgtacctggccagccactatgagaagctgaagggctcccccgaggataatgagcagaaacagctgtttgtggaacagcacaagcactacctggacgagatcatcgagcagatcagcgagttctccaagagagtgatcctggccgacgctaatctggacaaagtgctgtccgcctacaacaagcaccgggataagcccatcagagagcaggccgagaatatcatccacctgtttaccctgaccaatctgggagcccctgccgccttcaagtactttgacaccaccatcgaccggaagaggtacaccagcaccaaagaggtgctggacgccaccctgatccaccagagcatcaccggcctgtacgagacacggatcgacctgtctcagctgggaggtgactccggcggaagctctggtggcagcaagcggaccgccgacggctctgaattcgagagcggtggttcggccacagtggtgtccggccaaaagcaggaccgccagggcggagaacgcagaaggtcccagctcgatagggatcagtgtgcctactgcaaggagaagggccactgggccaaagactgcccgaaaaagccgcgcggcccacgcggcccaaggccacaaacatccctccttccaaagaagaagcggaaggtggagctcagcggaggatcttccggaggatctagcggctccgagacaccaggaacatccgaaagcgctacaccagaatctagcggaggctcttccggaggatctaggcctaccctcaacatcgaggatgagtatcgcctccacgaaacctccaaagaaccggacgtgtccctcggcagcacatggctcagcgacttcccacaagcgtgggccgaaaccggcggcatgggcctcgccgtccgccaagccccactcattatcccgctgaaggcgacctccacaccggtgtccatcaagcagtacccgatgagccaagaggcgaggctcgggattaagccgcacattcagcgcctcctcgatcaaggcattctcgtgccgtgccaatccccgtggaatacaccactcctcccggtcaaaaagccgggcaccaacgactatcgcccggtccaagatctccgcgaggtcaacaagcgcgtggaagatatccacccgaccgtcccgaacccgtataatctgctctccgggctcccaccatcccaccagtggtatacagtgctggacctcaaagacgccttcttctgtctccgcctccacccaacaagccagccgctcttcgccttcgagtggcgcgacccggagatgggcatctccggccaactgacatggacacgcctcccgcaaggcttcaagaacagcccgacactcttcaacgaggcgctccatagggacctcgcggattttcgcatccagcatccggacctcatcctcctccagtatgtggatgatctcctcctcgccgcgacctccgagctggattgtcaacaaggcacacgcgcgctcctccaaacactcgggaacctcggctatcgcgcgtccgcgaaaaaggcccaaatctgccagaagcaagtgaagtacctcgggtatctgctcaaggaaggccaacgctggctcaccgaagcgcgcaaagaaacagtgatggggcaaccgacaccgaaaacaccacgccagctgcgcgagtttctcggcaaagccggcttctgtcgcctcttcatcccgggctttgccgagatggccgcgccactctacccactcaccaagccgggcacactgtttaactgggggccggatcagcagaaagcctaccaagagatcaaacaagcgctcctcaccgccccagcgctcgggctcccagatctcacaaagccgttcgagctgttcgtcgatgagaagcaaggctacgcgaagggcgtgctcacacagaagctcggcccgtggaggaggccagtggcctatctctccaaaaaactcgatccagtggccgccggctggccaccgtgtctgcgcatggtcgccgcgattgccgtgctcacaaaggatgccggcaaactcacaatgggccagccgctggtgatcctcgcgccacatgccgtggaagccctcgtcaaacagccgccggataggtggctctccaatgcgcgcatgacccattaccaagcgctcctcctcgacaccgatcgcgtccagttcggcccagtggtcgccctcaatccggcgacactgctgccactcccagaggagggcctccaacacaactgtctggatattctcgcggaagcgcatggcacaaggccagacctcacagatcaaccgctcagcggcggcagcccgaagaagaaaaggaaggtgtga

SEQ ID NO: 7 - DNA, 346 bp, synthetic construct
  source 1..346: mol_type = other DNA
tgagacttttcaacaaaggataatttcgggaaacctcctcggattccattgcccagctatctgtcacttcatcgaaaggacagtagaaaaggaaggtggctcctacaaatgccatcattgcgataaaggaaaggctatcattcaagatctctctgccgacagtggtcccaaagatggacccccacccacgaggagcatcgtggaaaaagaagaggttccaaccacgtctacaaagcaagtggattgatgtgacatctccactgacgtaagggatgacgcacaatcccactatccttcgcaagacccttcctctatataaggaagttcatttcatttggagaggaca

SEQ ID NO: 8 - DNA, 88 bp, synthetic construct
  source 1..88: mol_type = other DNA
aagttgaaaacaatcttcaaaagtcccacatcgcttagataagaaaacgaagctgagtttatatacagctagagtcgaagtagtgatt

SEQ ID NO: 9 - DNA, 993 bp, synthetic construct
  source 1..993: mol_type = other DNA
atggagtcaaagattcaaatagaggacctaacagaactcgccgtaaagactggcgaacagttcatacagagtctcttacgactcaatgacaagaagaaaatcttcgtcaacatggtggagcacgacacacttgtctactccaaaaatatcaaagatacagtctcagaagatcaaagggcaattgagacttttcaacaaagggtaatatccggaaacctcctcggattccattgcccagctatctgtcactttattgtgaagatagtggaaaaggaaggtggctcctacaaatgccatcattgcgataaaggaaaggccatcgttgaagatgcctctgccgacagtggtcccaaagatggacccccacccacgaggagcatcgtggaaaaagaagatgttccaaccacatcttcaaagcaagtggattgatgtgattggcagacatactgtcccacaaatgaagatggaatctgtaaaagaaaacgcgtgaaataatgcgtctgacaaaggttaggtcggctgcctttaatcaataccaaagtggtccctaccacgatggaaaaactgtgcagtcggtttggctttttctgacgaacaaataagattcgtggccgacaggtgggggtccaccatgtgaaggcatcttcagactccaataatggagcaatgacgtaagggcttacgaaataagtaagggtagtttgggaaatgtccactcacccgtcagtctataaatacttagcccctccctcattgttaagggagcaaaatctcagagagatagtcctagagagagaaagagagcaagtagcctagaagtagtcaaggcggcgaagtattcaggcacgtggccaggaagaagaaaagccaagacgacgaaaacaggtaagagctaagcatctagaaagttgaaaacaatcttcaaaagtcccacatcgcttagataagaaaacgaagctgagtttatatacagctagagtcgaagtagtgatt

SEQ ID NO: 10 - DNA, 943 bp, synthetic construct
  source 1..943: mol_type = other DNA
aaagcagaatgctgagctaaaagaaaggctttttccattttcgagagacaatgagaaaagaagaagaagaagaagaagaagaagaagaagaaaagagtaaataataaagccccacaggaggcgaagttcttgtagctccatgttatctaagttattgatattgtttgccctatattttatttctgtcattgtgtatgttttgttcagtttcgatctccttgcaaaatgcagagattatgagatgaataaactaagttatattattatacgtgttaatattctcctcctctctctagctagccttttgttttctctttttcttatttgattttctttaaatcaatccattttaggagagggccagggagtgatccagcaaaacatgaagattagaagaaacttccctcttttttttcctgaaaacaatttaacgtcgagatttatctctttttgtaatggaatcatttctacagttatgacaccaactcggtccatttgcacccctaatcataatagctttaatatttcaagatattattaagttaacgttgtcaatatcctggaaattttgcaaaatgaatcaagcctatatggctgtaatatgaatttaaaagcagctcgatgtggtggtaatatgtaatttacttgattctaaaaaaatatcccaagtattaataatttctgctaggaagaaggttagctacgatttacagcaaagccagaatacaaagaaccataaagtgattgaagctcgaaatatacgaaggaacaaatatttttaaaaaaatacgcaatgacttggaacaaaagaaagtgatatattttttgttcttaaacaagcatcccctctaaagaatggcagttttcctttgcatgtaactattatgctcccttcgttacaaaaattttggactactattgggaacttcttctgaaaatagtg

SEQ ID NO: 11 - DNA, 1154 bp, synthetic construct
  source 1..1154: mol_type = other DNA
aaagcagaatgctgagctaaaagaaaggctttttccattttcgagagacaatgagaaaagaagaagaagaagaagaagaagaagaagaagaaaagagtaaataataaagccccacaggaggcgaagttcttgtagctccatgttatctaagttattgatattgtttgccctatattttatttctgtcattgtgtatgttttgttcagtttcgatctccttgcaaaatgcagagattatgagatgaataaactaagttatattattatacgtgttaatattctcctcctctctctagctagccttttgttttctctttttcttatttgattttctttaaatcaatccattttaggagagggccagggagtgatccagcaaaacatgaagattagaagaaacttccctcttttttttcctgaaaacaatttaacgtcgagatttatctctttttgtaatggaatcatttctacagttatgacgtccgcaaaaatcaccagtctctctctacaaatctatctctctctatttttctccagaataatgtgtgagtagttcccagataagggaattagggttcttatagggtttcgctcatgtgttgagcatataagaaacccttagtatgtatttgtatttgtaaaatacttctatcaataaaatttctaattcctaaaaccaaaatccagtgacaccaactcggtccatttgcacccctaatcataatagctttaatatttcaagatattattaagttaacgttgtcaatatcctggaaattttgcaaaatgaatcaagcctatatggctgtaatatgaatttaaaagcagctcgatgtggtggtaatatgtaatttacttgattctaaaaaaatatcccaagtattaataatttctgctaggaagaaggttagctacgatttacagcaaagccagaatacaaagaaccataaagtgattgaagctcgaaatatacgaaggaacaaatatttttaaaaaaatacgcaatgacttggaacaaaagaaagtgatatattttttgttcttaaacaagcatcccctctaaagaatggcagttttcctttgcatgtaactattatgctcccttcgttacaaaaattttggactactattgggaacttcttctgaaaatagtg

SEQ ID NO: 12 - DNA, 20 bp, synthetic construct
  source 1..20: mol_type = other DNA
ctattacaggtcaagtgcca

SEQ ID NO: 13 - DNA, 20 bp, synthetic construct
  source 1..20: mol_type = other DNA
tcagtaccaatcatcctcct

SEQ ID NO: 14 - DNA, 20 bp, synthetic construct
  source 1..20: mol_type = other DNA
gagataatattagaagtagg

SEQ ID NO: 15 - DNA, 20 bp, synthetic construct
  source 1..20: mol_type = other DNA
aaaagaagcgttacaggcca

SEQ ID NO: 16 - DNA, 20 bp, synthetic construct
  source 1..20: mol_type = other DNA
tctcgaagtgccactgtccc

SEQ ID NO: 17 - DNA, 20 bp, synthetic construct
  source 1..20: mol_type = other DNA
attgtgcaagaaacttagtg

SEQ ID NO: 18 - DNA, 20 bp, synthetic construct
  source 1..20: mol_type = other DNA
atcatcatgttttcatttgt

SEQ ID NO: 19 - DNA, 20 bp, synthetic construct
  source 1..20: mol_type = other DNA
caactattccttggaaatgc

SEQ ID NO: 20 - DNA, 20 bp, synthetic construct
  source 1..20: mol_type = other DNA
acagtaactgctgctgtcaa

SEQ ID NO: 21 - DNA, 20 bp, synthetic construct
  source 1..20: mol_type = other DNA
cttgaagcaatctttaattc

SEQ ID NO: 22 - DNA, 20 bp, synthetic construct
  source 1..20: mol_type = other DNA
agctccttcaacgttctcaa

SEQ ID NO: 23 - DNA, 20 bp, synthetic construct
  source 1..20: mol_type = other DNA
tagagaagtatgctcctgaa

SEQ ID NO: 24 - DNA, 20 bp, synthetic construct
  source 1..20: mol_type = other DNA
gttccaccggaagtaaaaac

SEQ ID NO: 25 - DNA, 20 bp, synthetic construct
  source 1..20: mol_type = other DNA
agaaaaaccagatgctggaa

SEQ ID NO: 26 - DNA, 26 bp, synthetic construct
  source 1..26: mol_type = other DNA
caatcatcctcctagacacttgacct

SEQ ID NO: 27 - DNA, 34 bp, synthetic construct
  source 1..34: mol_type = other DNA
gtgctacaggtcaagtgtctaggaggatgattgg

SEQ ID NO: 28 - DNA, 31 bp, synthetic construct
  source 1..31: mol_type = other DNA
aatatcttgttcctatgacttctaatattat

SEQ ID NO: 29 - DNA, 29 bp, synthetic construct
  source 1..29: mol_type = other DNA
gaagtgccactgtttcaggcctgtaacgc

SEQ ID NO: 30 - DNA, 25 bp, synthetic construct
  source 1..25: mol_type = other DNA
tcgaagtgccactggcctgtaacgc

SEQ ID NO: 31 - DNA, 25 bp, synthetic construct
  source 1..25: mol_type = other DNA
gcgttacaggcctgaaacagtggca

SEQ ID NO: 32 - DNA, 38 bp, synthetic construct
  source 1..38: mol_type = other DNA
aattaattggacctcacaattttcactaagtttcttgc

SEQ ID NO: 33 - DNA, 47 bp, synthetic construct
  source 1..47: mol_type = other DNA
tatcaacttttgcagactgtggtttcttacctacaaatgaaaacatg

SEQ ID NO: 34 - DNA, 45 bp, synthetic construct
  source 1..45: mol_type = other DNA
tgctgctgtcaaagaacgcattgcgattcctgcatttccaaggaa

SEQ ID NO: 35 - DNA, 38 bp, synthetic construct
  source 1..38: mol_type = other DNA
gaaatgcaggaatcgcaatgcgttctttgacagcagca

SEQ ID NO: 36 - DNA, 32 bp, synthetic construct
  source 1..32: mol_type = other DNA
gtggattcaccatatcagaattaaagattgct

SEQ ID NO: 37 - DNA, 31 bp, synthetic construct
  source 1..31: mol_type = other DNA
tcactaatatcttacatctaagaacgttgaa

SEQ ID NO: 38 - DNA, 24 bp, synthetic construct
  source 1..24: mol_type = other DNA
aagatgatggattaaggagcatac

SEQ ID NO: 39 - DNA, 28 bp, synthetic construct
  source 1..28: mol_type = other DNA
ggaaccgacaaaccagattttacttccg

SEQ ID NO: 40 - DNA, 42 bp, synthetic construct
  source 1..42: mol_type = other DNA
tttataacccaaaactaaaagctcatccataccagcatctgg

SEQ ID NO: 41 - DNA, 37 bp, synthetic construct
  source 1..37: mol_type = other DNA
cagtcgaagacaaaatgaaacggacagccgacggaag

SEQ ID NO: 42 - DNA, 38 bp, synthetic construct
  source 1..38: mol_type = other DNA
catacgaagacaaatcttcaatgttcagggtgcttccg

SEQ ID NO: 43 - DNA, 41 bp, synthetic construct
  source 1..41: mol_type = other DNA
cagtcgaagacaaagatgagtatagactgcatgaaacaagc

SEQ ID NO: 44 - DNA, 43 bp, synthetic construct
  source 1..43: mol_type = other DNA
catacgaagacaaaagcttagtccagcttcactctcttagcgg

SEQ ID NO: 45 - DNA, 37 bp, synthetic construct; identical to SEQ ID NO: 41
  source 1..37: mol_type = other DNA

SEQ ID NO: 46 - DNA, 38 bp, synthetic construct; identical to SEQ ID NO: 42
  source 1..38: mol_type = other DNA

SEQ ID NO: 47 - DNA, 41 bp, synthetic construct; identical to SEQ ID NO: 43
  source 1..41: mol_type = other DNA

SEQ ID NO: 48 - DNA, 34 bp, synthetic construct
  source 1..34: mol_type = other DNA
catacgaagacaatttggatcacctcgccggcgg

SEQ ID NO: 49 - DNA, 39 bp, synthetic construct
  source 1..39: mol_type = other DNA
cagtcgaagacaacaaagacctgccaatgcaataaagga

SEQ ID NO: 50 - DNA, 72 bp, synthetic construct
  source 1..72: mol_type = other DNA
catacgaagacaaaagcttacaccttccttttcttcttcgggctgccgaaaaccttataaaggtcgggcagg

SEQ ID NO: 51 - DNA, 37 bp, synthetic construct; identical to SEQ ID NO: 41
  source 1..37: mol_type = other DNA

SEQ ID NO: 52 - DNA, 45 bp, synthetic construct
  source 1..45: mol_type = other DNA
catacgaagacaacgaaccaccgctctcgaattcagagccgtcgg

SEQ ID NO: 53 - DNA, 62 bp, synthetic construct
  source 1..62: mol_type = other DNA
cagtcgaagacaaaatgcctaagaaaaagagaaaagtggacaagaagtactcgatcggcctc

SEQ ID NO: 54 - DNA, 36 bp, synthetic construct
  source 1..36: mol_type = other DNA
cagtcgaagacaatcacttgtggcatggagagaacc

SEQ ID NO: 55 - DNA, 39 bp, synthetic construct
  source 1..39: mol_type = other DNA
cagtcgaagacaagtgaatatcgtcaaaaagacagaggt

SEQ ID NO: 56 - DNA, 34 bp, synthetic construct
  source 1..34: mol_type = other DNA
cagtcgaagacaatatcttccacgcgcttgttga

SEQ ID NO: 57 - DNA, 33 bp, synthetic construct
  source 1..33: mol_type = other DNA
cagtcgaagacaagatatccacccgaccgtccc

SEQ ID NO: 58 - DNA, 57 bp, synthetic construct
  source 1..57: mol_type = other DNA
cagtcgaagacaaaagctcacaccttccttttcttcttcgggctgccgccgctgagc

SEQ ID NO: 59 - DNA, 62 bp, synthetic construct; identical to SEQ ID NO: 53
  source 1..62: mol_type = other DNA

SEQ ID NO: 60 - DNA, 36 bp, synthetic construct; identical to SEQ ID NO: 54
  source 1..36: mol_type = other DNA

SEQ ID NO: 61 - DNA, 39 bp, synthetic construct; identical to SEQ ID NO: 55
  source 1..39: mol_type = other DNA

SEQ ID NO: 62 - DNA, 42 bp, synthetic construct
  source 1..42: mol_type = other DNA
catacgaagacaacgaaccaaggagggatgtttgtggccttg

SEQ ID NO: 63 - DNA, 53 bp, synthetic construct
  source 1..53: mol_type = other DNA
cagtcgaagacaattcgccaaagaagaagcggaaggtggagctcagcggagga

SEQ ID NO: 64 - DNA, 34 bp, synthetic construct; identical to SEQ ID NO: 56
  source 1..34: mol_type = other DNA

SEQ ID NO: 65 - DNA, 33 bp, synthetic construct; identical to SEQ ID NO: 57
  source 1..33: mol_type = other DNA

SEQ ID NO: 66 - DNA, 57 bp, synthetic construct; identical to SEQ ID NO: 58
  source 1..57: mol_type = other DNA

SEQ ID NO: 67 - DNA, 38 bp, synthetic construct
  source 1..38: mol_type = other DNA
cagtcgaagacaattcggccacagtggtgtccggccaa

SEQ ID NO: 68 - DNA, 34 bp, synthetic construct; identical to SEQ ID NO: 56
  source 1..34: mol_type = other DNA

SEQ ID NO: 69 - DNA, 33 bp, synthetic construct; identical to SEQ ID NO: 57
  source 1..33: mol_type = other DNA

SEQ ID NO: 70 - DNA, 57 bp, synthetic construct; identical to SEQ ID NO: 58
  source 1..57: mol_type = other DNA

SEQ ID NO: 71 - DNA, 37 bp, synthetic construct; identical to SEQ ID NO: 41
  source 1..37: mol_type = other DNA

SEQ ID NO: 72 - DNA, 40 bp, synthetic construct
  source 1..40: mol_type = other DNA
catacgaagacaatggcgtccagcttcactctcttagcgg

SEQ ID NO: 73 - DNA, 34 bp, synthetic construct
  source 1..34: mol_type = other DNA
cagtcgaagacaagccacagtggtgtccggccaa

SEQ ID NO: 74 - DNA, 43 bp, synthetic construct
  source 1..43: mol_type = other DNA
catacgaagacaaaagcttaaaggagggatgtttgtggccttg

SEQ ID NO: 75 - DNA, 37 bp, synthetic construct; identical to SEQ ID NO: 41
  source 1..37: mol_type = other DNA

SEQ ID NO: 76 - DNA, 39 bp, synthetic construct
  source 1..39: mol_type = other DNA
catacgaagacaatggcgctctcgaattcagagccgtcg

SEQ ID NO: 77 - DNA, 34 bp, synthetic construct; identical to SEQ ID NO: 73
  source 1..34: mol_type = other DNA

SEQ ID NO: 78 - DNA, 33 bp, synthetic construct
  source 1..33: mol_type = other DNA
cagtcgaagacaaagggtaggcctagatcctcc

SEQ ID NO: 79 - DNA, 38 bp, synthetic construct
  source 1..38: mol_type = other DNA
cagtcgaagacaaccctgaacattgaagatgagtatag

SEQ ID NO: 80 - DNA, 37 bp, synthetic construct
  source 1..37: mol_type = other DNA
catacgaagacaacagacaggggctgatcggtcaggt

SEQ ID NO: 81 - DNA, 35 bp, synthetic construct
  source 1..35: mol_type = other DNA
cagtcgaagacaatctggcggctcaaaaagaaccg

SEQ ID NO: 82 - DNA, 43 bp, synthetic construct; identical to SEQ ID NO: 44
  source 1..43: mol_type = other DNA

SEQ ID NO: 83 - DNA, 43 bp, synthetic construct
  source 1..43: mol_type = other DNA
cagtcgaagacaaggaggattagtttgtcaaatagtagagttc

SEQ ID NO: 84 - DNA, 39 bp, synthetic construct
  source 1..39: mol_type = other DNA
catacgaagacaagaactctaaattaatttttactcttt

SEQ ID NO: 85 - DNA, 39 bp, synthetic construct
  source 1..39: mol_type = other DNA
cagtcgaagacaagttctactgccttcaaatttctattt

SEQ ID NO: 86 - DNA, 39 bp, synthetic construct
  source 1..39: mol_type = other DNA
catacgaagacaaatcatctagtaaaacaactgaaaaac

SEQ ID NO: 87 - DNA, 39 bp, synthetic construct
  source 1..39: mol_type = other DNA
cagtcgaagacaatgattttcactgtctccttgttagat

SEQ ID NO: 88 - DNA, 40 bp, synthetic construct
  source 1..40: mol_type = other DNA
catacgaagacaacattcttgagacactaagaaactgcat

SEQ ID NO: 89 - DNA, 37 bp, synthetic construct
  source 1..37: mol_type = other DNA
cagtcgaagacaatgcactattacaggtcaagtgcca

SEQ ID NO: 90 - DNA, 37 bp, synthetic construct
  source 1..37: mol_type = other DNA
cagtcgaagacaaaaactggcacttgacctgtaatag

SEQ ID NO: 91 - DNA, 62 bp, synthetic construct
  source 1..62: mol_type = other DNA
cagtcgaagacaatgcacctaacccataggcgtttccgtttaagagctatgctggaaacagc

SEQ ID NO: 92 - DNA, 37 bp, synthetic construct
  source 1..37: mol_type = other DNA
cagtcgaagacaacgcggcaccgactcggtgcgactt

SEQ ID NO: 93 - DNA, 40 bp, synthetic construct
  source 1..40: mol_type = other DNA
cagtcgaagacaagtgccaatcatcctcctagacacttga

SEQ ID NO: 94 - DNA, 40 bp, synthetic construct
  source 1..40: mol_type = other DNA
cagtcgaagacaacgcgaggtcaagtgtctaggaggatga

SEQ ID NO: 95 - DNA, 44 bp, synthetic construct
  source 1..44: mol_type = other DNA
cagtcggtctcaggagaagttgaaaacaatcttcaaaagtccca

SEQ ID NO: 96 - DNA, 41 bp, synthetic construct
  source 1..41: mol_type = other DNA
cagtcggtctcaagcgaaaaaaaagtcccattcgccatgcc

SEQ ID NO: 97 - DNA, 37 bp, synthetic construct
  source 1..37: mol_type = other DNA
cagtcgaagacaatgcagagataatattagaagtagg

SEQ ID NO: 98 - DNA, 37 bp, synthetic construct
  source 1..37: mol_type = other DNA
cagtcgaagacaaaaaccctacttctaatattatctc

SEQ ID NO: 99 - DNA, 45 bp, synthetic construct
  source 1..45: mol_type = other DNA
cagtcgaagacaagtgcaatatcttgttcctatgacttctaatat

SEQ ID NO: 100 - DNA, 45 bp, synthetic construct
  source 1..45: mol_type = other DNA
cagtcgaagacaacgcgataatattagaagtcataggaacaagat

SEQ ID NO: 101 - DNA, 37 bp, synthetic construct
  source 1..37: mol_type = other DNA
cagtcgaagacaatgcaaaaagaagcgttacaggcca

SEQ ID NO: 102 - DNA, 37 bp, synthetic construct
  source 1..37: mol_type = other DNA
cagtcgaagacaaaaactggcctgtaacgcttctttt

SEQ ID NO: 103 - DNA, 42 bp, synthetic construct
  source 1..42: mol_type = other DNA
cagtcgaagacaagtgcgaagtgccactgtttcaggcctgta

SEQ ID NO: 104 - DNA, 42 bp, synthetic construct
  source 1..42: mol_type = other DNA
cagtcgaagacaacgcggcgttacaggcctgaaacagtggca

SEQ ID NO: 105 - DNA, 40 bp, synthetic construct
  source 1..40: mol_type = other DNA
cagtcgaagacaagtgctcgaagtgccactggcctgtaac

SEQ ID NO: 106 - DNA, 40 bp, synthetic construct
  source 1..40: mol_type = other DNA
cagtcgaagacaacgcggcgttacaggccagtggcacttc

SEQ ID NO: 107 - DNA, 37 bp, synthetic construct
  source 1..37: mol_type = other DNA
cagtcgaagacaatgcaattgtgcaagaaacttagtg

SEQ ID NO: 108 - DNA, 37 bp, synthetic construct
  source 1..37: mol_type = other DNA
cagtcgaagacaaaaaccactaagtttcttgcacaat

SEQ ID NO: 109 - DNA, 48 bp, synthetic construct
  source 1..48: mol_type = other DNA
cagtcgaagacaagtgcaattaattggacctcacaattttcactaagt

SEQ ID NO: 110 - DNA, 48 bp, synthetic construct
  source 1..48: mol_type = other DNA
cagtcgaagacaacgcggcaagaaacttagtgaaaattgtgaggtcca

SEQ ID NO: 111 - DNA, 37 bp, synthetic construct
  source 1..37: mol_type = other DNA
cagtcgaagacaatgcaatcatcatgttttcatttgt

SEQ ID NO: 112 - DNA, 37 bp, synthetic construct
  source 1..37: mol_type = other DNA
cagtcgaagacaaaaacacaaatgaaaacatgatgat

SEQ ID NO: 113 - DNA, 51 bp, synthetic construct
  source 1..51: mol_type = other DNA
cagtcgaagacaagtgctatcaacttttgcagactgtggtttcttacctac

SEQ ID NO: 114 - DNA, 51 bp, synthetic construct
  source 1..51: mol_type = other DNA
cagtcgaagacaacgcgcatgttttcatttgtaggtaagaaaccacagtct

SEQ ID NO: 115 - DNA, 37 bp, synthetic construct
  source 1..37: mol_type = other DNA
cagtcgaagacaatgcacaactattccttggaaatgc

SEQ ID NO: 116 - DNA, 37 bp, synthetic construct
  source 1..37: mol_type = other DNA
cagtcgaagacaaaaacgcatttccaaggaatagttg

SEQ ID NO: 117 - DNA, 50 bp, synthetic construct
  source 1..50: mol_type = other DNA
cagtcgaagacaagtgctgctgctgtcaaagaacgcattgcgattcctgc

SEQ ID NO: 118 - DNA, 50 bp, synthetic construct
  source 1..50: mol_type = other DNA
cagtcgaagacaacgcgttccttggaaatgcaggaatcgcaatgcgttct

SEQ ID NO: 119 - DNA, 37 bp, synthetic construct
  source 1..37: mol_type = other DNA
cagtcgaagacaatgcacttgaagcaatctttaattc

SEQ ID NO: 120 - DNA, 37 bp, synthetic construct
  source 1..37: mol_type = other DNA
cagtcgaagacaaaaacgaattaaagattgcttcaag

SEQ ID NO: 121 - DNA, 45 bp, synthetic construct
  source 1..45: mol_type = other DNA
cagtcgaagacaagtgcgtggattcaccatatcagaattaaagat

SEQ ID NO: 122 - DNA, 45 bp, synthetic construct
  source 1..45: mol_type = other DNA
cagtcgaagacaacgcgagcaatctttaattctgatatggtgaat

SEQ ID NO: 123 - DNA, 37 bp, synthetic construct
  source 1..37: mol_type = other DNA
cagtcgaagacaatgcaagctccttcaacgttctcaa

SEQ ID NO: 124 - DNA, 37 bp, synthetic construct
  source 1..37: mol_type = other DNA
cagtcgaagacaaaaacttgagaacgttgaaggagct

SEQ ID NO: 125 - DNA, 44 bp, synthetic construct
  source 1..44: mol_type = other DNA
cagtcgaagacaagtgctcactaatatcttacatctaagaacgt

SEQ ID NO: 126 - DNA, 45 bp, synthetic construct
  source 1..45: mol_type = other DNA
cagtcgaagacaacgcgttcaacgttcttagatgtaagatattag

SEQ ID NO: 127 - DNA, 37 bp, synthetic construct
  source 1..37: mol_type = other DNA
cagtcgaagacaatgcatagagaagtatgctcctgaa

SEQ ID NO: 128 - DNA, 37 bp, synthetic construct
  source 1..37: mol_type = other DNA
cagtcgaagacaaaaacttcaggagcatacttctcta

SEQ ID NO: 129 - DNA, 41 bp, synthetic construct
  source 1..41: mol_type = other DNA
cagtcgaagacaagtgcaagatgatggattaaggagcatac

SEQ ID NO: 130 - DNA, 40 bp, synthetic construct
  source 1..40: mol_type = other DNA
cagtcgaagacaacgcggtatgctccttaatccatcatct

SEQ ID NO: 131 - DNA, 37 bp, synthetic construct
  source 1..37: mol_type = other DNA
cagtcgaagacaatgcagttccaccggaagtaaaaac

SEQ ID NO: 132 - DNA, 37 bp, synthetic construct
  source 1..37: mol_type = other DNA
cagtcgaagacaaaaacgtttttacttccggtggaac

SEQ ID NO: 133 - DNA, 43 bp, synthetic construct
  source 1..43: mol_type = other DNA
cagtcgaagacaagtgcggaaccgacaaaccagattttacttc

SEQ ID NO: 134 - DNA, 43 bp, synthetic construct
  source 1..43: mol_type = other DNA
cagtcgaagacaacgcgcggaagtaaaatctggtttgtcggtt

SEQ ID NO: 135 - DNA, 37 bp, synthetic construct
  source 1..37: mol_type = other DNA
cagtcgaagacaatgcaagaaaaaccagatgctggaa

SEQ ID NO: 136 - DNA, 37 bp, synthetic construct
  source 1..37: mol_type = other DNA
cagtcgaagacaaaaacttccagcatctggtttttct

SEQ ID NO: 137 - DNA, 50 bp, synthetic construct
  source 1..50: mol_type = other DNA
cagtcgaagacaagtgctttataacccaaaactaaaagctcatccatacc

SEQ ID NO: 138 - DNA, 50 bp, synthetic construct
  source 1..50: mol_type = other DNA
cagtcgaagacaacgcgccagatgctggtatggatgagcttttagttttg

SEQ ID NO: 139 - DNA, 37 bp, synthetic construct
  source 1..37: mol_type = other DNA
cagtcgaagacaatgcatcagtaccaatcatcctcct

SEQ ID NO: 140 - DNA, 37 bp, synthetic construct
  source 1..37: mol_type = other DNA
cagtcgaagacaaaaacaggaggatgattggtactga

SEQ ID NO: 141 - DNA, 42 bp, synthetic construct
  source 1..42: mol_type = other DNA
cagtcgaagacaagtgctacaggtcaagtgtctaggaggatg

SEQ ID NO: 142 - DNA, 43 bp, synthetic construct
  source 1..43: mol_type = other DNA
cagtcgaagacaacgcgccaatcatcctcctagacacttgacc

SEQ ID NO: 143 - DNA, 37 bp, synthetic construct
  source 1..37: mol_type = other DNA
cagtcgaagacaatgcatctcgaagtgccactgtccc

SEQ ID NO: 144 - DNA, 37 bp, synthetic construct
  source 1..37: mol_type = other DNA
cagtcgaagacaaaaacgggacagtggcacttcgaga

SEQ ID NO: 145 - DNA, 42 bp, synthetic construct
  source 1..42: mol_type = other DNA
cagtcgaagacaagtgcgcgttacaggcctgaaacagtggca

SEQ ID NO: 146 - DNA, 42 bp, synthetic construct
  source 1..42: mol_type = other DNA
cagtcgaagacaacgcgtgccactgtttcaggcctgtaacgc

SEQ ID NO: 147 - DNA, 37 bp, synthetic construct
  source 1..37: mol_type = other DNA
cagtcgaagacaatgcaacagtaactgctgctgtcaa

SEQ ID NO: 148 - DNA, 37 bp, synthetic construct
  source 1..37: mol_type = other DNA
cagtcgaagacaaaaacttgacagcagcagttactgt

SEQ ID NO: 149 - DNA, 47 bp, synthetic construct
  source 1..47: mol_type = other DNA
cagtcgaagacaagtgcgaaatgcaggaatcgcaatgcgttctttga

SEQ ID NO: 150 - DNA, 47 bp, synthetic construct
  source 1..47: mol_type = other DNA
cagtcgaagacaacgcgtgctgctgtcaaagaacgcattgcgattcc

SEQ ID NO: 151 - DNA, 37 bp, synthetic construct
  source 1..37: mol_type = other DNA
cagtcgaagacaatgcacatttacgaatagcagaatt

SEQ ID NO: 152 - DNA, 37 bp, synthetic construct
  source 1..37: mol_type = other DNA
cagtcgaagacaaaaacaattctgctattcgtaaatg

SEQ ID NO: 153 - DNA, 44 bp, synthetic construct
  source 1..44: mol_type = other DNA
cagtcgaagacaagtgcgtattgaggctagacagcctaactctg

SEQ ID NO: 154 - DNA, 44 bp, synthetic construct
  source 1..44: mol_type = other DNA
cagtcgaagacaacgcggaatagcagagttaggctgtctagcct

SEQ ID NO: 155 - DNA, 22 bp, synthetic construct
  source 1..22: mol_type = other DNA
cctcaccatctccatgtttctc

SEQ ID NO: 156 - DNA, 22 bp, synthetic construct
  source 1..22: mol_type = other DNA
gtctcagctcctcacttgattg

SEQ ID NO: 157 - DNA, 58 bp, synthetic construct
  source 1..58: mol_type = other DNA
acactctttccctacacgacgctcttccgatctgctacaaatcttgttagtggtcttg

SEQ ID NO: 158 - DNA, 59 bp, synthetic construct
  source 1..59: mol_type = other DNA
gtgactggagttcagacgtgtgctcttccgatctgcttcgtaatagatctcgttacctc

SEQ ID NO: 159 - DNA, 25 bp, synthetic construct
  source 1..25: mol_type = other DNA
atgcgaatcgtagaaatggaattag

SEQ ID NO: 160 - DNA, 22 bp, synthetic construct
  source 1..22: mol_type = other DNA
actcgtttcttcggtccttaat

SEQ ID NO: 161 - DNA, 51 bp, synthetic construct
  source 1..51: mol_type = other DNA
acactctttccctacacgacgctcttccgatctaggacctgagacagtaga

SEQ ID NO: 162 - DNA, 57 bp, synthetic construct
  source 1..57: mol_type = other DNA
gtgactggagttcagacgtgtgctcttccgatctagacatcacagtaataaatacga

SEQ ID NO: 163 - DNA, 23 bp, synthetic construct
  source 1..23: mol_type = other DNA
ccctaatttggtgatgttgtacc

SEQ ID NO: 164 - DNA, 21 bp, synthetic construct
  source 1..21: mol_type = other DNA
cactgatagccctctcacttt

SEQ ID NO: 165 - DNA, 57 bp, synthetic construct
  source 1..57: mol_type = other DNA
acactctttccctacacgacgctcttccgatctctatatgatgggagaatatatgtg

SEQ ID NO: 166 - DNA, 57 bp, synthetic construct
  source 1..57: mol_type = other DNA
gtgactggagttcagacgtgtgctcttccgatctaagtctgatgaaaggagcagctg

SEQ ID NO: 167 - DNA, 21 bp, synthetic construct
  source 1..21: mol_type = other DNA
ctttggtgcgcatgagtctaa

SEQ ID NO: 168 - DNA, 20 bp, synthetic construct
  source 1..20: mol_type = other DNA
acggtcaggtccataccaca

SEQ ID NO: 169 - DNA, 55 bp, synthetic construct
  source 1..55: mol_type = other DNA
acactctttccctacacgacgctcttccgatctaaatggggcccctccagatatt

SEQ ID NO: 170 - DNA, 56 bp, synthetic construct
  source 1..56: mol_type = other DNA
gtgactggagttcagacgtgtgctcttccgatctctaacaactgtggctgagctac

SEQ ID NO: 171 - DNA, 25 bp, synthetic construct
  source 1..25: mol_type = other DNA
acaaagattatgagctagggaatgt

SEQ ID NO: 172 - DNA, 23 bp, synthetic construct
  source 1..23: mol_type = other DNA
ccttcagaattccactccaatga

SEQ ID NO: 173 - DNA, 53 bp, synthetic construct
  source 1..53: mol_type = other DNA
acactctttccctacacgacgctcttccgatctcgccaaacaaatccttgacc

SEQ ID NO: 174 - DNA, 59 bp, synthetic construct
  source 1..59: mol_type = other DNA
gtgactggagttcagacgtgtgctcttccgatcttgagggataagaatgagaagaagac

SEQ ID NO: 175 - DNA, 23 bp, synthetic construct
  source 1..23: mol_type = other DNA
tgagttacttacaaccttgtgct

SEQ ID NO: 176 - DNA, 28 bp, synthetic construct
  source 1..28: mol_type = other DNA
gtaatttatcaccagggcaactattatc

SEQ ID NO: 177 - DNA, 52 bp, synthetic construct
  source 1..52: mol_type = other DNA
acactctttccctacacgacgctcttccgatctggcagtttcctgtcggtaa

SEQ ID NO: 178 - DNA, 55 bp, synthetic construct
  source 1..55: mol_type = other DNA
gtgactggagttcagacgtgtgctcttccgatctaaacaaatggcacgaagaagg

SEQ ID NO: 179 - DNA, 27 bp, synthetic construct
  source 1..27: mol_type = other DNA
ggagtctatataagaagtgtgttaggg

SEQ ID NO: 180 - DNA, 26 bp, synthetic construct
  source 1..26: mol_type = other DNA
tcattaagaagaagtccagaagaaga

SEQ ID NO: 181 - DNA, 51 bp, synthetic construct
  source 1..51: mol_type = other DNA
acactctttccctacacgacgctcttccgatctcagagccaaagcctcgat

SEQ ID NO: 182 - DNA, 57 bp, synthetic construct
  source 1..57: mol_type = other DNA
gtgactggagttcagacgtgtgctcttccgatctagcatcacctacttgaccatatt

SEQ ID NO: 183 - DNA, 24 bp, synthetic construct
  source 1..24: mol_type = other DNA
ccggttagtgatactcaggtattg

SEQ ID NO: 184 - DNA, 23 bp, synthetic construct
  source 1..23: mol_type = other DNA
tgactgcttcctaagatgctaaa

SEQ ID NO: 185 - DNA, 59 bp, synthetic construct
  source 1..59: mol_type = other DNA
acactctttccctacacgacgctcttccgatctctcgacgtttttctctttcaacagat

SEQ ID NO: 186 - DNA, 63 bp, synthetic construct
  source 1..63: mol_type = other DNA
gtgactggagttcagacgtgtgctcttccgatctcacttattaaaaacttatgtaaatctaac

SEQ ID NO: 187 - DNA, 25 bp, synthetic construct
  source 1..25: mol_type = other DNA
ctttcaggttcttatcgttggattc

SEQ ID NO: 188 - DNA, 25 bp, synthetic construct
  source 1..25: mol_type = other DNA
aggttagctaggtagattaggtagt

SEQ ID NO: 189 - DNA, 61 bp, synthetic construct
  source 1..61: mol_type = other DNA
acactctttccctacacgacgctcttccgatctggagacagttcataattggagagattat

SEQ ID NO: 190 - DNA, 56 bp, synthetic construct
  source 1..56: mol_type = other DNA
gtgactggagttcagacgtgtgctcttccgatctttgaagtatgactcagatagca

SEQ ID NO: 191 - DNA, 27 bp, synthetic construct
  source 1..27: mol_type = other DNA
aagtagtggacaaacataaagtagtgg

SEQ ID NO: 192 - DNA, 26 bp, synthetic construct
  source 1..26: mol_type = other DNA
aataatctatgtcgaacctctttcgg

SEQ ID NO: 193 - DNA, 58 bp, synthetic construct
  source 1..58: mol_type = other DNA
acactctttccctacacgacgctcttccgatctatatcctaacggggcgaggccaaat

SEQ ID NO: 194 - DNA, 60 bp, synthetic construct
  source 1..60: mol_type = other DNA
gtgactggagttcagacgtgtgctcttccgatctgcatgatccaattagtttttacccct

SEQ ID NO: 195 - DNA, 23 bp, synthetic construct
  source 1..23: mol_type = other DNA
gtgaatattattgctggcctgtt

SEQ ID NO: 196 - DNA, 22 bp, synthetic construct
  source 1..22: mol_type = other DNA
caactagtacaacaggtctcgt

SEQ ID NO: 197 - DNA, 53 bp, synthetic construct
  source 1..53: mol_type = other DNA
acactctttccctacacgacgctcttccgatctggtgctgtttcttcagggaa

SEQ ID NO: 198 - DNA, 56 bp, synthetic construct
  source 1..56: mol_type = other DNA
gtgactggagttcagacgtgtgctcttccgatcttagccatctcaagctgttcaag

SEQ ID NO: 199 - DNA, 24 bp, synthetic construct
  source 1..24: mol_type = other DNA
gactctaactaatctgtggtggtt

SEQ ID NO: 200 - DNA, 22 bp, synthetic construct
  source 1..22: mol_type = other DNA
gaaacgaactccgggaatatct

SEQ ID NO: 201 - DNA, 60 bp, synthetic construct
  source 1..60: mol_type = other DNA
acactctttccctacacgacgctcttccgatctctgcttacatatcttaaaaacatctat

SEQ ID NO: 202 - DNA, 60 bp, synthetic construct
  source 1..60: mol_type = other DNA
gtgactggagttcagacgtgtgctcttccgatctgcaatctttttcccattcttgatgag

SEQ ID NO: 203 - DNA, 23 bp, synthetic construct
  source 1..23: mol_type = other DNA
tgagagagcatacacaagcatag

SEQ ID NO: 204 - DNA, 22 bp, synthetic construct
  source 1..22: mol_type = other DNA
tgagaagcaagatggtgttagg

SEQ ID NO: 205 - DNA, 56 bp, synthetic construct
  source 1..56: mol_type = other DNA
acactctttccctacacgacgctcttccgatctggtttttggcccttgcatttaac

SEQ ID NO: 206 - DNA, 58 bp, synthetic construct
  source 1..58: mol_type = other DNA
gtgactggagttcagacgtgtgctcttccgatctggaacgaatgcagcaatcttcttc

SEQ ID NO: 207 - DNA, 24 bp, synthetic construct
  source 1..24: mol_type = other DNA
ctacagttctaggtgtgcactaat

SEQ ID NO: 208 - DNA, 21 bp, synthetic construct
  source 1..21: mol_type = other DNA
cgaccaaatccagcaatcaac

SEQ ID NO: 209 - DNA, 57 bp, synthetic construct
  source 1..57: mol_type = other DNA
acactctttccctacacgacgctcttccgatctctccaagtcatgcagaattaacac

SEQ ID NO: 210 - DNA, 57 bp, synthetic construct; identical to SEQ ID NO: 209
  source 1..57: mol_type = other DNA

SEQ ID NO: 211 - DNA, 149 bp, synthetic construct
  source 1..149: mol_type = other DNA
gctacaaatcttgttagtggtcttgcggatgctttgttagatagtattccgattgttgctattacaggtcaagtgccaaggaggatgattggtactgatgcgttccaggaaacgcctattgttgaggtaacgagatctattacgaagca

SEQ ID NO: 212 - DNA, 26 bp, synthetic construct
  source 1..26: mol_type = other DNA
aggtcaagtgtctaggaggatgattg

SEQ ID NO: 213 - DNA, 26 bp, synthetic construct
  source 1..26: mol_type = other DNA
caatcatcctcctagacacttgacct

SEQ ID NO: 214 - DNA, 155 bp, synthetic construct
  source 1..155: mol_type = other DNA
aggacctgagacagtagaggacttcgctaaaatggagttgcaggaaattcgagataatattagaagtaggaggaacaagatatttttgcatatggaggaggtctgtgtttttttttcttccttctcaaaattcgtatttattactgtgatgtcta

SEQ ID NO: 215 - DNA, 31 bp, synthetic construct
  source 1..31: mol_type = other DNA
ataatattagaagtcataggaacaagatatt

SEQ ID NO: 216 - DNA, 31 bp, synthetic construct; identical to SEQ ID NO: 28
  source 1..31: mol_type = other DNA

SEQ ID NO: 217 - DNA, 210 bp, synthetic construct
  source 1..210: mol_type = other DNA
tttcagcttcagtgcagaagccaaaacaaaagaagcgttacaggccagggacagtggcacttcgagaaatcagacactttcagaagacgtgggatcttcttattcgaataagaagatcccacgtcttctgaaagtgtctgatttctcgaagtgccactgtccctggcctgtaacgcttcttttgttttggcttctgcactgaagctgaaa

SEQ ID NO: 218 - DNA, 29 bp, synthetic construct
  source 1..29: mol_type = other DNA
gcgttacaggcctgaaacagtggcacttc

SEQ ID NO: 219 - DNA, 25 bp, synthetic construct
  source 1..25: mol_type = other DNA
gcgttacaggccagtggcacttcga

SEQ ID NO: 220 - DNA, 96 bp, synthetic construct
  source 1..96: mol_type = other DNA
tctgatttctcgaagtgccactgtttcaggcctgtaacgcttcttttgcaaaagaagcgttacaggcctgaaacagtggcacttcgagaaatcaga

SEQ ID NO: 221 - DNA, 84 bp, synthetic construct
  source 1..84: mol_type = other DNA
tctgatttctcgaagtgccactggcctgtaacgcttcttttgcaaaagaagcgttacaggccagtggcacttcgagaaatcaga

SEQ ID NO: 222 - DNA, 155 bp, synthetic construct
  source 1..155: mol_type = other DNA
taaatggggcccctccagatatttttccaacagttattctttatatataagtatataaattgtgcaagaaacttagtgaggtccaattaattaaaagagaaattaagcaatagagaaaatggcagcaacaggtagctcagccacagttgttagag

SEQ ID NO: 223 - DNA, 38 bp, synthetic construct
  source 1..38: mol_type = other DNA
gcaagaaacttagtgaaaattgtgaggtccaattaatt

SEQ ID NO: 224 - DNA, 38 bp, synthetic construct; identical to SEQ ID NO: 32
  source 1..38: mol_type = other DNA

SEQ ID NO: 225 - DNA, 158 bp, synthetic construct
  source 1..158: mol_type = other DNA
cttgagggataagaatgagaagaagacctgaatttttcttgaaaatcatcatgttttcatttgtaggtaaaaaaccacaatttgcaaaagttgatactgtggtgaatagtgaaaaagtatgtaaattaaggcctttttggtcaaggatttgtttggcg

SEQ ID NO: 226 - DNA, 47 bp, synthetic construct; identical to SEQ ID NO: 33
  source 1..47: mol_type = other DNA

SEQ ID NO: 227 - DNA, 54 bp, synthetic construct
  source 1..54: mol_type = other DNA
accacagtatcaacttttgcagactgtggtttcttacctacaaatgaaaacatg

SEQ ID NO: 228 - DNA, 260 bp, synthetic construct
  source 1..260: mol_type = other DNA
ggcagtttcctgtcggtaaaaagtctgaggaagaaatccaactattccttggaaatgcaggaacagcaatgcgtccgttgacagcagcagttactgtagctggaggacattcaaggtctttcaatcgttccttcttcgtgccatttgtttaacgattgaaagaccttgaatgtcctccagctacagtaactgctgctgtcaacggacgcattgctgttcctgcatttccaaggaatagttggatttcttcctcagacttt

SEQ ID NO: 229 - DNA, 45 bp, synthetic construct
  source 1..45: mol_type = other DNA
ttccttggaaatgcaggaatcgcaatgcgttctttgacagcagca

SEQ ID NO: 230 - DNA, 112 bp, synthetic construct
  source 1..112: mol_type = other DNA
tacagtaactgctgctgtcaaagaacgcattgcgattcctgcatttccaaggaatatattccttggaaatgcaggaatcgcaatgcgttctttgacagcagcagttactgta

SEQ ID NO: 231 - DNA, 147 bp, synthetic construct
  source 1..147: mol_type = other DNA
cagagccaaagcctcgatggaatccaagacctgagcaaattcgtatacttgaagcaatctttaattcaggcatggtgaatccaccaagggatgagataaggaaaatccgagctaaacttcaagaatatggtcaagtaggtgatgcta

SEQ ID NO: 232 - DNA, 32 bp, synthetic construct
  source 1..32: mol_type = other DNA
agcaatctttaattctgatatggtgaatccac

SEQ ID NO: 233 - DNA, 32 bp, synthetic construct; identical to SEQ ID NO: 36
  source 1..32: mol_type = other DNA

SEQ ID NO: 234 - DNA, 150 bp, synthetic construct
  source 1..150: mol_type = other DNA
tctcgacgtttttctctttcaacagatgaactacaatgagtatgtgaggctaaaagctagagttgagctccttcaacgttctcaaaggtaagatattagtgatgtaattaaatgattttagttagatttacataagtttttaataagtga

SEQ ID NO: 235 - DNA, 31 bp, synthetic construct
  source 1..31: mol_type = other DNA
ttcaacgttcttagatgtaagatattagtga

SEQ ID NO: 236 - DNA, 31 bp, synthetic construct; identical to SEQ ID NO: 37
  source 1..31: mol_type = other DNA

SEQ ID NO: 237 - DNA, 169 bp, synthetic construct
  source 1..169: mol_type = other DNA
ggagacagttcataattggagagattatctcagacttcattgttatcctctagagaagtatgctcctgaatggccttctaatccatcatctttcaggtaaacaccattaattaactgtttaattactttctttatgttaatatacattgctatctgagtcatacttcaa

SEQ ID NO: 238 - DNA, 42 bp, synthetic construct
  source 1..42: mol_type = other DNA
cctctagagaagtatgctccttaatccatcatctttcaggta

SEQ ID NO: 239 - DNA, 66 bp, synthetic construct
  source 1..66: mol_type = other DNA
tacctgaaagatgatggattaaggagcatacttctctagaggaagatgatggattaaggagcatac

SEQ ID NO: 240 - DNA, 122 bp, synthetic construct
  source 1..122: mol_type = other DNA
tttggtggtttaccgccgtaaaaaacgagcgccttttttaccccaaccttttgtgttccaccggaagtaaaaaccggcttgtcggttccggtagccttccaataacccgatgttgcagcccg

SEQ ID NO: 241 - DNA, 28 bp, synthetic construct
  source 1..28: mol_type = other DNA
ggaaccgacaaaccagattttacttccg

SEQ ID NO: 242 - DNA, 48 bp, synthetic construct
  source 1..48: mol_type = other DNA
gaaggctaccggaaccgacaaaccagattttacttccggtggaacaca

SEQ ID NO: 243 - DNA, 115 bp, synthetic construct
  source 1..115: mol_type = other DNA
aagtaagatttgggaagaagatgaagaagaaaaaccagatgctggaatggatgagcttttagctgttttgggttataaagtgaagtcgtctgatatggcggatgttgctcaaaaa

SEQ ID NO: 244 - DNA, 42 bp, synthetic construct
  source 1..42: mol_type = other DNA
ccagatgctggtatggatgagcttttagttttgggttataaa

SEQ ID NO: 245 - DNA, 58 bp, synthetic construct
  source 1..58: mol_type = other DNA
cttcactttataacccaaaactaaaagctcatccataccagcatctggtttttcttct

SEQ ID NO: 246 - DNA, 251 bp, synthetic construct
  source 1..251: mol_type = other DNA
tctgcttacatatcttaaaaacatctataattgtatctaacctgtgaagttgctaatatgtgtttgcagaggtattgaggctaaacagccaaattctgctattcgtaaatgtgctagggttcaactcatcaagaatgggaaaaagattgcatgagttgaaccctagcacatttacgaatagcagaatttggctgtttagcctcaatacctctgcaaacacatattagcaacttcacaggttagatacaatt

SEQ ID NO: 247 - DNA, 51 bp, synthetic construct
  source 1..51: mol_type = other DNA
ttgcagaggtattgaggctagacagcctaactctgctattcgtaaatgtgc

SEQ ID NO: 248 - DNA, 33 bp, synthetic construct
  source 1..33: mol_type = other DNA
gtattgaggctagacagcctaactctgctattc

SEQ ID NO: 249 - DNA, 248 bp, synthetic construct
  source 1..248: mol_type = other DNA
tggtttttggcccttgcatttaaccaatcaaaacaatttgaaatgatttttgcagaggtattgaggctaagcagcccaattctgctattcgtaaatgtgctagggttcaattgatcaaaaatgggaagaagattgctgcattcgttccccatttttgatcaattgaaccctagcacatttacgaatagcagaattgggctgcttagcctcaatacctctgcaaaaatcatttcaaattgttttgattg

SEQ ID NO: 250 - DNA, 52 bp, synthetic construct
  source 1..52: mol_type = other DNA
ttgcagaggtattgaggctagacagcctaactctgctattcgtaaatgtgct

SEQ ID NO: 251 - DNA, 33 bp, synthetic construct; identical to SEQ ID NO: 248
  source 1..33: mol_type = other DNA

SEQ ID NO: 252 - DNA, 248 bp, synthetic construct
  source 1..248: mol_type = other DNA
tctccaagtcatgcagaattaacacttggctctaatgttcaaacttgctggaatgtttgtgcagaggtattgaagctaagcagccgaattctgccattcgtaaatgtgctagggttcaactcatcaaaaatgggaagaagattgctgccatgagttgaaccctagcacatttacgaatggcagaattcggctgcttagcttcaatacctctgcacaaacattccagcaagtttgaacattagagccaa

SEQ ID NO: 253 - DNA, 62 bp, synthetic construct
  source 1..62: mol_type = other DNA
tgtttgtgcagaggtattgaggctagacagcctaactctgctattcgtaaatgtgctagggt

SEQ ID NO: 254 - DNA, 33 bp, synthetic construct; identical to SEQ ID NO: 248
  source 1..33: mol_type = other DNA

SEQ ID NO: 255 - DNA, 6564 bp, synthetic construct
  source 1..6564: mol_type = other DNA
atgaaacggacagccgacggaagcgagttcgagtcaccaaagaagaagcggaaagtcgacaagaagtacagcatcggcctggacatcggcaccaactctgtgggctgggccgtgatcaccgacgagtacaaggtgcccagcaagaaattcaaggtgctgggcaacaccgaccggcacagcatcaagaagaacctgatcggagccctgctgttcgacagcggcgaaacagccgaggccacccggctgaagagaaccgccagaagaagatacaccagacggaagaaccggatctgctatctgcaagagatcttcagcaacgagatggccaaggtggacgacagcttcttccacagactggaagagtccttcctggtggaagaggataagaagcacgagcggcaccccatcttcggcaacatcgtggacgaggtggcctaccacgagaagtaccccaccatctaccacctgagaaagaaactggtggacagcaccgacaaggccgacctgcggctgatctatctggccctggcccacatgatcaagttccggggccacttcctgatcgagggcgacctgaaccccgacaacagcgacgtggacaagctgttcatccagctggtgcagacctacaaccagctgttcgaggaaaaccccatcaacgccagcggcgtggacgccaaggccatcctgtctgccagactgagcaagagcagaaagctggaaaatctgatcgcccagctgcccggcgagaagaagaatggcctgttcggaaacctgattgccctgagcctgggcctgacccccaacttcaagagcaacttcgacctggccgaggatgccaaactgcagctgagcaaggacacctacgacgacgacctggacaacctgctggcccagatcggcgaccagtacgccgacctgtttctggccgccaagaacctgtccgacgccatcctgctgagcgacatcctgagagtgaacaccgagatcaccaaggcccccctgagcgcctctatgatcaagagatacgacgagcaccaccaggacctgaccctgctgaaagctctcgtgcggcagcagctgcctgagaagtacaaagagattttcttcgaccagagcaagaacggctacgccggctacattgacggcggagccagccaggaagagttctacaagttcatcaagcccatcctggaaaagatggacggcaccgaggaactgctcgtgaagctgaagagagaggacctgctgcggaagcagcggaccttcgacaacggcagcatcccccaccagatccacctgggagagctgcacgccattctgcggcggcaggaagatttttacccattcctgaaggacaaccgggaaaagatcgagaagatcctgaccttccgcatcccctactacgtgggccctctggccaggggaaacagcagattcgcctggatgaccagaaagagcgaggaaaccatcaccccctggaacttcgaggaagtggtggacaagggcgcttccgcccagagcttcatcgagcggatgaccaacttcgataagaacctgcccaacgagaaggtgctgcccaagcacagcctgctgtacgagtacttcaccgtgtataacgagctgaccaaagtgaaatacgtgaccgagggaatgagaaagcccgccttcctgagcggcgagcagaaaaaggccatcgtggacctgctgttcaagaccaaccggaaagtgaccgtgaagcagctgaaagaggactacttcaagaaaatcgagtgcttcgactccgtggaaatctccggcgtggaagatcggttcaacgcctccctgggcacataccacgatctgctgaaaattatcaaggacaaggacttcctggacaatgaggaaaacgaggacattctggaagatatcgtgctgaccctgacactgtttgaggacagagagatgatcgaggaacggctgaaaacctatgcccacctgttcgacgacaaagtgatgaagcagctgaagcggcggagatacaccggctggggcaggctgagccggaagctgatcaacggcatccgggacaagcagtccggcaagacaatcctggatttcctgaagtccgacggcttcgccaacagaaacttcatgcagctgatccacgacgacagcctgacctttaaagaggacatccagaaagcccaggtgtccggccagggcgatagcctgcacgagcacattgccaatctggccggcagccccgccattaagaagggcatcctgcagacagtgaaggtggtggacgagctcgtgaaagtgatgggccggcacaagcccgagaacatcgtgatcgaaatggccagagagaaccagaccacccagaagggacagaagaacagccgcgagagaatgaagcggatcgaagagggcatcaaagagctgggcagccagatcctgaaagaacaccccgtggaaaacacccagctgcagaacgagaagctgtacctgtactacctgcagaatgggcgggatatgtacgtggaccaggaactggacatcaaccggctgtccgactacgatgtggacgctatcgtgcctcagagctttctgaaggacgactccatcgacaacaaggtgctgaccagaagcgacaagaaccggggcaagagcgacaacgtgccctccgaagaggtcgtgaagaagatgaagaactactggcggcagctgctgaacgccaagctgattacccagagaaagttcgacaatctgaccaaggccgagagaggcggcctgagcgaactggataaggccggcttcatcaagagacagctggtggaaacccggcagatcacaaagcacgtggcacagatcctggactcccggatgaacactaagtacgacgagaatgacaagctgatccgggaagtgaaagtgatcaccctgaagtccaagctggtgtccgatttccggaaggatttccagttttacaaagtgcgcgagatcaacaactaccaccacgcccacgacgcctacctgaacgccgtcgtgggaaccgccctgatcaaaaagtaccctaagctggaaagcgagttcgtgtacggcgactacaaggtgtacgacgtgcggaagatgatcgccaagagcgagcaggaaatcggcaaggctaccgccaagtacttcttctacagcaacatcatgaactttttcaagaccgagattaccctggccaacggcgagatccggaagcggcctctgatcgagacaaacggcgaaaccggggagatcgtgtgggataagggccgggattttgccaccgtgcggaaagtgctgagcatgccccaagtgaatatcgtgaaaaagaccgaggtgcagacaggcggcttcagcaaagagtctatcctgcccaagaggaacagcgataagctgatcgccagaaagaaggactgggaccctaagaagtacggcggcttcgacagccccaccgtggcctattctgtgctggtggtggccaaagtggaaaagggcaagtccaagaaactgaagagtgtgaaagagctgctggggatcaccatcatggaaagaagcagcttcgagaagaatcccatcgactttctggaagccaagggctacaaagaagtgaaaaaggacctgatcatcaagctgcctaagtactccctgttcgagctggaaaacggccggaagagaatgctggcctctgccggcgaactgcagaagggaaacgaactggccctgccctccaaatatgtgaacttcctgtacctggccagccactatgagaagctgaagggctcccccgaggataatgagcagaaacagctgtttgtggaacagcacaagcactacctggacgagatcatcgagcagatcagcgagttctccaagagagtgatcctggccgacgctaatctggacaaagtgctgtccgcctacaacaagcaccgggataagcccatcagagagcaggccgagaatatcatccacctgtttaccctgaccaatctgggagcccctgccgccttcaagtactttgacaccaccatcgaccggaagaggtacaccagcaccaaagaggtgctggacgccaccctgatccaccagagcatcaccggcctgtacgagacacggatcgacctgtctcagctgggaggtgactccggcggaagctctggtggcagcaagcggaccgccgacggctctgaattcgagagccctaagaagaaaagaaaggtgagcggaggctctagcggcggaagcaccctgaacattgaagatgagtatagactgcatgaaacaagcaaggaacccgacgtgtccctgggctccacctggctgtccgactttccccaggcctgggccgagacaggaggaatgggcctggccgtgcggcaggcacccctgatcatccctctgaaggccacctctacacccgtgagcatcaagcagtaccctatgtctcaggaggccagactgggcatcaagcctcacatccagaggctgctggaccagggcatcctggtgccatgccagagcccctggaacacaccactgctgcccgtgaagaagccaggcaccaatgactatagacccgtgcaggatctgagagaggtgaacaagagggtggaggatatccaccccaccgtgcccaacccttacaatctgctgtccggcctgcccccttctcaccagtggtatacagtgctggacctgaaggatgccttcttttgtctgagactgcaccctaccagccagccactgttcgcctttgagtggagggaccctgagatgggcatctctggccagctgacctggacacgcctgcctcagggcttcaagaatagcccaacactgtttaacgaggccctgcaccgcgacctggcagatttccggatccagcacccagatctgatcctgctgcagtacgtggacgatctgctgctggccgccaccagcgagctggattgccagcagggaacacgcgccctgctgcagaccctgggaaacctgggatatagggcatccgccaagaaggcccagatctgtcagaagcaggtgaagtacctgggctatctgctgaaggagggccagagatggctgacagaggccaggaaggagacagtgatgggccagccaacacccaagaccccaagacagctgagggagttcctgggcaaagcaggattttgcaggctgttcatcccaggattcgcagagatggcagcacctctgtacccactgaccaagccgggcaccctgtttaattggggccctgaccagcagaaggcctatcaggagatcaagcaggccctgctgacagcaccagccctgggcctgccagacctgaccaagcctttcgagctgtttgtggatgagaagcagggctacgccaagggcgtgctgacccagaagctgggaccatggagacggcccgtggcctatctgtccaagaagctggacccagtggcagcaggatggccaccatgcctgaggatggtggcagcaatcgccgtgctgacaaaggatgccggcaagctgaccatgggacagccactggtcatcctggcaccacacgcagtggaggccctggtgaagcagcctccagatcgctggctgtctaacgcccggatgacacactaccaggccctgctgctggacaccgatcgcgtgcagtttggccctgtggtggccctgaatccagccaccctgctgcctctgccagaggagggcctgcagcacaactgtctggacatcctggcagaggcacacggaacaaggccagacctgaccgatcagcccctgcctgacgccgatcacacatggtataccgatggaagctccctgctgcaggagggccagaggaaggcaggagcagcagtgaccacagagacagaagtgatctgggccaaggccctgccagcaggcacatccgcccagcgggccgagctgatcgccctgacccaggccctgaagatggccgagggcaagaagctgaacgtgtacacagactccagatatgccttcgccaccgcacacatccacggagagatctacaggcgccggggctggctgacctctgagggcaaggagatcaagaacaaggatgagatcctggccctgctgaaggccctgtttctgcccaagcggctgagcatcatccactgtcctggacaccagaagggacactccgccgaggcaaggggcaatcggatggccgaccaggccgccagaaaggctgctattactgaaactcccgacacttccactctgctgattgaaaactcctccccttctggcggctcaaaaagaaccgccgacggcagcgaattcgagtctcccaagaagaagaggaaagtcggctctggccctgccgctaagagagtgaagctggacgccacagtggtgtccggccaaaagcaggaccgccagggcggagaacgcagaaggtcccagctcgatagggatcagtgtgcctactgcaaggagaagggccactgggccaaagactgcccgaaaaagccgcgcggcccacgcggcccaaggccacaaacatccctcctttaa

SEQ ID NO: 256 - DNA, 6159 bp, synthetic construct
  source 1..6159: mol_type = other DNA
atgaaacggacagccgacggaagcgagttcgagtcaccaaagaagaagcggaaagtcgacaagaagtacagcatcggcctggacatcggcaccaactctgtgggctgggccgtgatcaccgacgagtacaaggtgcccagcaagaaattcaaggtgctgggcaacaccgaccggcacagcatcaagaagaacctgatcggagccctgctgttcgacagcggcgaaacagccgaggccacccggctgaagagaaccgccagaagaagatacaccagacggaagaaccggatctgctatctgcaagagatcttcagcaacgagatggccaaggtggacgacagcttcttccacagactggaagagtccttcctggtggaagaggataagaagcacgagcggcaccccatcttcggcaacatcgtggacgaggtggcctaccacgagaagtaccccaccatctaccacctgagaaagaaactggtggacagcaccgacaaggccgacctgcggctgatctatctggccctggcccacatgatcaagttccggggccacttcctgatcgagggcgacctgaaccccgacaacagcgacgtggacaagctgttcatccagctggtgcagacctacaaccagctgttcgaggaaaaccccatcaacgccagcggcgtggacgccaaggccatcctgtctgccagactgagcaagagcagaaagctggaaaatctgatcgcccagctgcccggcgagaagaagaatggcctgttcggaaacctgattgccctgagcctgggcctgacccccaacttcaagagcaacttcgacctggccgaggatgccaaactgcagctgagcaaggacacctacgacgacgacctggacaacctgctggcccagatcggcgaccagtacgccgacctgtttctggccgccaagaacctgtccgacgccatcctgctgagcgacatcctgagagtgaacaccgagatcaccaaggcccccctgagcgcctctatgatcaagagatacgacgagcaccaccaggacctgaccctgctgaaagctctcgtgcggcagcagctgcctgagaagtacaaagagattttcttcgaccagagcaagaacggctacgccggctacattgacggcggagccagccaggaagagttctacaagttcatcaagcccatcctggaaaagatggacggcaccgaggaactgctcgtgaagctgaagagagaggacctgctgcggaagcagcggaccttcgacaacggcagcatcccccaccagatccacctgggagagctgcacgccattctgcggcggcaggaagatttttacccattcctgaaggacaaccgggaaaagatcgagaagatcctgaccttccgcatcccctactacgtgggccctctggccaggggaaacagcagattcgcctggatgaccagaaagagcgaggaaaccatcaccccctggaacttcgaggaagtggtggacaagggcgcttccgcccagagcttcatcgagcggatgaccaacttcgataagaacctgcccaacgagaaggtgctgcccaagcacagcctgctgtacgagtacttcaccgtgtataacgagctgaccaaagtgaaatacgtgaccgagggaatgagaaagcccgccttcctgagcggcgagcagaaaaaggccatcgtggacctgctgttcaagaccaaccggaaagtgaccgtgaagcagctgaaagaggactacttcaagaaaatcgagtgcttcgactccgtggaaatctccggcgtggaagatcggttcaacgcctccctgggcacataccacgatctgctgaaaattatcaaggacaaggacttcctggacaatgaggaaaacgaggacattctggaagatatcgtgctgaccctgacactgtttgaggacagagagatgatcgaggaacggctgaaaacctatgcccacctgttcgacgacaaagtgatgaagcagctgaagcggcggagatacaccggctggggcaggctgagccggaagctgatcaacggcatccgggacaagcagtccggcaagacaatcctggatttcctgaagtccgacggcttcgccaacagaaacttcatgcagctgatccacgacgacagcctgacctttaaagaggacatccagaaagcccaggtgtccggccagggcgatagcctgcacgagcacattgccaatctggccggcagccccgccattaagaagggcatcctgcagacagtgaaggtggtggacgagctcgtgaaagtgatgggccggcacaagcccgagaacatcgtgatcgaaatggccagagagaaccagaccacccagaagggacagaagaacagccgcgagagaatgaagcggatcgaagagggcatcaaagagctgggcagccagatcctgaaagaacaccccgtggaaaacacccagctgcagaacgagaagctgtacctgtactacctgcagaatgggcgggatatgtacgtggaccaggaactggacatcaaccggctgtccgactacgatgtggacgctatcgtgcctcagagctttctgaaggacgactccatcgacaacaaggtgctgaccagaagcgacaagaaccggggcaagagcgacaacgtgccctccgaagaggtcgtgaagaagatgaagaactactggcggcagctgctgaacgccaagctgattacccagagaaagttcgacaatctgaccaaggccgagagaggcggcctgagcgaactggataaggccggcttcatcaagagacagctggtggaaacccggcagatcacaaagcacgtggcacagatcctggactcccggatgaacactaagtacgacgagaatgacaagctgatccgggaagtgaaagtgatcaccctgaagtccaagctggtgtccgatttccggaaggatttccagttttacaaagtgcgcgagatcaacaactaccaccacgcccacgacgcctacctgaacgccgtcgtgggaaccgccctgatcaaaaagtaccctaagctggaaagcgagttcgtgtacggcgactacaaggtgtacgacgtgcggaagatgatcgccaagagcgagcaggaaatcggcaaggctaccgccaagtacttcttctacagcaacatcatgaactttttcaagaccgagattaccctggccaacggcgagatccggaagcggcctctgatcgagacaaacggcgaaaccggggagatcgtgtgggataagggccgggattttgccaccgtgcggaaagtgctgagcatgccccaagtgaatatcgtgaaaaagaccgaggtgcagacaggcggcttcagcaaagagtctatcctgcccaagaggaacagcgataagctgatcgccagaaagaaggactgggaccctaagaagtacggcggcttcgacagccccaccgtggcctattctgtgctggtggtggccaaagtggaaaagggcaagtccaagaaactgaagagtgtgaaagagctgctggggatcaccatcatggaaagaagcagcttcgagaagaatcccatcgactttctggaagccaagggctacaaagaagtgaaaaaggacctgatcatcaagctgcctaagtactccctgttcgagctggaaaacggccggaagagaatgctggcctctgccggcgaactgcagaagggaaacgaactggccctgccctccaaatatgtgaacttcctgtacctggccagccactatgagaagctgaagggctcccccgaggataatgagcagaaacagctgtttgtggaacagcacaagcactacctggacgagatcatcgagcagatcagcgagttctccaagagagtgatcctggccgacgctaatctggacaaagtgctgtccgcctacaacaagcaccgggataagcccatcagagagcaggccgagaatatcatccacctgtttaccctgaccaatctgggagcccctgccgccttcaagtactttgacaccaccatcgaccggaagaggtacaccagcaccaaagaggtgctggacgccaccctgatccaccagagcatcaccggcctgtacgagacacggatcgacctgtctcagctgggaggtgactccggcggaagctctggtggcagcaagcggaccgccgacggctctgaattcgagagcgccacagtggtgtccggccaaaagcaggaccgccagggcggagaacgcagaaggtcccagctcgatagggatcagtgtgcctactgcaaggagaagggccactgggccaaagactgcccgaaaaagccgcgcggcccacgcggcccaaggccacaaacatccctccttccaaagaagaagcggaaggtggagctcagcggaggatcttccggaggatctagcggctccgagacaccaggaacatccgaaagcgctacaccagaatctagcggaggctcttccggaggatctaggcctaccctgaacattgaagatgagtatagactgcatgaaacaagcaaggaacccgacgtgtccctgggctccacctggctgtccgactttccccaggcctgggccgagacaggaggaatgggcctggccgtgcggcaggcacccctgatcatccctctgaaggccacctctacacccgtgagcatcaagcagtaccctatgtctcaggaggccagactgggcatcaagcctcacatccagaggctgctggaccagggcatcctggtgccatgccagagcccctggaacacaccactgctgcccgtgaagaagccaggcaccaatgactatagacccgtgcaggatctgagagaggtgaacaagagggtggaggatatccaccccaccgtgcccaacccttacaatctgctgtccggcctgcccccttctcaccagtggtatacagtgctggacctgaaggatgccttcttttgtctgagactgcaccctaccagccagccactgttcgcctttgagtggagggaccctgagatgggcatctctggccagctgacctggacacgcctgcctcagggcttcaagaatagcccaacactgtttaacgaggccctgcaccgcgacctggcagatttccggatccagcacccagatctgatcctgctgcagtacgtggacgatctgctgctggccgccaccagcgagctggattgccagcagggaacacgcgccctgctgcagaccctgggaaacctgggatatagggcatccgccaagaaggcccagatctgtcagaagcaggtgaagtacctgggctatctgctgaaggagggccagagatggctgacagaggccaggaaggagacagtgatgggccagccaacacccaagaccccaagacagctgagggagttcctgggcaaagcaggattttgcaggctgttcatcccaggattcgcagagatggcagcacctctgtacccactgaccaagccgggcaccctgtttaattggggccctgaccagcagaaggcctatcaggagatcaagcaggccctgctgacagcaccagccctgggcctgccagacctgaccaagcctttcgagctgtttgtggatgagaagcagggctacgccaagggcgtgctgacccagaagctgggaccatggagacggcccgtggcctatctgtccaagaagctggacccagtggcagcaggatggccaccatgcctgaggatggtggcagcaatcgccgtgctgacaaaggatgccggcaagctgaccatgggacagccactggtcatcctggcaccacacgcagtggaggccctggtgaagcagcctccagatcgctggctgtctaacgcccggatgacacactaccaggccctgctgctggacaccgatcgcgtgcagtttggccctgtggtggccctgaatccagccaccctgctgcctctgccagaggagggcctgcagcacaactgtctggacatcctggcagaggcacacggaacaaggccagacctgaccgatcagcccctgtctggcggctcaaaaagaaccgccgacggcagcgaattcgagtctcccaagaagaagaggaaagtcggctctggccctgccgctaagagagtgaagctggactaa

SEQ ID NO: 257 - DNA, 181 bp, synthetic construct
  source 1..181: mol_type = other DNA
ctattacaggtcaagtgccagtttaagagctaggccaacatgaggatcacccatgtctgcagggcctagcaagtttaaataaggctagtccgttatcaacttgaaaaagtggcaccgagtcggtgcaatcatcctcctagacacttgacctgtagggaacatgaggatcacccatgttccc

SEQ ID NO: 258 - DNA, 282 bp, synthetic construct
  source 1..282: mol_type = other DNA
gcaccagtggtctagtggtagaatagtaccctgccacggtacagacccgggttcgattcccggctggtgcacctaacccataggcgtttccgtttaagagctatgctggaaacagcatagcaagtttaaataaggctagtccgttatcgacttgaaaaagtcgcaccgagtcggtgccgcggttctatctagttacgcgttaaaccaactagaaggccggcatggtcccagcctcctcgctggcgccggctgggcaacatgcttcggcatggcgaatgggac

SEQ ID NO: 259 - DNA, 301 bp, synthetic construct
  source 1..301: mol_type = other DNA
gcaccagtggtctagtggtagaatagtaccctgccacggtacagacccgggttcgattcccggctggtgcannnnnnnnnnnnnnnnnnngtttaagagctatgctggaaacagcatagcaagtttaaataaggctagtccgttatcgacttgaaaaagtcgcaccgagtcggtgcnnnnnnnnnnnnnnnnnnnncgcggttctatctagttacgcgttaaaccaactagaaggccggcatggtcccagcctcctcgctggcgccggctgggcaacatgcttcggcatggcgaatgggac

SEQ ID NO: 260 - DNA, 5880 bp, synthetic construct
  source 1..5880: mol_type = other DNA
atgaaacggacagccgacggaagcgagttcgagtcaccaaagaagaagcggaaagtcgacaagaagtacagcatcggcctggacatcggcaccaactctgtgggctgggccgtgatcaccgacgagtacaaggtgcccagcaagaaattcaaggtgctgggcaacaccgaccggcacagcatcaagaagaacctgatcggagccctgctgttcgacagcggcgaaacagccgaggccacccggctgaagagaaccgccagaagaagatacaccagacggaagaaccggatctgctatctgcaagagatcttcagcaacgagatggccaaggtggacgacagcttcttccacagactggaagagtccttcctggtggaagaggataagaagcacgagcggcaccccatcttcggcaacatcgtggacgaggtggcctaccacgagaagtaccccaccatctaccacctgagaaagaaactggtggacagcaccgacaaggccgacctgcggctgatctatctggccctggcccacatgatcaagttccggggccacttcctgatcgagggcgacctgaaccccgacaacagcgacgtggacaagctgttcatccagctggtgcagacctacaaccagctgttcgaggaaaaccccatcaacgccagcggcgtggacgccaaggccatcctgtctgccagactgagcaagagcagaaagctggaaaatctgatcgcccagctgcccggcgagaagaagaatggcctgttcggaaacctgattgccctgagcctgggcctgacccccaacttcaagagcaacttcgacctggccgaggatgccaaactgcagctgagcaaggacacctacgacgacgacctggacaacctgctggcccagatcggcgaccagtacgccgacctgtttctggccgccaagaacctgtccgacgccatcctgctgagcgacatcctgagagtgaacaccgagatcaccaaggcccccctgagcgcctctatgatcaagagatacgacgagcaccaccaggacctgaccctgctgaaagctctcgtgcggcagcagctgcctgagaagtacaaagagattttcttcgaccagagcaagaacggctacgccggctacattgacggcggagccagccaggaagagttctacaagttcatcaagcccatcctggaaaagatggacggcaccgaggaactgctcgtgaagctgaagagagaggacctgctgcggaagcagcggaccttcgacaacggcagcatcccccaccagatccacctgggagagctgcacgccattctgcggcggcaggaagatttttacccattcctgaaggacaaccgggaaaagatcgagaagatcctgaccttccgcatcccctactacgtgggccctctggccaggggaaacagcagattcgcctggatgaccagaaagagcgaggaaaccatcaccccctggaacttcgaggaagtggtggacaagggcgcttccgcccagagcttcatcgagcggatgaccaacttcgataagaacctgcccaacgagaaggtgctgcccaagcacagcctgctgtacgagtacttcaccgtgtataacgagctgaccaaagtgaaatacgtgaccgagggaatgagaaagcccgccttcctgagcggcgagcagaaaaaggccatcgtggacctgctgttcaagaccaaccggaaagtgaccgtgaagcagctgaaagaggactacttcaagaaaatcgagtgcttcgactccgtggaaatctccggcgtggaagatcggttcaacgcctccctgggcacataccacgatctgctgaaaattatcaaggacaaggacttcctggacaatgaggaaaacgaggacattctggaagatatcgtgctgaccctgacactgtttgaggacagagagatgatcgaggaacggctgaaaacctatgcccacctgttcgacgacaaagtgatgaagcagctgaagcggcggagatacaccggctggggcaggctgagccggaagctgatcaacggcatccgggacaagcagtccggcaagacaatcctggatttcctgaagtccgacggcttcgccaacagaaacttcatgcagctgatccacgacgacagcctgacctttaaagaggacatccagaaagcccaggtgtccggccagggcgatagcctgcacgagcacattgccaatctggccggcagccccgccattaagaagggcatcctgcagacagtgaaggtggtggacgagctcgtgaaagtgatgggccggcacaagcccgagaacatcgtgatcgaaatggccagagagaaccagaccacccagaagggacagaagaacagccgcgagagaatgaagcggatcgaagagggcatcaaagagctgggcagccagatcctgaaagaacaccccgtggaaaacacccagctgcagaacgagaagctgtacctgtactacctgcagaatgggcgggatatgtacgtggaccaggaactggacatcaaccggctgtccgactacgatgtggacgctatcgtgcctcagagctttctgaaggacgactccatcgacaacaaggtgctgaccagaagcgacaagaaccggggcaagagcgacaacgtgccctccgaagaggtcgtgaagaagatgaagaactactggcggcagctgctgaacgccaagctgattacccagagaaagttcgacaatctgaccaaggccgagagaggcggcctgagcgaactggataaggccggcttcatcaagagacagctggtggaaacccggcagatcacaaagcacgtggcacagatcctggactcccggatgaacactaagtacgacgagaatgacaagctgatccgggaagtgaaagtgatcaccctgaagtccaagctggtgtccgatttccggaaggatttccagttttacaaagtgcgcgagatcaacaactaccaccacgcccacgacgcctacctgaacgccgtcgtgggaaccgccctgatcaaaaagtaccctaagctggaaagcgagttcgtgtacggcgactacaaggtgtacgacgtgcggaagatgatcgccaagagcgagcaggaaatcggcaaggctaccgccaagtacttcttctacagcaacatcatgaactttttcaagaccgagattaccctggccaacggcgagatccggaagcggcctctgatcgagacaaacggcgaaaccggggagatcgtgtgggataagggccgggattttgccaccgtgcggaaagtgctgagcatgccccaagtgaatatcgtgaaaaagaccgaggtgcagacaggcggcttcagcaaagagtctatcctgcccaagaggaacagcgataagctgatcgccagaaagaaggactgggaccctaagaagtacggcggcttcgacagccccaccgtggcctattctgtgctggtggtggccaaagtggaaaagggcaagtccaagaaactgaagagtgtgaaagagctgctggggatcaccatcatggaaagaagcagcttcgagaagaatcccatcgactttctggaagccaagggctacaaagaagtgaaaaaggacctgatcatcaagctgcctaagtactccctgttcgagctggaaaacggccggaagagaatgctggcctctgccggcgaactgcagaagggaaacgaactggccctgccctccaaatatgtgaacttcctgtacctggccagccactatgagaagctgaagggctcccccgaggataatgagcagaaacagctgtttgtggaacagcacaagcactacctggacgagatcatcgagcagatcagcgagttctccaagagagtgatcctggccgacgctaatctggacaaagtgctgtccgcctacaacaagcaccgggataagcccatcagagagcaggccgagaatatcatccacctgtttaccctgaccaatctgggagcccctgccgccttcaagtactttgacaccaccatcgaccggaagaggtacaccagcaccaaagaggtgctggacgccaccctgatccaccagagcatcaccggcctgtacgagacacggatcgacctgtctcagctgggaggtgactccggcggaagctctggtggcagcaagcggaccgccgacggctctgaattcgagagccctaagaagaaaagaaaggtgagcggaggctctagcggcggaagcatcagcagctctaagcacaccctgagccagatgaacaaggtgagcaacatcgtgaaggaacccgagctgcccgacatctacaaggaatttaaggacatcaccgccgacaccaataccgagaagctgcctaagcctattaagggcctggaatttgaagtggaactgacacaggagaactacagactgcctatccggaactatcctctgactccagtcaagatgcaggccatgaacgacgagatcaatcaaggcctgaaaggcggcatcatcagagagagcaaggccatcaacgcctgccctgttatattcgtgcccagaaaggaaggcacactgcgcatggtggtcgactacaggcccctgaacaagtacgtgaagcccaacgtctaccccctgccactgattgaacaactgctggccaagatccagggcagcaccattttcaccaagctggacctgaaaagcgcctaccaccagatcagagtgcgaaagggagatgagcacaagctggccttccggtgccccagaggagttttcgagtacctggtgatgccttacggcatcaagacagcccctgcccactttcagtacttcatcaacacaatcctgggcgaggccaaggaaagccacgtggtgtgctacatggacgacatcctgatccattccaagtccgagtccgaacacgtgaaacatgtgaaggacgtgctgcaaaagctgaagaacgctaatctgatcatcaaccaggccaaatgcgagtttcaccagagccaagtgaagttcctgggctaccacatcagcgagaagggcttaaccccatgtcaggagaacatcgacaaggtgctgcagtggaaacagcctaaaaaccagaaggaactgagacagttcctgggccaggtgaactacctgagaaaattcatccccaaaaccagccagttgacccaccctctgaacaaactcctgaaaaaggatgtcagatggaaatggacccctacccagacccaggctatcgagaatatcaagcaatgtctggtgtctcctcctgtgctgaggcacttcgacttcagcaagaagatcctgcttgagacagacgtttctgatgtggccgtgggagccgtgctgagccagaagcatgatgatgataagtactaccctgtgggctattacagcgctaaaatgagcaaagcccagctgaattattctgtgtccgacaaggagatgctggctatcatcaaaagcctggagcactggcggcactacctggaatctacaatcgagcccttcaagatcctgaccgaccacagaaacctgattggaagaatcacaaacgagagcgaaccagagaacaagcggctggccagatggcagctgttcctgcaggacttcaacttcgagatcaactacagacctggctctgcaaatcacatcgccgatgccctgtctagaatcgtggacgagactgagcctatccctaaggacaacgaagataacagcatcaacttcgtgaaccagatcagcatctctggcggctcaaaaagaaccgccgacggcagcgaattcgagtctcccaagaagaagaggaaagtcggctctggccctgccgctaagagagtgaagctggactaa

SEQ ID NO: 261 - DNA, 6048 bp, synthetic construct
  source 1..6048: mol_type = other DNA
atgaaacggacagccgacggaagcgagttcgagtcaccaaagaagaagcggaaagtcgacaagaagtacagcatcggcctggacatcggcaccaactctgtgggctgggccgtgatcaccgacgagtacaaggtgcccagcaagaaattcaaggtgctgggcaacaccgaccggcacagcatcaagaagaacctgatcggagccctgctgttcgacagcggcgaaacagccgaggccacccggctgaagagaaccgccagaagaagatacaccagacggaagaaccggatctgctatctgcaagagatcttcagcaacgagatggccaaggtggacgacagcttcttccacagactggaagagtccttcctggtggaagaggataagaagcacgagcggcaccccatcttcggcaacatcgtggacgaggtggcctaccacgagaagtaccccaccatctaccacctgagaaagaaactggtggacagcaccgacaaggccgacctgcggctgatctatctggccctggcccacatgatcaagttccggggccacttcctgatcgagggcgacctgaaccccgacaacagcgacgtggacaagctgttcatccagctggtgcagacctacaaccagctgttcgaggaaaaccccatcaacgccagcggcgtggacgccaaggccatcctgtctgccagactgagcaagagcagaaagctggaaaatctgatcgcccagctgcccggcgagaagaagaatggcctgttcggaaacctgattgccctgagcctgggcctgacccccaacttcaagagcaacttcgacctggccgaggatgccaaactgcagctgagcaaggacacctacgacgacgacctggacaacctgctggcccagatcggcgaccagtacgccgacctgtttctggccgccaagaacctgtccgacgccatcctgctgagcgacatcctgagagtgaacaccgagatcaccaaggcccccctgagcgcctctatgatcaagagatacgacgagcaccaccaggacctgaccctgctgaaagctctcgtgcggcagcagctgcctgagaagtacaaagagattttcttcgaccagagcaagaacggctacgccggctacattgacggcggagccagccaggaagagttctacaagttcatcaagcccatcctggaaaagatggacggcaccgaggaactgctcgtgaagctgaagagagaggacctgctgcggaagcagcggaccttcgacaacggcagcatcccccaccagatccacctgggagagctgcacgccattctgcggcggcaggaagatttttacccattcctgaaggacaaccgggaaaagatcgagaagatcctgaccttccgcatcccctactacgtgggccctctggccaggggaaacagcagattcgcctggatgaccagaaagagcgaggaaaccatcaccccctggaacttcgaggaagtggtggacaagggcgcttccgcccagagcttcatcgagcggatgaccaacttcgataagaacctgcccaacgagaaggtgctgcccaagcacagcctgctgtacgagtacttcaccgtgtataacgagctgaccaaagtgaaatacgtgaccgagggaatgagaaagcccgccttcctgagcggcgagcagaaaaaggccatcgtggacctgctgttcaagaccaaccggaaagtgaccgtgaagcagctgaaagaggactacttcaagaaaatcgagtgcttcgactccgtggaaatctccggcgtggaagatcggttcaacgcctccctgggcacataccacgatctgctgaaaattatcaaggacaaggacttcctggacaatgaggaaaacgaggacattctggaagatatcgtgctgaccctgacactgtttgaggacagagagatgatcgaggaacggctgaaaacctatgcccacctgttcgacgacaaagtgatgaagcagctgaagcggcggagatacaccggctggggcaggctgagccggaagctgatcaacggcatccgggacaagcagtccggcaagacaatcctggatttcctgaagtccgacggcttcgccaacagaaacttcatgcagctgatccacgacgacagcctgacctttaaagaggacatccagaaagcccaggtgtccggccagggcgatagcctgcacgagcacattgccaatctggccggcagccccgccattaagaagggcatcctgcagacagtgaaggtggtggacgagctcgtgaaagtgatgggccggcacaagcccgagaacatcgtgatcgaaatggccagagagaaccagaccacccagaagggacagaagaacagccgcgagagaatgaagcggatcgaagagggcatcaaagagctgggcagccagatcctgaaagaacaccccgtggaaaacacccagctgcagaacgagaagctgtacctgtactacctgcagaatgggcgggatatgtacgtggaccaggaactggacatcaaccggctgtccgactacgatgtggacgctatcgtgcctcagagctttctgaaggacgactccatcgacaacaaggtgctgaccagaagcgacaagaaccggggcaagagcgacaacgtgccctccgaagaggtcgtgaagaagatgaagaactactggcggcagctgctgaacgccaagctgattacccagagaaagttcgacaatctgaccaaggccgagagaggcggcctgagcgaactggataaggccggcttcatcaagagacagctggtggaaacccggcagatcacaaagcacgtggcacagatcctggactcccggatgaacactaagtacgacgagaatgacaagctgatccgggaagtgaaagtgatcaccctgaagtccaagctggtgtccgatttccggaaggatttccagttttacaaagtgcgcgagatcaacaactaccaccacgcccacgacgcctacctgaacgccgtcgtgggaaccgccctgatcaaaaagtaccctaagctggaaagcgagttcgtgtacggcgactacaaggtgtacgacgtgcggaagatgatcgccaagagcgagcaggaaatcggcaaggctaccgccaagtacttcttctacagcaacatcatgaactttttcaagaccgagattaccctggccaacggcgagatccggaagcggcctctgatcgagacaaacggcgaaaccggggagatcgtgtgggataagggccgggattttgccaccgtgcggaaagtgctgagcatgccccaagtgaatatcgtgaaaaagaccgaggtgcagacaggcggcttcagcaaagagtctatcctgcccaagaggaacagcgataagctgatcgccagaaagaaggactgggaccctaagaagtacggcggcttcgacagccccaccgtggcctattctgtgctggtggtggccaaagtggaaaagggcaagtccaagaaactgaagagtgtgaaagagctgctggggatcaccatcatggaaagaagcagcttcgagaagaatcccatcgactttctggaagccaagggctacaaagaagtgaaaaaggacctgatcatcaagctgcctaagtactccctgttcgagctggaaaacggccggaagagaatgctggcctctgccggcgaactgcagaagggaaacgaactggccctgccctccaaatatgtgaacttcctgtacctggccagccactatgagaagctgaagggctcccccgaggataatgagcagaaacagctgtttgtggaacagcacaagcactacctggacgagatcatcgagcagatcagcgagttctccaagagagtgatcctggccgacgctaatctggacaaagtgctgtccgcctacaacaagcaccgggataagcccatcagagagcaggccgagaatatcatccacctgtttaccctgaccaatctgggagcccctgccgccttcaagtactttgacaccaccatcgaccggaagaggtacaccagcaccaaagaggtgctggacgccaccctgatccaccagagcatcaccggcctgtacgagacacggatcgacctgtctcagctgggaggtgactccggcggaagctctggtggcagcaagcggaccgccgacggctctgaattcgagagccctaagaagaaaagaaaggtgagcggaggctctagcggcggaagcatcagcagctctaagcacaccctgagccagatgaacaaggtgagcaacatcgtgaaggaacccgagctgcccgacatctacaaggaatttaaggacatcaccgccgacaccaataccgagaagctgcctaagcctattaagggcctggaatttgaagtggaactgacacaggagaactacagactgcctatccggaactatcctctgactccagtcaagatgcaggccatgaacgacgagatcaatcaaggcctgaaaggcggcatcatcagagagagcaaggccatcaacgcctgccctgttatattcgtgcccagaaaggaaggcacactgcgcatggtggtcgactacaggcccctgaacaagtacgtgaagcccaacgtctaccccctgccactgattgaacaactgctggccaagatccagggcagcaccattttcaccaagctggacctgaaaagcgcctaccaccagatcagagtgcgaaagggagatgagcacaagctggccttccggtgccccagaggagttttcgagtacctggtgatgccttacggcatcaagacagcccctgcccactttcagtacttcatcaacacaatcctgggcgaggccaaggaaagccacgtggtgtgctacatggacgacatcctgatccattccaagtccgagtccgaacacgtgaaacatgtgaaggacgtgctgcaaaagctgaagaacgctaatctgatcatcaaccaggccaaatgcgagtttcaccagagccaagtgaagttcctgggctaccacatcagcgagaagggcttaaccccatgtcaggagaacatcgacaaggtgctgcagtggaaacagcctaaaaaccagaaggaactgagacagttcctgggccaggtgaactacctgagaaaattcatccccaaaaccagccagttgacccaccctctgaacaaactcctgaaaaaggatgtcagatggaaatggacccctacccagacccaggctatcgagaatatcaagcaatgtctggtgtctcctcctgtgctgaggcacttcgacttcagcaagaagatcctgcttgagacagacgtttctgatgtggccgtgggagccgtgctgagccagaagcatgatgatgataagtactaccctgtgggctattacagcgctaaaatgagcaaagcccagctgaattattctgtgtccgacaaggagatgctggctatcatcaaaagcctggagcactggcggcactacctggaatctacaatcgagcccttcaagatcctgaccgaccacagaaacctgattggaagaatcacaaacgagagcgaaccagagaacaagcggctggccagatggcagctgttcctgcaggacttcaacttcgagatcaactacagacctggctctgcaaatcacatcgccgatgccctgtctagaatcgtggacgagactgagcctatccctaaggacaacgaagataacagcatcaacttcgtgaaccagatcagcatctctggcggctcaaaaagaaccgccgacggcagcgaattcgagtctcccaagaagaagaggaaagtcggctctggccctgccgctaagagagtgaagctggacgccacagtggtgtccggccaaaagcaggaccgccagggcggagaacgcagaaggtcccagctcgatagggatcagtgtgcctactgcaaggagaagggccactgggccaaagactgcccgaaaaagccgcgcggcccacgcggcccaaggccacaaacatccctcctttaa

SEQ ID NO: 262 - DNA, 5856 bp, synthetic construct
  source 1..5856: mol_type = other DNA
atgaaacggacagccgacggaagcgagttcgagtcaccaaagaagaagcggaaagtcgacaagaagtacagcatcggcctggacatcggcaccaactctgtgggctgggccgtgatcaccgacgagtacaaggtgcccagcaagaaattcaaggtgctgggcaacaccgaccggcacagcatcaagaagaacctgatcggagccctgctgttcgacagcggcgaaacagccgaggccacccggctgaagagaaccgccagaagaagatacaccagacggaagaaccggatctgctatctgcaagagatcttcagcaacgagatggccaaggtggacgacagcttcttccacagactggaagagtccttcctggtggaagaggataagaagcacgagcggcaccccatcttcggcaacatcgtggacgaggtggcctaccacgagaagtaccccaccatctaccacctgagaaagaaactggtggacagcaccgacaaggccgacctgcggctgatctatctggccctggcccacatgatcaagttccggggccacttcctgatcgagggcgacctgaaccccgacaacagcgacgtggacaagctgttcatccagctggtgcagacctacaaccagctgttcgaggaaaaccccatcaacgccagcggcgtggacgccaaggccatcctgtctgccagactgagcaagagcagaaagctggaaaatctgatcgcccagctgcccggcgagaagaagaatggcctgttcggaaacctgattgccctgagcctgggcctgacccccaacttcaagagcaacttcgacctggccgaggatgccaaactgcagctgagcaaggacacctacgacgacgacctggacaacctgctggcccagatcggcgaccagtacgccgacctgtttctggccgccaagaacctgtccgacgccatcctgctgagcgacatcctgagagtgaacaccgagatcaccaaggcccccctgagcgcctctatgatcaagagatacgacgagcaccaccaggacctgaccctgctgaaagctctcgtgcggcagcagctgcctgagaagtacaaagagattttcttcgaccagagcaagaacggctacgccggctacattgacggcggagccagccaggaagagttctacaagttcatcaagcccatcctggaaaagatggacggcaccgaggaactgctcgtgaagctgaagagagaggacctgctgcggaagcagcggaccttcgacaacggcagcatcccccaccagatccacctgggagagctgcacgccattctgcggcggcaggaagatttttacccattcctgaaggacaaccgggaaaagatcgagaagatcctgaccttccgcatcccctactacgtgggccctctggccaggggaaacagcagattcgcctggatgaccagaaagagcgaggaaaccatcaccccctggaacttcgaggaagtggtggacaagggcgcttccgcccagagcttcatcgagcggatgaccaacttcgataagaacctgcccaacgagaaggtgctgcccaagcacagcctgctgtacgagtacttcaccgtgtataacgagctgaccaaagtgaaatacgtgaccgagggaatgagaaagcccgccttcctgagcggcgagcagaaaaaggccatcgtggacctgctgttcaagaccaaccggaaagtgaccgtgaagcagctgaaagaggactacttcaagaaaatcgagtgcttcgactccgtggaaatctccggcgtggaagatcggttcaacgcctccctgggcacataccacgatctgctgaaaattatcaaggacaaggacttcctggacaatgaggaaaacgaggacattctggaagatatcgtgctgaccctgacactgtttgaggacagagagatgatcgaggaacggctgaaaacctatgcccacctgttcgacgacaaagtgatgaagcagctgaagcggcggagatacaccggctggggcaggctgagccggaagctgatcaacggcatccgggacaagcagtccggcaagacaatcctggatttcctgaagtccgacggcttcgccaacagaaacttcatgcagctgatccacgacgacagcctgacctttaaagaggacatccagaaagcccaggtgtccggccagggcgatagcctgcacgagcacattgccaatctggccggcagccccgccattaagaagggcatcctgcagacagtgaaggtggtggacgagctcgtgaaagtgatgggccggcacaagcccgagaacatcgtgatcgaaatggccagagagaaccagaccacccagaagggacagaagaacagccgcgagagaatgaagcggatcgaagagggcatcaaagagctgggcagccagatcctgaaagaacaccccgtggaaaacacccagctgcagaacgagaagctgtacctgtactacctgcagaatgggcgggatatgtacgtggaccaggaactggacatcaaccggctgtccgactacgatgtggacgctatcgtgcctcagagctttctgaaggacgactccatcgacaacaaggtgctgaccagaagcgacaagaaccggggcaagagcgacaacgtgccctccgaagaggtcgtgaagaagatgaagaactactggcggcagctgctgaacgccaagctgattacccagagaaagttcgacaatctgaccaaggccgagagaggcggcctgagcgaactggataaggccggcttcatcaagagacagctggtggaaacccggcagatcacaaagcacgtggcacagatcctggactcccggatgaacactaagtacgacgagaatgacaagctgatccgggaagtgaaagtgatcaccctgaagtccaagctggtgtccgatttccggaaggatttccagttttacaaagtgcgcgagatcaacaactaccaccacgcccacgacgcctacctgaacgccgtcgtgggaaccgccctgatcaaaaagtaccctaagctggaaagcgagttcgtgtacggcgactacaaggtgtacgacgtgcggaagatgatcgccaagagcgagcaggaaatcggcaaggctaccgccaagtacttcttctacagcaacatcatgaactttttcaagaccgagattaccctggccaacggcgagatccggaagcggcctctgatcgagacaaacggcgaaaccggggagatcgtgtgggataagggccgggattttgccaccgtgcggaaagtgctgagcatgccccaagtgaatatcgtgaaaaagaccgaggtgcagacaggcggcttcagcaaagagtctatcctgcccaagaggaacagcgataagctgatcgccagaaagaaggactgggaccctaagaagtacggcggcttcgacagccccaccgtggcctattctgtgctggtggtggccaaagtggaaaagggcaagtccaagaaactgaagagtgtgaaagagctgctggggatcaccatcatggaaagaagcagcttcgagaagaatcccatcgactttctggaagccaagggctacaaagaagtgaaaaaggacctgatcatcaagctgcctaagtactccctgttcgagctggaaaacggccggaagagaatgctggcctctgccggcgaactgcagaagggaaacgaactggccctgccctccaaatatgtgaacttcctgtacctggccagccactatgagaagctgaagggctcccccgaggataatgagcagaaacagctgtttgtggaacagcacaagcactacctggacgagatcatcgagcagatcagcgagttctccaagagagtgatcctggccgacgctaatctggacaaagtgctgtccgcctacaacaagcaccgggataagcccatcagagagcaggccgagaatatcatccacctgtttaccctgaccaatctgggagcccctgccgccttcaagtactttgacaccaccatcgaccggaagaggtacaccagcaccaaagaggtgctggacgccaccctgatccaccagagcatcaccggcctgtacgagacacggatcgacctgtctcagctgggaggtgactccggcggaagctctggtggcagcaagcggaccgccgacggctctgaattcgagagccctaagaagaaaagaaaggtgagcggaggctctagcggcggaagcaccctgaacattgaagacgagtatagactgcatgaaacaagcaaggaacccgacgtgtccctgggctccacctggctgtccgactttccccaggcctgggccgagacaggaggaatgggcctggccgtgcggcaggcacccctgatcatccctctgaaggccacctctacacccgtgagcatcaagcagtaccctatgtctcaggaggccagactgggcatcaagcctcacatccagaggctgctggaccagggcatcctggtgccatgccagagcccctggaacacaccactgctgcccgtgaagaagccaggcaccaatgactatagacccgtgcaggatctgagagaggtgaacaagagggtggaggatatccaccccaacgtgcccaacccttacaatctgctgtccggcctgcccccttctcaccagtggtatacagtgctggacctgaaggatgccttcttttgtctgagactgcaccctaccagccagccactgttcgcctttgagtggagggaccctgagatgggcatctctggccagctgacctggacacgcctgcctcagggcttcaagaatagcccaacactgttttgcgaggccctgcaccgcgacctggcagatttccggatccagcacccagatctgatcctgctgcagtactacgacgatctgctgctggccgccaccagcgagctggattgccagcagggaacacgcgccctgctgcagaccctgggaaacctgggatatagggcatccgccaagaaggcccagatctgtcagaagcaggtgaagtacctgggctatctgctgaaggagggccagagatggctgacagaggccaggaaggagacagtgatgggccagccaacacccaagaccccaagacagctgagggagttcctgggcaaagcaggattttgcaggctgttcatcccaggattcgcagagatggcagcacctctgtacccactgaccaagccgggcaccctgtttaattggggccctgaccagcagaaggcctatcaggagatcaagcaggccctgctgacagcaccagccctgggcctgccagacctgaccaagcctttcgagctgtttgtggatgagaagcagggctacgccaagggcgtgctgacccagaagctgggaccatggagacggcccgtggcctatctgtccaagaagctggacccagtggcagcaggatggccaccatgcctgaggatggtggcagcaatcgccgtgctgacaaaggatgccggcaagctgaccatgggacagccactggtcatcctggcaccacacgcagtggaggccctggtgaagcagcctccagatcgctggctgtctaacgcccggatgacacactaccaggccctgctgctggacaccgatcgcgtgcagtttggccctgtggtggccctgaatccagccaccctgctgcctctgccagaggagggcctgcagcacaactgtctggactctggcggctcaaaaagaaccgccgacggcagcgaattcgagtctcccaagaagaagaggaaagtcggctctggccctgccgctaagagagtgaagctggactaa

SEQ ID NO: 263 - DNA, 6024 bp, synthetic construct
  source 1..6024: mol_type = other DNA
atgaaacggacagccgacggaagcgagttcgagtcaccaaagaagaagcggaaagtcgacaagaagtacagcatcggcctggacatcggcaccaactctgtgggctgggccgtgatcaccgacgagtacaaggtgcccagcaagaaattcaaggtgctgggcaacaccgaccggcacagcatcaagaagaacctgatcggagccctgctgttcgacagcggcgaaacagccgaggccacccggctgaagagaaccgccagaagaagatacaccagacggaagaaccggatctgctatctgcaagagatcttcagcaacgagatggccaaggtggacgacagcttcttccacagactggaagagtccttcctggtggaagaggataagaagcacgagcggcaccccatcttcggcaacatcgtggacgaggtggcctaccacgagaagtaccccaccatctaccacctgagaaagaaactggtggacagcaccgacaaggccgacctgcggctgatctatctggccctggcccacatgatcaagttccggggccacttcctgatcgagggcgacctgaaccccgacaacagcgacgtggacaagctgttcatccagctggtgcagacctacaaccagctgttcgaggaaaaccccatcaacgccagcggcgtggacgccaaggccatcctgtctgccagactgagcaagagcagaaagctggaaaatctgatcgcccagctgcccggcgagaagaagaatggcctgttcggaaacctgattgccctgagcctgggcctgacccccaacttcaagagcaacttcgacctggccgaggatgccaaactgcagctgagcaaggacacctacgacgacgacctggacaacctgctggcccagatcggcgaccagtacgccgacctgtttctggccgccaagaacctgtccgacgccatcctgctgagcgacatcctgagagtgaacaccgagatcaccaaggcccccctgagcgcctctatgatcaagagatacgacgagcaccaccaggacctgaccctgctgaaagctctcgtgcggcagcagctgcctgagaagtacaaagagattttcttcgaccagagcaagaacggctacgccggctacattgacggcggagccagccaggaagagttctacaagttcatcaagcccatcctggaaaagatggacggcaccgaggaactgctcgtgaagctgaagagagaggacctgctgcggaagcagcggaccttcgacaacggcagcatcccccaccagatccacctgggagagctgcacgccattctgcggcggcaggaagatttttacccattcctgaaggacaaccgggaaaagatcgagaagatcctgaccttccgcatcccctactacgtgggccctctggccaggggaaacagcagattcgcctggatgaccagaaagagcgaggaaaccatcaccccctggaacttcgaggaagtggtggacaagggcgcttccgcccagagcttcatcgagcggatgaccaacttcgataagaacctgcccaacgagaaggtgctgcccaagcacagcctgctgtacgagtacttcaccgtgtataacgagctgaccaaagtgaaatacgtgaccgagggaatgagaaagcccgccttcctgagcggcgagcagaaaaaggccatcgtggacctgctgttcaagaccaaccggaaagtgaccgtgaagcagctgaaagaggactacttcaagaaaatcgagtgcttcgactccgtggaaatctccggcgtggaagatcggttcaacgcctccctgggcacataccacgatctgctgaaaattatcaaggacaaggacttcctggacaatgaggaaaacgaggacattctggaagatatcgtgctgaccctgacactgtttgaggacagagagatgatcgaggaacggctgaaaacctatgcccacctgttcgacgacaaagtgatgaagcagctgaagcggcggagatacaccggctggggcaggctgagccggaagctgatcaacggcatccgggacaagcagtccggcaagacaatcctggatttcctgaagtccgacggcttcgccaacagaaacttcatgcagctgatccacgacgacagcctgacctttaaagaggacatccagaaagcccaggtgtccggccagggcgatagcctgcacgagcacattgccaatctggccggcagccccgccattaagaagggcatcctgcagacagtgaaggtggtggacgagctcgtgaaagtgatgggccggcacaagcccgagaacatcgtgatcgaaatggccagagagaaccagaccacccagaagggacagaagaacagccgcgagagaatgaagcggatcgaagagggcatcaaagagctgggcagccagatcctgaaagaacaccccgtggaaaacacccagctgcagaacgagaagctgtacctgtactacctgcagaatgggcgggatatgtacgtggaccaggaactggacatcaaccggctgtccgactacgatgtggacgctatcgtgcctcagagctttctgaaggacgactccatcgacaacaaggtgctgaccagaagcgacaagaaccggggcaagagcgacaacgtgccctccgaagaggtcgtgaagaagatgaagaactactggcggcagctgctgaacgccaagctgattacccagagaaagttcgacaatctgaccaaggccgagagaggcggcctgagcgaactggataaggccggcttcatcaagagacagctggtggaaacccggcagatcacaaagcacgtggcacagatcctggactcccggatgaacactaagtacgacgagaatgacaagctgatccgggaagtgaaagtgatcaccctgaagtccaagctggtgtccgatttccggaaggatttccagttttacaaagtgcgcgagatcaacaactaccaccacgcccacgacgcctacctgaacgccgtcgtgggaaccgccctgatcaaaaagtaccctaagctggaaagcgagttcgtgtacggcgactacaaggtgtacgacgtgcggaagatgatcgccaagagcgagcaggaaatcggcaaggctaccgccaagtacttcttctacagcaacatcatgaactttttcaagaccgagattaccctggccaacggcgagatccggaagcggcctctgatcgagacaaacggcgaaaccggggagatcgtgtgggataagggccgggattttgccaccgtgcggaaagtgctgagcatgccccaagtgaatatcgtgaaaaagaccgaggtgcagacaggcggcttcagcaaagagtctatcctgcccaagaggaacagcgataagctgatcgccagaaagaaggactgggaccctaagaagtacggcggcttcgacagccccaccgtggcctattctgtgctggtggtggccaaagtggaaaagggcaagtccaagaaactgaagagtgtgaaagagctgctggggatcaccatcatggaaagaagcagcttcgagaagaatcccatcgactttctggaagccaagggctacaaagaagtgaaaaaggacctgatcatcaagctgcctaagtactccctgttcgagctggaaaacggccggaagagaatgctggcctctgccggcgaactgcagaagggaaacgaactggccctgccctccaaatatgtgaacttcctgtacctggccagccactatgagaagctgaagggctcccccgaggataatgagcagaaacagctgtttgtggaacagcacaagcactacctggacgagatcatcgagcagatcagcgagttctccaagagagtgatcctggccgacgctaatctggacaaagtgctgtccgcctacaacaagcaccgggataagcccatcagagagcaggccgagaatatcatccacctgtttaccctgaccaatctgggagcccctgccgccttcaagtactttgacaccaccatcgaccggaagaggtacaccagcaccaaagaggtgctggacgccaccctgatccaccagagcatcaccggcctgtacgagacacggatcgacctgtctcagctgggaggtgactccggcggaagctctggtggcagcaagcggaccgccgacggctctgaattcgagagccctaagaagaaaagaaaggtgagcggaggctctagcggcggaagcaccctgaacattgaagacgagtatagactgcatgaaacaagcaaggaacccgacgtgtccctgggctccacctggctgtccgactttccccaggcctgggccgagacaggaggaatgggcctggccgtgcggcaggcacccctgatcatccctctgaaggccacctctacacccgtgagcatcaagcagtaccctatgtctcaggaggccagactgggcatcaagcctcacatccagaggctgctggaccagggcatcctggtgccatgccagagcccctggaacacaccactgctgcccgtgaagaagccaggcaccaatgactatagacccgtgcaggatctgagagaggtgaacaagagggtggaggatatccaccccaacgtgcccaacccttacaatctgctgtccggcctgcccccttctcaccagtggtatacagtgctggacctgaaggatgccttcttttgtctgagactgcaccctaccagccagccactgttcgcctttgagtggagggaccctgagatgggcatctctggccagctgacctggacacgcctgcctcagggcttcaagaatagcccaacactgttttgcgaggccctgcaccgcgacctggcagatttccggatccagcacccagatctgatcctgctgcagtactacgacgatctgctgctggccgccaccagcgagctggattgccagcagggaacacgcgccctgctgcagaccctgggaaacctgggatatagggcatccgccaagaaggcccagatctgtcagaagcaggtgaagtacctgggctatctgctgaaggagggccagagatggctgacagaggccaggaaggagacagtgatgggccagccaacacccaagaccccaagacagctgagggagttcctgggcaaagcaggattttgcaggctgttcatcccaggattcgcagagatggcagcacctctgtacccactgaccaagccgggcaccctgtttaattggggccctgaccagcagaaggcctatcaggagatcaagcaggccctgctgacagcaccagccctgggcctgccagacctgaccaagcctttcgagctgtttgtggatgagaagcagggctacgccaagggcgtgctgacccagaagctgggaccatggagacggcccgtggcctatctgtccaagaagctggacccagtggcagcaggatggccaccatgcctgaggatggtggcagcaatcgccgtgctgacaaaggatgccggcaagctgaccatgggacagccactggtcatcctggcaccacacgcagtggaggccctggtgaagcagcctccagatcgctggctgtctaacgcccggatgacacactaccaggccctgctgctggacaccgatcgcgtgcagtttggccctgtggtggccctgaatccagccaccctgctgcctctgccagaggagggcctgcagcacaactgtctggactctggcggctcaaaaagaaccgccgacggcagcgaattcgagtctcccaagaagaagaggaaagtcggctctggccctgccgctaagagagtgaagctggacgccacagtggtgtccggccaaaagcaggaccgccagggcggagaacgcagaaggtcccagctcgatagggatcagtgtgcctactgcaaggagaagggccactgggccaaagactgcccgaaaaagccgcgcggcccacgcggcccaaggccacaaacatccctcctttaa

SEQ ID NO: 264 - DNA, 5856 bp, synthetic construct
  source 1..5856: mol_type = other DNA
atgaaacggacagccgacggaagcgagttcgagtcaccaaagaagaagcggaaagtcgacaagaagtacagcatcggcctggacatcggcaccaactctgtgggctgggccgtgatcaccgacgagtacaaggtgcccagcaagaaattcaaggtgctgggcaacaccgaccggcacagcatcaagaagaacctgatcggagccctgctgttcgacagcggcgaaacagccgaggccacccggctgaagagaaccgccagaagaagatacaccagacggaagaaccggatctgctatctgcaagagatcttcagcaacgagatggccaaggtggacgacagcttcttccacagactggaagagtccttcctggtggaagaggataagaagcacgagcggcaccccatcttcggcaacatcgtggacgaggtggcctaccacgagaagtaccccaccatctaccacctgagaaagaaactggtggacagcaccgacaaggccgacctgcggctgatctatctggccctggcccacatgatcaagttccggggccacttcctgatcgagggcgacctgaaccccgacaacagcgacgtggacaagctgttcatccagctggtgcagacctacaaccagctgttcgaggaaaaccccatcaacgccagcggcgtggacgccaaggccatcctgtctgccagactgagcaagagcagaaagctggaaaatctgatcgcccagctgcccggcgagaagaagaatggcctgttcggaaacctgattgccctgagcctgggcctgacccccaacttcaagagcaacttcgacctggccgaggatgccaaactgcagctgagcaaggacacctacgacgacgacctggacaacctgctggcccagatcggcgaccagtacgccgacctgtttctggccgccaagaacctgtccgacgccatcctgctgagcgacatcctgagagtgaacaccgagatcaccaaggcccccctgagcgcctctatgatcaagagatacgacgagcaccaccaggacctgaccctgctgaaagctctcgtgcggcagcagctgcctgagaagtacaaagagattttcttcgaccagagcaagaacggctacgccggctacattgacggcggagccagccaggaagagttctacaagttcatcaagcccatcctggaaaagatggacggcaccgaggaactgctcgtgaagctgaagagagaggacctgctgcggaagcagcggaccttcgacaacggcagcatcccccaccagatccacctgggagagctgcacgccattctgcggcggcaggaagatttttacccattcctgaaggacaaccgggaaaagatcgagaagatcctgaccttccgcatcccctactacgtgggccctctggccaggggaaacagcagattcgcctggatgaccagaaagagcgaggaaaccatcaccccctggaacttcgaggaagtggtggacaagggcgcttccgcccagagcttcatcgagcggatgaccaacttcgataagaacctgcccaacgagaaggtgctgcccaagcacagcctgctgtacgagtacttcaccgtgtataacgagctgaccaaagtgaaatacgtgaccgagggaatgagaaagcccgccttcctgagcggcgagcagaaaaaggccatcgtggacctgctgttcaagaccaaccggaaagtgaccgtgaagcagctgaaagaggactacttcaagaaaatcgagtgcttcgactccgtggaaatctccggcgtggaagatcggttcaacgcctccctgggcacataccacgatctgctgaaaattatcaaggacaaggacttcctggacaatgaggaaaacgaggacattctggaagatatcgtgctgaccctgacactgtttgaggacagagagatgatcgaggaacggctgaaaacctatgcccacctgttcgacgacaaagtgatgaagcagctgaagcggcggagatacaccggctggggcaggctgagccggaagctgatcaacggcatccgggacaagcagtccggcaagacaatcctggatttcctgaagtccgacggcttcgccaacagaaacttcatgcagctgatccacgacgacagcctgacctttaaagaggacatccagaaagcccaggtgtccggccagggcgatagcctgcacgagcacattgccaatctggccggcagccccgccattaagaagggcatcctgcagacagtgaaggtggtggacgagctcgtgaaagtgatgggccggcacaagcccgagaacatcgtgatcgaaatggccagagagaaccagaccacccagaagggacagagaaacagccgcgagagaatgaagcggatcgaagagggcatcaaagagctgggcagccagatcctgaaagaacaccccgtggaaaacacccagctgcagaacgagaagctgtacctgtactacctgcagaatgggcgggatatgtacgtggaccaggaactggacatcaaccggctgtccgactacgatgtggacgctatcgtgcctcagagctttctgaaggacgactccatcgacaacaaggtgctgaccagaagcgacaagaaccggggcaagagcgacaacgtgccctccgaagaggtcgtgaagaagatgaagaactactggcggcagctgctgaacgccaagctgattacccagagaaagttcgacaatctgaccaaggccgagagaggcggcctgagcgaactggataaggccggcttcatcgctagacagctggtggaaacccggcagatcacaaagcacgtggcacagatcctggactcccggatgaacactaagtacgacgagaatgacaagctgatccgggaagtgaaagtgatcaccctgaagtccaagctggtgtccgatttccggaaggatttccagttttacaaagtgcgcgagatcaacaactaccaccacgcccacgacgcctacctgaacgccgtcgtgggaaccgccctgatcaaaaagtaccctaagctggaaagcgagttcgtgtacggcgactacaaggtgtacgacgtgcggaagatgatcgccaagagcgagcaggaaatcggcaaggctaccgccaagtacttcttctacagcaacatcatgaactttttcaagaccgagattaccctggccaacggcgagatccggaagcggcctctgatcgagacaaacggcgaaaccggggagatcgtgtgggataagggccgggattttgccaccgtgcggaaagtgctgagcatgccccaagtgaatatcgtgaaaaagaccgaggtgcagacaggcggcttcagcaaagagtctatcctgcccaagaggaacagcgataagctgatcgccagaaagaaggactgggaccctaagaagtacggcggcttcgacagccccaccgtggcctattctgtgctggtggtggccaaagtggaaaagggcaagtccaagaaactgaagagtgtgaaagagctgctggggatcaccatcatggaaagaagcagcttcgagaagaatcccatcgactttctggaagccaagggctacaaagaagtgaaaaaggacctgatcatcaagctgcctaagtactccctgttcgagctggaaaacggccggaagagaatgctggcctctgccggcgaactgcagaagggaaacgaactggccctgccctccaaatatgtgaacttcctgtacctggccagccactatgagaagctgaagggctcccccgaggataatgagcagaaacagctgtttgtggaacagcacaagcactacctggacgagatcatcgagcagatcagcgagttctccaagagagtgatcctggccgacgctaatctggacaaagtgctgtccgcctacaacaagcaccgggataagcccatcagagagcaggccgagaatatcatccacctgtttaccctgaccaatctgggagcccctgccgccttcaagtactttgacaccaccatcgaccggaagaggtacaccagcaccaaagaggtgctggacgccaccctgatccaccagagcatcaccggcctgtacgagacacggatcgacctgtctcagctgggaggtgactccggcggaagctctggtggcagcaagcggaccgccgacggctctgaattcgagagccctaagaagaaaagaaaggtgagcggaggctctagcggcggaagcaccctgaacattgaagacgagtatagactgcatgaaacaagcaaggaacccgacgtgtccctgggctccacctggctgtccgactttccccaggcctgggccgagacaggaggaatgggcctggccgtgcggcaggcacccctgatcatccctctgaaggccacctctacacccgtgagcatcaagcagtaccctatgtctcaggaggccagactgggcatcaagcctcacatccagaggctgctggaccagggcatcctggtgccatgccagagcccctggaacacaccactgctgcccgtgaagaagccaggcaccaatgactatagacccgtgcaggatctgagagaggtgaacaagagggtggaggatatccaccccaacgtgcccaacccttacaatctgctgtccggcctgcccccttctcaccagtggtatacagtgctggacctgaaggatgccttcttttgtctgagactgcaccctaccagccagccactgttcgcctttgagtggagggaccctgagatgggcatctctggccagctgacctggacacgcctgcctcagggcttcaagaatagcccaacactgttttgcgaggccctgcaccgcgacctggcagatttccggatccagcacccagatctgatcctgctgcagtactacgacgatctgctgctggccgccaccagcgagctggattgccagcagggaacacgcgccctgctgcagaccctgggaaacctgggatatagggcatccgccaagaaggcccagatctgtcagaagcaggtgaagtacctgggctatctgctgaaggagggccagagatggctgacagaggccaggaaggagacagtgatgggccagccaacacccaagaccccaagacagctgagggagttcctgggcaaagcaggattttgcaggctgttcatcccaggattcgcagagatggcagcacctctgtacccactgaccaagccgggcaccctgtttaattggggccctgaccagcagaaggcctatcaggagatcaagcaggccctgctgacagcaccagccctgggcctgccagacctgaccaagcctttcgagctgtttgtggatgagaagcagggctacgccaagggcgtgctgacccagaagctgggaccatggagacggcccgtggcctatctgtccaagaagctggacccagtggcagcaggatggccaccatgcctgaggatggtggcagcaatcgccgtgctgacaaaggatgccggcaagctgaccatgggacagccactggtcatcctggcaccacacgcagtggaggccctggtgaagcagcctccagatcgctggctgtctaacgcccggatgacacactaccaggccctgctgctggacaccgatcgcgtgcagtttggccctgtggtggccctgaatccagccaccctgctgcctctgccagaggagggcctgcagcacaactgtctggactctggcggctcaaaaagaaccgccgacggcagcgaattcgagtctcccaagaagaagaggaaagtcggctctggccctgccgctaagagagtgaagctggactaa

SEQ ID NO: 265 - DNA, 6024 bp, synthetic construct
  source 1..6024: mol_type = other DNA
atgaaacggacagccgacggaagcgagttcgagtcaccaaagaagaagcggaaagtcgacaagaagtacagcatcggcctggacatcggcaccaactctgtgggctgggccgtgatcaccgacgagtacaaggtgcccagcaagaaattcaaggtgctgggcaacaccgaccggcacagcatcaagaagaacctgatcggagccctgctgttcgacagcggcgaaacagccgaggccacccggctgaagagaaccgccagaagaagatacaccagacggaagaaccggatctgctatctgcaagagatcttcagcaacgagatggccaaggtggacgacagcttcttccacagactggaagagtccttcctggtggaagaggataagaagcacgagcggcaccccatcttcggcaacatcgtggacgaggtggcctaccacgagaagtaccccaccatctaccacctgagaaagaaactggtggacagcaccgacaaggccgacctgcggctgatctatctggccctggcccacatgatcaagttccggggccacttcctgatcgagggcgacctgaaccccgacaacagcgacgtggacaagctgttcatccagctggtgcagacctacaaccagctgttcgaggaaaaccccatcaacgccagcggcgtggacgccaaggccatcctgtctgccagactgagcaagagcagaaagctggaaaatctgatcgcccagctgcccggcgagaagaagaatggcctgttcggaaacctgattgccctgagcctgggcctgacccccaacttcaagagcaacttcgacctggccgaggatgccaaactgcagctgagcaaggacacctacgacgacgacctggacaacctgctggcccagatcggcgaccagtacgccgacctgtttctggccgccaagaacctgtccgacgccatcctgctgagcgacatcctgagagtgaacaccgagatcaccaaggcccccctgagcgcctctatgatcaagagatacgacgagcaccaccaggacctgaccctgctgaaagctctcgtgcggcagcagctgcctgagaagtacaaagagattttcttcgaccagagcaagaacggctacgccggctacattgacggcggagccagccaggaagagttctacaagttcatcaagcccatcctggaaaagatggacggcaccgaggaactgctcgtgaagctgaagagagaggacctgctgcggaagcagcggaccttcgacaacggcagcatcccccaccagatccacctgggagagctgcacgccattctgcggcggcaggaagatttttacccattcctgaaggacaaccgggaaaagatcgagaagatcctgaccttccgcatcccctactacgtgggccctctggccaggggaaacagcagattcgcctggatgaccagaaagagcgaggaaaccatcaccccctggaacttcgaggaagtggtggacaagggcgcttccgcccagagcttcatcgagcggatgaccaacttcgataagaacctgcccaacgagaaggtgctgcccaagcacagcctgctgtacgagtacttcaccgtgtataacgagctgaccaaagtgaaatacgtgaccgagggaatgagaaagcccgccttcctgagcggcgagcagaaaaaggccatcgtggacctgctgttcaagaccaaccggaaagtgaccgtgaagcagctgaaagaggactacttcaagaaaatcgagtgcttcgactccgtggaaatctccggcgtggaagatcggttcaacgcctccctgggcacataccacgatctgctgaaaattatcaaggacaaggacttcctggacaatgaggaaaacgaggacattctggaagatatcgtgctgaccctgacactgtttgaggacagagagatgatcgaggaacggctgaaaacctatgcccacctgttcgacgacaaagtgatgaagcagctgaagcggcggagatacaccggctggggcaggctgagccggaagctgatcaacggcatccgggacaagcagtccggcaagacaatcctggatttcctgaagtccgacggcttcgccaacagaaacttcatgcagctgatccacgacgacagcctgacctttaaagaggacatccagaaagcccaggtgtccggccagggcgatagcctgcacgagcacattgccaatctggccggcagccccgccattaagaagggcatcctgcagacagtgaaggtggtggacgagctcgtgaaagtgatgggccggcacaagcccgagaacatcgtgatcgaaatggccagagagaaccagaccacccagaagggacagagaaacagccgcgagagaatgaagcggatcgaagagggcatcaaagagctgggcagccagatcctgaaagaacaccccgtggaaaacacccagctgcagaacgagaagctgtacctgtactacctgcagaatgggcgggatatgtacgtggaccaggaactggacatcaaccggctgtccgactacgatgtggacgctatcgtgcctcagagctttctgaaggacgactccatcgacaacaaggtgctgaccagaagcgacaagaaccggggcaagagcgacaacgtgccctccgaagaggtcgtgaagaagatgaagaactactggcggcagctgctgaacgccaagctgattacccagagaaagttcgacaatctgaccaaggccgagagaggcggcctgagcgaactggataaggccggcttcatcgctagacagctggtggaaacccggcagatcacaaagcacgtggcacagatcctggactcccggatgaacactaagtacgacgagaatgacaagctgatccgggaagtgaaagtgatcaccctgaagtccaagctggtgtccgatttccggaaggatttccagttttacaaagtgcgcgagatcaacaactaccaccacgcccacgacgcctacctgaacgccgtcgtgggaaccgccctgatcaaaaagtaccctaagctggaaagcgagttcgtgtacggcgactacaaggtgtacgacgtgcggaagatgatcgccaagagcgagcaggaaatcggcaaggctaccgccaagtacttcttctacagcaacatcatgaactttttcaagaccgagattaccctggccaacggcgagatccggaagcggcctctgatcgagacaaacggcgaaaccggggagatcgtgtgggataagggccgggattttgccaccgtgcggaaagtgctgagcatgccccaagtgaatatcgtgaaaaagaccgaggtgcagacaggcggcttcagcaaagagtctatcctgcccaagaggaacagcgataagctgatcgccagaaagaaggactgggaccctaagaagtacggcggcttcgacagccccaccgtggcctattctgtgctggtggtggccaaagtggaaaagggcaagtccaagaaactgaagagtgtgaaagagctgctggggatcaccatcatggaaagaagcagcttcgagaagaatcccatcgactttctggaagccaagggctacaaagaagtgaaaaaggacctgatcatcaagctgcctaagtactccctgttcgagctggaaaacggccggaagagaatgctggcctctgccggcgaactgcagaagggaaacgaactggccctgccctccaaatatgtgaacttcctgtacctggccagccactatgagaagctgaagggctcccccgaggataatgagcagaaacagctgtttgtggaacagcacaagcactacctggacgagatcatcgagcagatcagcgagttctccaagagagtgatcctggccgacgctaatctggacaaagtgctgtccgcctacaacaagcaccgggataagcccatcagagagcaggccgagaatatcatccacctgtttaccctgaccaatctgggagcccctgccgccttcaagtactttgacaccaccatcgaccggaagaggtacaccagcaccaaagaggtgctggacgccaccctgatccaccagagcatcaccggcctgtacgagacacggatcgacctgtctcagctgggaggtgactccggcggaagctctggtggcagcaagcggaccgccgacggctctgaattcgagagccctaagaagaaaagaaaggtgagcggaggctctagcggcggaagcaccctgaacattgaagacgagtatagactgcatgaaacaagcaaggaacccgacgtgtccctgggctccacctggctgtccgactttccccaggcctgggccgagacaggaggaatgggcctggccgtgcggcaggcacccctgatcatccctctgaaggccacctctacacccgtgagcatcaagcagtaccctatgtctcaggaggccagactgggcatcaagcctcacatccagaggctgctggaccagggcatcctggtgccatgccagagcccctggaacacaccactgctgcccgtgaagaagccaggcaccaatgactatagacccgtgcaggatctgagagaggtgaacaagagggtggaggatatccaccccaacgtgcccaacccttacaatctgctgtccggcctgcccccttctcaccagtggtatacagtgctggacctgaaggatgccttcttttgtctgagactgcaccctaccagccagccactgttcgcctttgagtggagggaccctgagatgggcatctctggccagctgacctggacacgcctgcctcagggcttcaagaatagcccaacactgttttgcgaggccctgcaccgcgacctggcagatttccggatccagcacccagatctgatcctgctgcagtactacgacgatctgctgctggccgccaccagcgagctggattgccagcagggaacacgcgccctgctgcagaccctgggaaacctgggatatagggcatccgccaagaaggcccagatctgtcagaagcaggtgaagtacctgggctatctgctgaaggagggccagagatggctgacagaggccaggaaggagacagtgatgggccagccaacacccaagaccccaagacagctgagggagttcctgggcaaagcaggattttgcaggctgttcatcccaggattcgcagagatggcagcacctctgtacccactgaccaagccgggcaccctgtttaattggggccctgaccagcagaaggcctatcaggagatcaagcaggccctgctgacagcaccagccctgggcctgccagacctgaccaagcctttcgagctgtttgtggatgagaagcagggctacgccaagggcgtgctgacccagaagctgggaccatggagacggcccgtggcctatctgtccaagaagctggacccagtggcagcaggatggccaccatgcctgaggatggtggcagcaatcgccgtgctgacaaaggatgccggcaagctgaccatgggacagccactggtcatcctggcaccacacgcagtggaggccctggtgaagcagcctccagatcgctggctgtctaacgcccggatgacacactaccaggccctgctgctggacaccgatcgcgtgcagtttggccctgtggtggccctgaatccagccaccctgctgcctctgccagaggagggcctgcagcacaactgtctggactctggcggctcaaaaagaaccgccgacggcagcgaattcgagtctcccaagaagaagaggaaagtcggctctggccctgccgctaagagagtgaagctggacgccacagtggtgtccggccaaaagcaggaccgccagggcggagaacgcagaaggtcccagctcgatagggatcagtgtgcctactgcaaggagaagggccactgggccaaagactgcccgaaaaagccgcgcggcccacgcggcccaaggccacaaacatccctcctttaa

SEQ ID NO: 266 - DNA, 5856 bp, synthetic construct
  source 1..5856: mol_type = other DNA
atgaaacggacagccgacggaagcgagttcgagtcaccaaagaagaagcggaaagtcgacaagaagtacagcatcggcctggacatcggcaccaactctgtgggctgggccgtgatcaccgacgagtacaaggtgcccagcaagaaattcaaggtgctgggcaacaccgaccggcacagcatcaagaagaacctgatcggagccctgctgttcgacagcggcgaaacagccgaggccacccggctgaagagaaccgccagaagaagatacaccagacggaagaaccggatctgctatctgcaagagatcttcagcaacgagatggccaaggtggacgacagcttcttccggagactggaagagtccttcctggtggaagaggataagaagcacgagcggcaccccatcttcggcaacatcgtggacgaggtggcctaccacgagaagtaccccaccatctaccacctgagaaagaaactggtggacagcaccgacaaggccgacctgcggctgatctatctggccctggcccacatgatcaagttccggggccacttcctgatcgagggcgacctgaaccccgacaacagcgacgtggacaagctgttcatccagctggtgcagacctacaaccagctgttcgaggaaaaccccatcaacgccagcggcgtggacgccaaggccatcctgtctgccagactgagcaagagcagaaagctggaaaatctgatcgcccagctgcccggcgagaagaagaatggcctgttcggaaacctgattgccctgagcctgggcctgacccccaacttcaagagcaacttcgacctggccgaggatgccaaactgcagctgagcaaggacacctacgacgacgacctggacaacctgctggcccagatcggcgaccagtacgccgacctgtttctggccgccaagaacctgtccgacgccatcctgctgagcgacatcctgagagtgaacaccgagatcaccaaggcccccctgagcgcctctatgatcaagagatacgacgagcaccaccaggacctgaccctgctgaaagctctcgtgcggcagcagctgcctgagaagtacaaagagattttcttcgaccagagcaagaacggctacgccggctacattgacggcggagccagccaggaagagttctacaagttcatcaagcccatcctggaaaagatggacggcaccgaggaactgctcgtgaagctgaagagagaggacctgctgcggaagcagcggaccttcgacaacggcagcatcccccaccagatccacctgggagagctgcacgccattctgcggcggcaggaagatttttacccattcctgaaggacaaccgggaaaagatcgagaagatcctgaccttccgcatcccctactacgtgggccctctggccaggggaaacagcagattcgcctggatgaccagaaagagcgagaaaaccatcaccccctggaacttcgaggaagtggtggacaagggcgcttccgcccagagcttcatcgagcggatgaccaacttcgataagaacctgcccaacgagaaggtgctgcccaagcacagcctgctgtacgagtacttcaccgtgtataacgagctgaccaaagtgaaatacgtgaccgagggaatgagaaagcccgccttcctgagcggcgagcagaaaaaggccatcgtggacctgctgttcaagaccaaccggaaagtgaccgtgaagcagctgaaagaggactacttcaagaaaatcgagtgcttcgactccgtggaaatctccggcgtggaagatcggttcaacgcctccctgggcacataccacgatctgctgaaaattatcaaggacaaggacttcctggacaatgaggaaaacgaggacattctggaagatatcgtgctgaccctgacactgtttgaggacagagagatggtggaggaacggctgaaaacctatgcccacctgttcgacaacaaagtgatgaagcagctgaagcggcggagatacaccggctggggcaggctgagccggaagctgatcaacggcatccgggacaagcagtccggcaagacaatcctggatttcctgaagtccgacggcttcgccaacagaaacttcatgcagctgatccacgacgacagcctgacctttaaagaggacatccagaaagcccaggtgtccggccagggcgatagcctgtacgagcacattgccaatctggccggcagccccgccattaagaagggcatcctgcagacagtgaaggtggtggacgagctcgtgaaagtgatgggccggcacaagcccgagaacatcgtgatcgaaatggccagagagaaccagaccacccagaagggacagaagaacagccgcgagagaatgaagcggatcgaagagggcatcaaagagctgggcagccagatcctgaaagaacaccccgtggaaaacacccagctgcagaacgagaagctgtacctgtactacctgcagaatgggcgggatatgtacgtggaccaggaactggacatcaaccggctgtccgactacgatgtggacgctatcgtgcctcagagctttctgaaggacgactccatcgacaacaaggtgctgaccagaagcgacaagaaccggggcaagagcgacaacgtgccctccgaagaggtcgtgaagaagatgaagaactactggcggcagctgctgaacgccaagctgattacccagagaaagttcgacaatctgaccaaggccgagagaggcggcctgagcgaactggataaggccggcttcatcgccagacagctggtggaaacccggcagatcacaaagcacgtggcacagatcctggactcccggatgaacactaagtacgacgagaatgacaagctgatccgggaagtgaaagtgatcaccctgaagtccaagctggtgtccgatttccggaaggatttccagttttacaaagtgcgcgagatcaacaactaccaccacgcccacgacgcctacctgaacgccgtcgtgggaaccgccctgatcaaaaagtaccctaagctggaaagcgagttcgtgtacggcgactacaaggtgtacgacgtgcggaagatgatcgccaagagcgagcaggaaatcggcaaggctaccgccaagtacttcttctacagcaacatcatgaactttttcaagaccgagattaccctggccaacggcgagatccggaagcggcctctgatcgagacaaacggcgaaaccggggagatcgtgtgggataagggccgggattttgccaccgtgcggaaagtgctgagcatgccccaagtgaatatcgtgaaaaagaccgaggtgcagacaggcggcttcagcaaagagtctatcctgcccaagaggaacagcgataagctgatcgccagaaagaaggactgggaccctaagaagtacggcggcttcgacagccccaccgtggcctattctgtgctggtggtggccaaagtggaaaagggcaagtccaagaaactgaagagtgtgaaagagctgctggggatcaccatcatggaaagaagcagcttcgagaagaatcccatcgactttctggaagccaagggctacaaagaagtgaaaaaggacctgatcatcaagctgcctaagtactccctgttcgagctggaaaacggccggaagagaatgctggcctctgccggcgaactgcagaagggaaacgaactggccctgccctccaaatatgtgaacttcctgtacctggccagccactatgagaagctgaagggctcccccgaggataatgagcagaaacagctgtttgtggaacagcacaagcactacctggacgagatcatcgagcagatcagcgagttctccaagagagtgatcctggccgacgctaatctggacaaagtgctgtccgcctacaacaagcaccgggataagcccatcagagagcaggccgagaatatcatccacctgtttaccctgaccaatctgggagcccctgccgccttcaagtactttgacaccaccatcgaccggaagaggtacaccagcaccaaagaggtgctggacgccaccctgatccaccagagcatcaccggcctgtacgagacacggatcgacctgtctcagctgggaggtgactccggcggaagctctggtggcagcaagcggaccgccgacggctctgaattcgagagccctaagaagaaaagaaaggtgagcggaggctctagcggcggaagcaccctgaacattgaagacgagtatagactgcatgaaacaagcaaggaacccgacgtgtccctgggctccacctggctgtccgactttccccaggcctgggccgagacaggaggaatgggcctggccgtgcggcaggcacccctgatcatccctctgaaggccacctctacacccgtgagcatcaagcagtaccctatgtctcaggaggccagactgggcatcaagcctcacatccagaggctgctggaccagggcatcctggtgccatgccagagcccctggaacacaccactgctgcccgtgaagaagccaggcaccaatgactatagacccgtgcaggatctgagagaggtgaacaagagggtggaggatatccaccccaacgtgcccaacccttacaatctgctgtccggcctgcccccttctcaccagtggtatacagtgctggacctgaaggatgccttcttttgtctgagactgcaccctaccagccagccactgttcgcctttgagtggagggaccctgagatgggcatctctggccagctgacctggacacgcctgcctcagggcttcaagaatagcccaacactgttttgcgaggccctgcaccgcgacctggcagatttccggatccagcacccagatctgatcctgctgcagtactacgacgatctgctgctggccgccaccagcgagctggattgccagcagggaacacgcgccctgctgcagaccctgggaaacctgggatatagggcatccgccaagaaggcccagatctgtcagaagcaggtgaagtacctgggctatctgctgaaggagggccagagatggctgacagaggccaggaaggagacagtgatgggccagccaacacccaagaccccaagacagctgagggagttcctgggcaaagcaggattttgcaggctgttcatcccaggattcgcagagatggcagcacctctgtacccactgaccaagccgggcaccctgtttaattggggccctgaccagcagaaggcctatcaggagatcaagcaggccctgctgacagcaccagccctgggcctgccagacctgaccaagcctttcgagctgtttgtggatgagaagcagggctacgccaagggcgtgctgacccagaagctgggaccatggagacggcccgtggcctatctgtccaagaagctggacccagtggcagcaggatggccaccatgcctgaggatggtggcagcaatcgccgtgctgacaaaggatgccggcaagctgaccatgggacagccactggtcatcctggcaccacacgcagtggaggccctggtgaagcagcctccagatcgctggctgtctaacgcccggatgacacactaccaggccctgctgctggacaccgatcgcgtgcagtttggccctgtggtggccctgaatccagccaccctgctgcctctgccagaggagggcctgcagcacaactgtctggactctggcggctcaaaaagaaccgccgacggcagcgaattcgagtctcccaagaagaagaggaaagtcggctctggccctgccgctaagagagtgaagctggactaa

SEQ ID NO: 267 - DNA, 6024 bp, synthetic construct
  source 1..6024: mol_type = other DNA
atgaaacggacagccgacggaagcgagttcgagtcaccaaagaagaagcggaaagtcgacaagaagtacagcatcggcctggacatcggcaccaactctgtgggctgggccgtgatcaccgacgagtacaaggtgcccagcaagaaattcaaggtgctgggcaacaccgaccggcacagcatcaagaagaacctgatcggagccctgctgttcgacagcggcgaaacagccgaggccacccggctgaagagaaccgccagaagaagatacaccagacggaagaaccggatctgctatctgcaagagatcttcagcaacgagatggccaaggtggacgacagcttcttccggagactggaagagtccttcctggtggaagaggataagaagcacgagcggcaccccatcttcggcaacatcgtggacgaggtggcctaccacgagaagtaccccaccatctaccacctgagaaagaaactggtggacagcaccgacaaggccgacctgcggctgatctatctggccctggcccacatgatcaagttccggggccacttcctgatcgagggcgacctgaaccccgacaacagcgacgtggacaagctgttcatccagctggtgcagacctacaaccagctgttcgaggaaaaccccatcaacgccagcggcgtggacgccaaggccatcctgtctgccagactgagcaagagcagaaagctggaaaatctgatcgcccagctgcccggcgagaagaagaatggcctgttcggaaacctgattgccctgagcctgggcctgacccccaacttcaagagcaacttcgacctggccgaggatgccaaactgcagctgagcaaggacacctacgacgacgacctggacaacctgctggcccagatcggcgaccagtacgccgacctgtttctggccgccaagaacctgtccgacgccatcctgctgagcgacatcctgagagtgaacaccgagatcaccaaggcccccctgagcgcctctatgatcaagagatacgacgagcaccaccaggacctgaccctgctgaaagctctcgtgcggcagcagctgcctgagaagtacaaagagattttcttcgaccagagcaagaacggctacgccggctacattgacggcggagccagccaggaagagttctacaagttcatcaagcccatcctggaaaagatggacggcaccgaggaactgctcgtgaagctgaagagagaggacctgctgcggaagcagcggaccttcgacaacggcagcatcccccaccagatccacctgggagagctgcacgccattctgcggcggcaggaagatttttacccattcctgaaggacaaccgggaaaagatcgagaagatcctgaccttccgcatcccctactacgtgggccctctggccaggggaaacagcagattcgcctggatgaccagaaagagcgagaaaaccatcaccccctggaacttcgaggaagtggtggacaagggcgcttccgcccagagcttcatcgagcggatgaccaacttcgataagaacctgcccaacgagaaggtgctgcccaagcacagcctgctgtacgagtacttcaccgtgtataacgagctgaccaaagtgaaatacgtgaccgagggaatgagaaagcccgccttcctgagcggcgagcagaaaaaggccatcgtggacctgctgttcaagaccaaccggaaagtgaccgtgaagcagctgaaagaggactacttcaagaaaatcgagtgcttcgactccgtggaaatctccggcgtggaagatcggttcaacgcctccctgggcacataccacgatctgctgaaaattatcaaggacaaggacttcctggacaatgaggaaaacgaggacattctggaagatatcgtgctgaccctgacactgtttgaggacagagagatggtggaggaacggctgaaaacctatgcccacctgttcgacaacaaagtgatgaagcagctgaagcggcggagatacaccggctggggcaggctgagccggaagctgatcaacggcatccgggacaagcagtccggcaagacaatcctggatttcctgaagtccgacggcttcgccaacagaaacttcatgcagctgatccacgacgacagcctgacctttaaagaggacatccagaaagcccaggtgtccggccagggcgatagcctgtacgagcacattgccaatctggccggcagccccgccattaagaagggcatcctgcagacagtgaaggtggtggacgagctcgtgaaagtgatgggccggcacaagcccgagaacatcgtgatcgaaatggccagagagaaccagaccacccagaagggacagaagaacagccgcgagagaatgaagcggatcgaagagggcatcaaagagctgggcagccagatcctgaaagaacaccccgtggaaaacacccagctgcagaacgagaagctgtacctgtactacctgcagaatgggcgggatatgtacgtggaccaggaactggacatcaaccggctgtccgactacgatgtggacgctatcgtgcctcagagctttctgaaggacgactccatcgacaacaaggtgctgaccagaagcgacaagaaccggggcaagagcgacaacgtgccctccgaagaggtcgtgaagaagatgaagaactactggcggcagctgctgaacgccaagctgattacccagagaaagttcgacaatctgaccaaggccgagagaggcggcctgagcgaactggataaggccggcttcatcgccagacagctggtggaaacccggcagatcacaaagcacgtggcacagatcctggactcccggatgaacactaagtacgacgagaatgacaagctgatccgggaagtgaaagtgatcaccctgaagtccaagctggtgtccgatttccggaaggatttccagttttacaaagtgcgcgagatcaacaactaccaccacgcccacgacgcctacctgaacgccgtcgtgggaaccgccctgatcaaaaagtaccctaagctggaaagcgagttcgtgtacggcgactacaaggtgtacgacgtgcggaagatgatcgccaagagcgagcaggaaatcggcaaggctaccgccaagtacttcttctacagcaacatcatgaactttttcaagaccgagattaccctggccaacggcgagatccggaagcggcctctgatcgagacaaacggcgaaaccggggagatcgtgtgggataagggccgggattttgccaccgtgcggaaagtgctgagcatgccccaagtgaatatcgtgaaaaagaccgaggtgcagacaggcggcttcagcaaagagtctatcctgcccaagaggaacagcgataagctgatcgccagaaagaaggactgggaccctaagaagtacggcggcttcgacagccccaccgtggcctattctgtgctggtggtggccaaagtggaaaagggcaagtccaagaaactgaagagtgtgaaagagctgctggggatcaccatcatggaaagaagcagcttcgagaagaatcccatcgactttctggaagccaagggctacaaagaagtgaaaaaggacctgatcatcaagctgcctaagtactccctgttcgagctggaaaacggccggaagagaatgctggcctctgccggcgaactgcagaagggaaacgaactggccctgccctccaaatatgtgaacttcctgtacctggccagccactatgagaagctgaagggctcccccgaggataatgagcagaaacagctgtttgtggaacagcacaagcactacctggacgagatcatcgagcagatcagcgagttctccaagagagtgatcctggccgacgctaatctggacaaagtgctgtccgcctacaacaagcaccgggataagcccatcagagagcaggccgagaatatcatccacctgtttaccctgaccaatctgggagcccctgccgccttcaagtactttgacaccaccatcgaccggaagaggtacaccagcaccaaagaggtgctggacgccaccctgatccaccagagcatcaccggcctgtacgagacacggatcgacctgtctcagctgggaggtgactccggcggaagctctggtggcagcaagcggaccgccgacggctctgaattcgagagccctaagaagaaaagaaaggtgagcggaggctctagcggcggaagcaccctgaacattgaagacgagtatagactgcatgaaacaagcaaggaacccgacgtgtccctgggctccacctggctgtccgactttccccaggcctgggccgagacaggaggaatgggcctggccgtgcggcaggcacccctgatcatccctctgaaggccacctctacacccgtgagcatcaagcagtaccctatgtctcaggaggccagactgggcatcaagcctcacatccagaggctgctggaccagggcatcctggtgccatgccagagcccctggaacacaccactgctgcccgtgaagaagccaggcaccaatgactatagacccgtgcaggatctgagagaggtgaacaagagggtggaggatatccaccccaacgtgcccaacccttacaatctgctgtccggcctgcccccttctcaccagtggtatacagtgctggacctgaaggatgccttcttttgtctgagactgcaccctaccagccagccactgttcgcctttgagtggagggaccctgagatgggcatctctggccagctgacctggacacgcctgcctcagggcttcaagaatagcccaacactgttttgcgaggccctgcaccgcgacctggcagatttccggatccagcacccagatctgatcctgctgcagtactacgacgatctgctgctggccgccaccagcgagctggattgccagcagggaacacgcgccctgctgcagaccctgggaaacctgggatatagggcatccgccaagaaggcccagatctgtcagaagcaggtgaagtacctgggctatctgctgaaggagggccagagatggctgacagaggccaggaaggagacagtgatgggccagccaacacccaagaccccaagacagctgagggagttcctgggcaaagcaggattttgcaggctgttcatcccaggattcgcagagatggcagcacctctgtacccactgaccaagccgggcaccctgtttaattggggccctgaccagcagaaggcctatcaggagatcaagcaggccctgctgacagcaccagccctgggcctgccagacctgaccaagcctttcgagctgtttgtggatgagaagcagggctacgccaagggcgtgctgacccagaagctgggaccatggagacggcccgtggcctatctgtccaagaagctggacccagtggcagcaggatggccaccatgcctgaggatggtggcagcaatcgccgtgctgacaaaggatgccggcaagctgaccatgggacagccactggtcatcctggcaccacacgcagtggaggccctggtgaagcagcctccagatcgctggctgtctaacgcccggatgacacactaccaggccctgctgctggacaccgatcgcgtgcagtttggccctgtggtggccctgaatccagccaccctgctgcctctgccagaggagggcctgcagcacaactgtctggactctggcggctcaaaaagaaccgccgacggcagcgaattcgagtctcccaagaagaagaggaaagtcggctctggccctgccgctaagagagtgaagctggacgccacagtggtgtccggccaaaagcaggaccgccagggcggagaacgcagaaggtcccagctcgatagggatcagtgtgcctactgcaaggagaagggccactgggccaaagactgcccgaaaaagccgcgcggcccacgcggcccaaggccacaaacatccctcctttaa

SEQ ID NO: 268 - DNA, 5856 bp, synthetic construct
  source 1..5856: mol_type = other DNA
atgaaacggacagccgacggaagcgagttcgagtcaccaaagaagaagcggaaagtcgacaagaagtacagcatcggcctggacatcggcaccaactctgtgggctgggccgtgatcaccgacgagtacaaggtgcccagcaagaaattcaaggtgctgggcaacaccgaccggcacagcatcaagaagaacctgatcggagccctgctgttcgacagcggcgaaacagccgaggccacccggctgaagagaaccgccagaagaagatacaccagacggaagaaccggatctgctatctgcaagagatcttcagcaacgagatggccaaggtggacgacagcttcttccggagactggaagagtccttcctggtggaagaggataagaagcacgagcggcaccccatcttcggcaacatcgtggacgaggtggcctaccacgagaagtaccccaccatctaccacctgagaaagaaactggtggacagcaccgacaaggccgacctgcggctgatctatctggccctggcccacatgatcaagttccggggccacttcctgatcgagggcgacctgaaccccgacaacagcgacgtggacaagctgttcatccagctggtgcagacctacaaccagctgttcgaggaaaaccccatcaacgccagcggcgtggacgccaaggccatcctgtctgccagactgagcaagagcagaaagctggaaaatctgatcgcccagctgcccggcgagaagaagaatggcctgttcggaaacctgattgccctgagcctgggcctgacccccaacttcaagagcaacttcgacctggccgaggatgccaaactgcagctgagcaaggacacctacgacgacgacctggacaacctgctggcccagatcggcgaccagtacgccgacctgtttctggccgccaagaacctgtccgacgccatcctgctgagcgacatcctgagagtgaacaccgagatcaccaaggcccccctgagcgcctctatgatcaagagatacgacgagcaccaccaggacctgaccctgctgaaagctctcgtgcggcagcagctgcctgagaagtacaaagagattttcttcgaccagagcaagaacggctacgccggctacattgacggcggagccagccaggaagagttctacaagttcatcaagcccatcctggaaaagatggacggcaccgaggaactgctcgtgaagctgaagagagaggacctgctgcggaagcagcggaccttcgacaacggcagcatcccccaccagatccacctgggagagctgcacgccattctgcggcggcaggaagatttttacccattcctgaaggacaaccgggaaaagatcgagaagatcctgaccttccgcatcccctactacgtgggccctctggccaggggaaacagcagattcgcctggatgaccagaaagagcgagaaaaccatcaccccctggaacttcgaggaagtggtggacaagggcgcttccgcccagagcttcatcgagcggatgaccaacttcgataagaacctgcccaacgagaaggtgctgcccaagcacagcctgctgtacgagtacttcaccgtgtataacgagctgaccaaagtgaaatacgtgaccgagggaatgagaaagcccgccttcctgagcggcgagcagaaaaaggccatcgtggacctgctgttcaagaccaaccggaaagtgaccgtgaagcagctgaaagaggactacttcaagaaaatcgagtgcttcgactccgtggaaatctccggcgtggaagatcggttcaacgcctccctgggcacataccacgatctgctgaaaattatcaaggacaaggacttcctggacaatgaggaaaacgaggacattctggaagatatcgtgctgaccctgacactgtttgaggacagagagatggtggaggaacggctgaaaacctatgcccacctgttcgacaacaaagtgatgaagcagctgaagcggtgcagatacaccggctggggcaggctgagccggaagctgatcaacggcatccgggacaagcagtccggcaagacaatcctggatttcctgaagtccgacggcttcgccaacagaaacttcatgcagctgatccacgacgacagcctgacctttaaagaggacatccagaaagcccaggtgtccggccagggcgatagcctgtacgagcacattgccaatctggccggcagccccgccattaagaagggcatcctgcagacagtgaaggtggtggacgagctcgtgaaagtgatgggccggcacaagcccgagaacatcgtgatcgaaatggccagagagaaccagaccacccagaagggacagaagaacagccgcgagagaatgaagcggatcgaagagggcatcaaagagctgggcagccagatcctgaaagaacaccccgtggaaaacacccagctgcagaacgagaagctgtacctgtactacctgcagaatgggcgggatatgtacgtggaccaggaactggacatcaaccggctgtccgactacgatgtggacgctatcgtgcctcagagctttctgaaggacgactccatcgacaacaaggtgctgaccagaagcgacaagaaccggggcaagagcgacaacgtgccctccgaagaggtcgtgaagaagatgaagaactactggcggcagctgctgaacgccaagctgattacccagagaaagttcgacaatctgaccaaggccgagagaggcggcctgagcgaactggataaggccggcttcatcaagagacagctggtggaaacccggcagatcacaaagcacgtggcacagatcctggactcccggatgaacactaagtacgacgagaatgacaagctgatccgggaagtgaaagtgatcaccctgaagtccaagctggtgtccgatttccggaaggatttccagttttacaaagtgcgcgagatcaacaactaccaccacgcccacgacgcctacctgaacgccgtcgtgggaaccgccctgatcaaaaagtaccctaagctggaaagcgagttcgtgtacggcgactacaaggtgtacgacgtgcggaagatgatcgccaagagcgagcaggaaatcggcaaggctaccgccaagtacttcttctacagcaacatcatgaactttttcaagaccgagattaccctggccaacggcgagatccggaagcggcctctgatcgagacaaacggcgaaaccggggagatcgtgtgggataagggccgggattttgccaccgtgcggaaagtgctgagcatgccccaagtgaatatcgtgaaaaagaccgaggtgcagacaggcggcttcagcaaagagtctatcctgcccaagaggaacagcgataagctgatcgccagaaagaaggactgggaccctaagaagtacggcggcttcgacagccccaccgtggcctattctgtgctggtggtggccaaagtggaaaagggcaagtccaagaaactgaagagtgtgaaagagctgctggggatcaccatcatggaaagaagcagcttcgagaagaatcccatcgactttctggaagccaagggctacaaagaagtgaaaaaggacctgatcatcaagctgcctaagtactccctgttcgagctggaaaacggccggaagagaatgctggcctctgccggcgaactgcagaagggaaacgaactggccctgccctccaaatatgtgaacttcctgtacctggccagccactatgagaagctgaagggctcccccgaggataatgagcagaaacagctgtttgtggaacagcacaagcactacctggacgagatcatcgagcagatcagcgagttctccaagagagtgatcctggccgacgctaatctggacaaagtgctgtccgcctacaacaagcaccgggataagcccatcagagagcaggccgagaatatcatccacctgtttaccctgaccaatctgggagcccctgccgccttcaagtactttgacaccaccatcgaccggaagaggtacaccagcaccaaagaggtgctggacgccaccctgatccaccagagcatcaccggcctgtacgagacacggatcgacctgtctcagctgggaggtgactccggcggaagctctggtggcagcaagcggaccgccgacggctctgaattcgagagccctaagaagaaaagaaaggtgagcggaggctctagcggcggaagcaccctgaacattgaagacgagtatagactgcatgaaacaagcaaggaacccgacgtgtccctgggctccacctggctgtccgactttccccaggcctgggccgagacaggaggaatgggcctggccgtgcggcaggcacccctgatcatccctctgaaggccacctctacacccgtgagcatcaagcagtaccctatgtctcaggaggccagactgggcatcaagcctcacatccagaggctgctggaccagggcatcctggtgccatgccagagcccctggaacacaccactgctgcccgtgaagaagccaggcaccaatgactatagacccgtgcaggatctgagagaggtgaacaagagggtggaggatatccaccccaacgtgcccaacccttacaatctgctgtccggcctgcccccttctcaccagtggtatacagtgctggacctgaaggatgccttcttttgtctgagactgcaccctaccagccagccactgttcgcctttgagtggagggaccctgagatgggcatctctggccagctgacctggacacgcctgcctcagggcttcaagaatagcccaacactgttttgcgaggccctgcaccgcgacctggcagatttccggatccagcacccagatctgatcctgctgcagtactacgacgatctgctgctggccgccaccagcgagctggattgccagcagggaacacgcgccctgctgcagaccctgggaaacctgggatatagggcatccgccaagaaggcccagatctgtcagaagcaggtgaagtacctgggctatctgctgaaggagggccagagatggctgacagaggccaggaaggagacagtgatgggccagccaacacccaagaccccaagacagctgagggagttcctgggcaaagcaggattttgcaggctgttcatcccaggattcgcagagatggcagcacctctgtacccactgaccaagccgggcaccctgtttaattggggccctgaccagcagaaggcctatcaggagatcaagcaggccctgctgacagcaccagccctgggcctgccagacctgaccaagcctttcgagctgtttgtggatgagaagcagggctacgccaagggcgtgctgacccagaagctgggaccatggagacggcccgtggcctatctgtccaagaagctggacccagtggcagcaggatggccaccatgcctgaggatggtggcagcaatcgccgtgctgacaaaggatgccggcaagctgaccatgggacagccactggtcatcctggcaccacacgcagtggaggccctggtgaagcagcctccagatcgctggctgtctaacgcccggatgacacactaccaggccctgctgctggacaccgatcgcgtgcagtttggccctgtggtggccctgaatccagccaccctgctgcctctgccagaggagggcctgcagcacaactgtctggactctggcggctcaaaaagaaccgccgacggcagcgaattcgagtctcccaagaagaagaggaaagtcggctctggccctgccgctaagagagtgaagctggactaa

SEQ ID NO: 269 - DNA, 6024 bp, synthetic construct
  source 1..6024: mol_type = other DNA
atgaaacggacagccgacggaagcgagttcgagtcaccaaagaagaagcggaaagtcgacaagaagtacagcatcggcctggacatcggcaccaactctgtgggctgggccgtgatcaccgacgagtacaaggtgcccagcaagaaattcaaggtgctgggcaacaccgaccggcacagcatcaagaagaacctgatcggagccctgctgttcgacagcggcgaaacagccgaggccacccggctgaagagaaccgccagaagaagatacaccagacggaagaaccggatctgctatctgcaagagatcttcagcaacgagatggccaaggtggacgacagcttcttccggagactggaagagtccttcctggtggaagaggataagaagcacgagcggcaccccatcttcggcaacatcgtggacgaggtggcctaccacgagaagtaccccaccatctaccacctgagaaagaaactggtggacagcaccgacaaggccgacctgcggctgatctatctggccctggcccacatgatcaagttccggggccacttcctgatcgagggcgacctgaaccccgacaacagcgacgtggacaagctgttcatccagctggtgcagacctacaaccagctgttcgaggaaaaccccatcaacgccagcggcgtggacgccaaggccatcctgtctgccagactgagcaagagcagaaagctggaaaatctgatcgcccagctgcccggcgagaagaagaatggcctgttcggaaacctgattgccctgagcctgggcctgacccccaacttcaagagcaacttcgacctggccgaggatgccaaactgcagctgagcaaggacacctacgacgacgacctggacaacctgctggcccagatcggcgaccagtacgccgacctgtttctggccgccaagaacctgtccgacgccatcctgctgagcgacatcctgagagtgaacaccgagatcaccaaggcccccctgagcgcctctatgatcaagagatacgacgagcaccaccaggacctgaccctgctgaaagctctcgtgcggcagcagctgcctgagaagtacaaagagattttcttcgaccagagcaagaacggctacgccggctacattgacggcggagccagccaggaagagttctacaagttcatcaagcccatcctggaaaagatggacggcaccgaggaactgctcgtgaagctgaagagagaggacctgctgcggaagcagcggaccttcgacaacggcagcatcccccaccagatccacctgggagagctgcacgccattctgcggcggcaggaagatttttacccattcctgaaggacaaccgggaaaagatcgagaagatcctgaccttccgcatcccctactacgtgggccctctggccaggggaaacagcagattcgcctggatgaccagaaagagcgagaaaaccatcaccccctggaacttcgaggaagtggtggacaagggcgcttccgcccagagcttcatcgagcggatgaccaacttcgataagaacctgcccaacgagaaggtgctgcccaagcacagcctgctgtacgagtacttcaccgtgtataacgagctgaccaaagtgaaatacgtgaccgagggaatgagaaagcccgccttcctgagcggcgagcagaaaaaggccatcgtggacctgctgttcaagaccaaccggaaagtgaccgtgaagcagctgaaagaggactacttcaagaaaatcgagtgcttcgactccgtggaaatctccggcgtggaagatcggttcaacgcctccctgggcacataccacgatctgctgaaaattatcaaggacaaggacttcctggacaatgaggaaaacgaggacattctggaagatatcgtgctgaccctgacactgtttgaggacagagagatggtggaggaacggctgaaaacctatgcccacctgttcgacaacaaagtgatgaagcagctgaagcggtgcagatacaccggctggggcaggctgagccggaagctgatcaacggcatccgggacaagcagtccggcaagacaatcctggatttcctgaagtccgacggcttcgccaacagaaacttcatgcagctgatccacgacgacagcctgacctttaaagaggacatccagaaagcccaggtgtccggccagggcgatagcctgtacgagcacattgccaatctggccggcagccccgccattaagaagggcatcctgcagacagtgaaggtggtggacgagctcgtgaaagtgatgggccggcacaagcccgagaacatcgtgatcgaaatggccagagagaaccagaccacccagaagggacagaagaacagccgcgagagaatgaagcggatcgaagagggcatcaaagagctgggcagccagatcctgaaagaacaccccgtggaaaacacccagctgcagaacgagaagctgtacctgtactacctgcagaatgggcgggatatgtacgtggaccaggaactggacatcaaccggctgtccgactacgatgtggacgctatcgtgcctcagagctttctgaaggacgactccatcgacaacaaggtgctgaccagaagcgacaagaaccggggcaagagcgacaacgtgccctccgaagaggtcgtgaagaagatgaagaactactggcggcagctgctgaacgccaagctgattacccagagaaagttcgacaatctgaccaaggccgagagaggcggcctgagcgaactggataaggccggcttcatcaagagacagctggtggaaacccggcagatcacaaagcacgtggcacagatcctggactcccggatgaacactaagtacgacgagaatgacaagctgatccgggaagtgaaagtgatcaccctgaagtccaagctggtgtccgatttccggaaggatttccagttttacaaagtgcgcgagatcaacaactaccaccacgcccacgacgcctacctgaacgccgtcgtgggaaccgccctgatcaaaaagtaccctaagctggaaagcgagttcgtgtacggcgactacaaggtgtacgacgtgcggaagatgatcgccaagagcgagcaggaaatcggcaaggctaccgccaagtacttcttctacagcaacatcatgaactttttcaagaccgagattaccctggccaacggcgagatccggaagcggcctctgatcgagacaaacggcgaaaccggggagatcgtgtgggataagggccgggattttgccaccgtgcggaaagtgctgagcatgccccaagtgaatatcgtgaaaaagaccgaggtgcagacaggcggcttcagcaaagagtctatcctgcccaagaggaacagcgataagctgatcgccagaaagaaggactgggaccctaagaagtacggcggcttcgacagccccaccgtggcctattctgtgctggtggtggccaaagtggaaaagggcaagtccaagaaactgaagagtgtgaaagagctgctggggatcaccatcatggaaagaagcagcttcgagaagaatcccatcgactttctggaagccaagggctacaaagaagtgaaaaaggacctgatcatcaagctgcctaagtactccctgttcgagctggaaaacggccggaagagaatgctggcctctgccggcgaactgcagaagggaaacgaactggccctgccctccaaatatgtgaacttcctgtacctggccagccactatgagaagctgaagggctcccccgaggataatgagcagaaacagctgtttgtggaacagcacaagcactacctggacgagatcatcgagcagatcagcgagttctccaagagagtgatcctggccgacgctaatctggacaaagtgctgtccgcctacaacaagcaccgggataagcccatcagagagcaggccgagaatatcatccacctgtttaccctgaccaatctgggagcccctgccgccttcaagtactttgacaccaccatcgaccggaagaggtacaccagcaccaaagaggtgctggacgccaccctgatccaccagagcatcaccggcctgtacgagacacggatcgacctgtctcagctgggaggtgactccggcggaagctctggtggcagcaagcggaccgccgacggctctgaattcgagagccctaagaagaaaagaaaggtgagcggaggctctagcggcggaagcaccctgaacattgaagacgagtatagactgcatgaaacaagcaaggaacccgacgtgtccctgggctccacctggctgtccgactttccccaggcctgggccgagacaggaggaatgggcctggccgtgcggcaggcacccctgatcatccctctgaaggccacctctacacccgtgagcatcaagcagtaccctatgtctcaggaggccagactgggcatcaagcctcacatccagaggctgctggaccagggcatcctggtgccatgccagagcccctggaacacaccactgctgcccgtgaagaagccaggcaccaatgactatagacccgtgcaggatctgagagaggtgaacaagagggtggaggatatccaccccaacgtgcccaacccttacaatctgctgtccggcctgcccccttctcaccagtggtatacagtgctggacctgaaggatgccttcttttgtctgagactgcaccctaccagccagccactgttcgcctttgagtggagggaccctgagatgggcatctctggccagctgacctggacacgcctgcctcagggcttcaagaatagcccaacactgttttgcgaggccctgcaccgcgacctggcagatttccggatccagcacccagatctgatcctgctgcagtactacgacgatctgctgctggccgccaccagcgagctggattgccagcagggaacacgcgccctgctgcagaccctgggaaacctgggatatagggcatccgccaagaaggcccagatctgtcagaagcaggtgaagtacctgggctatctgctgaaggagggccagagatggctgacagaggccaggaaggagacagtgatgggccagccaacacccaagaccccaagacagctgagggagttcctgggcaaagcaggattttgcaggctgttcatcccaggattcgcagagatggcagcacctctgtacccactgaccaagccgggcaccctgtttaattggggccctgaccagcagaaggcctatcaggagatcaagcaggccctgctgacagcaccagccctgggcctgccagacctgaccaagcctttcgagctgtttgtggatgagaagcagggctacgccaagggcgtgctgacccagaagctgggaccatggagacggcccgtggcctatctgtccaagaagctggacccagtggcagcaggatggccaccatgcctgaggatggtggcagcaatcgccgtgctgacaaaggatgccggcaagctgaccatgggacagccactggtcatcctggcaccacacgcagtggaggccctggtgaagcagcctccagatcgctggctgtctaacgcccggatgacacactaccaggccctgctgctggacaccgatcgcgtgcagtttggccctgtggtggccctgaatccagccaccctgctgcctctgccagaggagggcctgcagcacaactgtctggactctggcggctcaaaaagaaccgccgacggcagcgaattcgagtctcccaagaagaagaggaaagtcggctctggccctgccgctaagagagtgaagctggacgccacagtggtgtccggccaaaagcaggaccgccagggcggagaacgcagaaggtcccagctcgatagggatcagtgtgcctactgcaaggagaagggccactgggccaaagactgcccgaaaaagccgcgcggcccacgcggcccaaggccacaaacatccctcctttaa

SEQ ID NO: 270 - DNA, 20 bp, synthetic construct
  source 1..20: mol_type = other DNA
ctgtaccaatcatacgacga

SEQ ID NO: 271 - DNA, 30 bp, synthetic construct
  source 1..30: mol_type = other DNA
tcacaggacaagtttcacgtcgtatgattc

SEQ ID NO: 272 - DNA, 20 bp, synthetic construct
  source 1..20: mol_type = other DNA
gcaagaagatcttgtttcgt

SEQ ID NO: 273 - DNA, 32 bp, synthetic construct
  source 1..32: mol_type = other DNA
agataacattcgaagtcatcgaaacaagatct

SEQ ID NO: 274 - DNA, 20 bp, synthetic construct
  source 1..20: mol_type = other DNA
aaaagaagcgttacaggcca

SEQ ID NO: 275 - DNA, 30 bp, synthetic construct
  source 1..30: mol_type = other DNA
tctcttttagagcaactggcctgtatcgat

SEQ ID NO: 276 - DNA, 20 bp, synthetic construct
  source 1..20: mol_type = other DNA
atctggaggttgtgaactaa

SEQ ID NO: 277 - DNA, 28 bp, synthetic construct
  source 1..28: mol_type = other DNA
taaagctatgtcctcaaagttcacaacc

SEQ ID NO: 278 - DNA, 4101 bp, synthetic construct
  source 1..4101: mol_type = other DNA
gacaagaagtacagcatcggcctggacatcggcaccaactctgtgggctgggccgtgatcaccgacgagtacaaggtgcccagcaagaaattcaaggtgctgggcaacaccgaccggcacagcatcaagaagaacctgatcggagccctgctgttcgacagcggcgaaacagccgaggccacccggctgaagagaaccgccagaagaagatacaccagacggaagaaccggatctgctatctgcaagagatcttcagcaacgagatggccaaggtggacgacagcttcttccacagactggaagagtccttcctggtggaagaggataagaagcacgagcggcaccccatcttcggcaacatcgtggacgaggtggcctaccacgagaagtaccccaccatctaccacctgagaaagaaactggtggacagcaccgacaaggccgacctgcggctgatctatctggccctggcccacatgatcaagttccggggccacttcctgatcgagggcgacctgaaccccgacaacagcgacgtggacaagctgttcatccagctggtgcagacctacaaccagctgttcgaggaaaaccccatcaacgccagcggcgtggacgccaaggccatcctgtctgccagactgagcaagagcagaaagctggaaaatctgatcgcccagctgcccggcgagaagaagaatggcctgttcggaaacctgattgccctgagcctgggcctgacccccaacttcaagagcaacttcgacctggccgaggatgccaaactgcagctgagcaaggacacctacgacgacgacctggacaacctgctggcccagatcggcgaccagtacgccgacctgtttctggccgccaagaacctgtccgacgccatcctgctgagcgacatcctgagagtgaacaccgagatcaccaaggcccccctgagcgcctctatgatcaagagatacgacgagcaccaccaggacctgaccctgctgaaagctctcgtgcggcagcagctgcctgagaagtacaaagagattttcttcgaccagagcaagaacggctacgccggctacattgacggcggagccagccaggaagagttctacaagttcatcaagcccatcctggaaaagatggacggcaccgaggaactgctcgtgaagctgaagagagaggacctgctgcggaagcagcggaccttcgacaacggcagcatcccccaccagatccacctgggagagctgcacgccattctgcggcggcaggaagatttttacccattcctgaaggacaaccgggaaaagatcgagaagatcctgaccttccgcatcccctactacgtgggccctctggccaggggaaacagcagattcgcctggatgaccagaaagagcgaggaaaccatcaccccctggaacttcgaggaagtggtggacaagggcgcttccgcccagagcttcatcgagcggatgaccaacttcgataagaacctgcccaacgagaaggtgctgcccaagcacagcctgctgtacgagtacttcaccgtgtataacgagctgaccaaagtgaaatacgtgaccgagggaatgagaaagcccgccttcctgagcggcgagcagaaaaaggccatcgtggacctgctgttcaagaccaaccggaaagtgaccgtgaagcagctgaaagaggactacttcaagaaaatcgagtgcttcgactccgtggaaatctccggcgtggaagatcggttcaacgcctccctgggcacataccacgatctgctgaaaattatcaaggacaaggacttcctggacaatgaggaaaacgaggacattctggaagatatcgtgctgaccctgacactgtttgaggacagagagatgatcgaggaacggctgaaaacctatgcccacctgttcgacgacaaagtgatgaagcagctgaagcggcggagatacaccggctggggcaggctgagccggaagctgatcaacggcatccgggacaagcagtccggcaagacaatcctggatttcctgaagtccgacggcttcgccaacagaaacttcatgcagctgatccacgacgacagcctgacctttaaagaggacatccagaaagcccaggtgtccggccagggcgatagcctgcacgagcacattgccaatctggccggcagccccgccattaagaagggcatcctgcagacagtgaaggtggtggacgagctcgtgaaagtgatgggccggcacaagcccgagaacatcgtgatcgaaatggccagagagaaccagaccacccagaagggacagaagaacagccgcgagagaatgaagcggatcgaagagggcatcaaagagctgggcagccagatcctgaaagaacaccccgtggaaaacacccagctgcagaacgagaagctgtacctgtactacctgcagaatgggcgggatatgtacgtggaccaggaactggacatcaaccggctgtccgactacgatgtggacgctatcgtgcctcagagctttctgaaggacgactccatcgacaacaaggtgctgaccagaagcgacaagaaccggggcaagagcgacaacgtgccctccgaagaggtcgtgaagaagatgaagaactactggcggcagctgctgaacgccaagctgattacccagagaaagttcgacaatctgaccaaggccgagagaggcggcctgagcgaactggataaggccggcttcatcaagagacagctggtggaaacccggcagatcacaaagcacgtggcacagatcctggactcccggatgaacactaagtacgacgagaatgacaagctgatccgggaagtgaaagtgatcaccctgaagtccaagctggtgtccgatttccggaaggatttccagttttacaaagtgcgcgagatcaacaactaccaccacgcccacgacgcctacctgaacgccgtcgtgggaaccgccctgatcaaaaagtaccctaagctggaaagcgagttcgtgtacggcgactacaaggtgtacgacgtgcggaagatgatcgccaagagcgagcaggaaatcggcaaggctaccgccaagtacttcttctacagcaacatcatgaactttttcaagaccgagattaccctggccaacggcgagatccggaagcggcctctgatcgagacaaacggcgaaaccggggagatcgtgtgggataagggccgggattttgccaccgtgcggaaagtgctgagcatgccccaagtgaatatcgtgaaaaagaccgaggtgcagacaggcggcttcagcaaagagtctatcctgcccaagaggaacagcgataagctgatcgccagaaagaaggactgggaccctaagaagtacggcggcttcctttggcccaccgtggcctattctgtgctggtggtggccaaagtggaaaagggcaagtccaagaaactgaagagtgtgaaagagctgctggggatcaccatcatggaaagaagcagcttcgagaagaatcccatcgactttctggaagccaagggctacaaagaagtgaaaaaggacctgatcatcaagctgcctaagtactccctgttcgagctggaaaacggccggaagagaatgctggcctctgccaagcaactgcagaagggaaacgaactggccctgccctccaaatatgtgaacttcctgtacctggccagccactatgagaagctgaagggctcccccgaggataatgagcagaaacagctgtttgtggaacagcacaagcactacctggacgagatcatcgagcagatcagcgagttctccaagagagtgatcctggccgacgctaatctggacaaagtgctgtccgcctacaacaagcaccgggataagcccatcagagagcaggccgagaatatcatccacctgtttaccctgaccaatctgggagcccctgccgccttcaagtactttgacaccaccatcgaccggaagcaatacaggagcaccaaagaggtgctggacgccaccctgatccaccagagcatcaccggcctgtacgagacacggatcgacctgtctcagctgggaggtgac